European Patent Specification EP 3 362 567 B1, published May 6, 2026. Title: GENETICALLY ENGINEERED BACTERIUM COMPRISING ENERGY-GENERATING FERMENTATION PATHWAY. Applicant: LanzaTech New Zealand Limited. The sequence listing filed with the application follows.

SEQUENCE LISTING (195 sequences)

SEQ ID NO: 1 - protein, 392 aa, Clostridium acetobutylicum
  MISC_FEATURE: ThlA, WP_010966157.1
MKEVVIASAVRTAIGSYGKSLKDVPAVDLGATAIKEAVKKAGIKPEDVNEVILGNVLQAGLGQNPARQASFKAGLPVEIPAMTINKVCGSGLRTVSLAAQIIKAGDADVIIAGGMENMSRAPYLANNARWGYRMGNAKFVDEMITDGLWDAFNDYHMGITAENIAERWNISREEQDEFALASQKKAEEAIKSGQFKDEIVPVVIKGRKGETVVDTDEHPRFGSTIEGLAKLKPAFKKDGTVTAGNASGLNDCAAVLVIMSAEKAKELGVKPLAKIVSYGSAGVDPAIMGYGPFYATKAAIEKAGWTVDELDLIESNEAFAAQSLAVAKDLKFDMNKVNVNGGAIALGHPIGASGARILVTLVHAMQKRDAKKGLATLCIGGGQGTAILLEKC

SEQ ID NO: 2 - protein, 393 aa, Cupriavidus necator
  MISC_FEATURE: PhaA, WP_013956452.1
MTDVVIVSAARTAVGKFGGSLAKIPAPELGAVVIKAALERAGVKPEQVSEVIMGQVLTAGSGQNPARQAAIKAGLPAMVPAMTINKVCGSGLKAVMLAANAIMAGDAEIVVAGGQENMSAAPHVLPGSRDGFRMGDAKLVDTMIVDGLWDVYNQYHMGITAENVAKEYGITREAQDELAVGSQNKAEAAQKAGKFDEEIVPVLIPQRKGDPVAFKTDEFVRQGATLDSMSGLKPAFDKAGTVTAANASGLNDGAAAVVVMSAAKAKELGLTPLATIKSYANAGVDPKVMGMGPVPASKRALSRAEWTPQDLDLMEINEAFAAQALAVHQQMGWDTSKVNVNGGAIAIGHPIGASGCRILVTLLHEMKRRDAKKGLASLCIGGGMGVALAVERK

SEQ ID NO: 3 - protein, 394 aa, Cupriavidus necator
  MISC_FEATURE: BktB, WP_011615089.1
MTREVVVVSGVRTAIGTFGGSLKDVAPAELGALVVREALARAQVSGDDVGHVVFGNVIQTEPRDMYLGRVAAVNGGVTINAPALTVNRLCGSGLQAIVSAAQTILLGDTDVAIGGGAESMSRAPYLAPAARWGARMGDAGLVDMMLGALHDPFHRIHMGVTAENVAKEYDISRAQQDEAALESHRRASAAIKAGYFKDQIVPVVSKGRKGDVTFDTDEHVRHDATIDDMTKLRPVFVKENGTVTAGNASGLNDAAAAVVMMERAEAERRGLKPLARLVSYGHAGVDPKAMGIGPVPATKIALERAGLQVSDLDVIEANEAFAAQACAVTKALGLDPAKVNPNGSGISLGHPIGATGALITVKALHELNRVQGRYALVTMCIGGGQGIAAIFERI

SEQ ID NO: 4 - protein, 394 aa, Escherichia coli
  MISC_FEATURE: AtoB, NP_416728.1
MKNCVIVSAVRTAIGSFNGSLASTSAIDLGATVIKAAIERAKIDSQHVDEVIMGNVLQAGLGQNPARQALLKSGLAETVCGFTVNKVCGSGLKSVALAAQAIQAGQAQSIVAGGMENMSLAPYLLDAKARSGYRLGDGQVYDVILRDGLMCATHGYHMGITAENVAKEYGITREMQDELALHSQRKAAAAIESGAFTAEIVPVNVVTRKKTFVFSQDEFPKANSTAEALGALRPAFDKAGTVTAGNASGINDGAAALVIMEESAALAAGLTPLARIKSYASGGVPPALMGMGPVPATQKALQLAGLQLADIDLIEANEAFAAQFLAVGKNLGFDSEKVNVNGGAIALGHPIGASGARILVTLLHAMQARDKTLGLATLCIGGGQGIAMVIERLN

SEQ ID NO: 5 - protein, 217 aa, Clostridium beijerinckii
  MISC_FEATURE: CtfA, WP_012059996.1
MNKLVKLTDLKRIFKDGMTIMVGGFLDCGTPENIIDMLVDLNIKNLTIISNDTAFPNKGIGKLIVNGQVSKVIASHIGTNPETGKKMSSGELKVELSPQGTLIERIRAAGSGLGGVLTPTGLGTIVEEGKKKVTIDGKEYLLELPLSADVSLIKGSIVDEFGNTFYRAATKNFNPYMAMAAKTVIVEAENLVKCEDLKRDAIMTPGVLVDYIVKEAA

SEQ ID NO: 6 - protein, 221 aa, Clostridium beijerinckii
  MISC_FEATURE: CtfB, WP_012059997.1
MIVDKVLAKEIIAKRVAKELKKDQLVNLGIGLPTLVANYVPKEMNITFESENGMVGMAQMASSGENDPDIINAGGEYVTLLPQGSFFDSSMSFALIRGGHVDVAVLGALEVDEKGNLANWIVPNKIVPGMGGAMDLAIGAKKIIVAMQHTGKSKPKIVKKCTLPLTAKAQVDLIVTELCVIDVTNDGLLLKEIHKDTTIDEIKFLTDADLIIPDNLKIMDI

SEQ ID NO: 7 - protein, 286 aa, Escherichia coli
  MISC_FEATURE: TesB, NP_414986.1
MSQALKNLLTLLNLEKIEEGLFRGQSEDLGLRQVFGGQVVGQALYAAKETVPEERLVHSFHSYFLRPGDSKKPIIYDVETLRDGNSFSARRVAAIQNGKPIFYMTASFQAPEAGFEHQKTMPSAPAPDGLPSETQIAQSLAHLLPPVLKDKFICDRPLEVRPVEFHNPLKGHVAEPHRQVWIRANGSVPDDLRVHQYLLGYASDLNFLPVALQPHGIGFLEPGIQIATIDHSMWFHRPFNLNEWLLYSVESTSASSARGFVRGEFYTQDGVLVASTVQEGVMRNHN

SEQ ID NO: 8 - protein, 436 aa, Clostridium autoethanogenum
  MISC_FEATURE: putative thioesterase 1, AGY74947.1
MNNDNCTIKITPEVSRVDEPVDIKINGLPKNEKVIIRAVSSDYYCINASILEIGDNTLWESYAVFETDECGNINFENAVPVDGTYSNCDKMGLFYSMRPKQIRKSKLIQKLSSINENRKYKITFTVEKNGKIIGSKEHTRVYCDDTIKSIDVVEKNLLARYFTSKDNIKHPAIIVLSGSDGRIEKAQAIAELFAMRGYSALAVCYFGLEGTPEDLNMIPLEYVENAVKWLKRQDTVDENKIAIYGRSKGGELVLLAASMFKDIACVIANTPSCYVYEGIKSNKLPSHHSSWMYRGREIPYLKFNFHIILRLIIKMMKKEKGALAWMYKKLIEEGDRDKATIALDKINGSVLMISSAADEIWPSKMHSETVCSIFEKSHFKHEYKHITFAKSGHILTVPFQSIYPSEKYPYDVESWAKANMDSWNETIKFLEKWASK

SEQ ID NO: 9 - protein, 137 aa, Clostridium autoethanogenum
  MISC_FEATURE: putative thioesterase 2, AGY75747.1
MYINETKVVVRYAETDKMGIVHHSNYYIYFEEARTQFIKKTGISYSQMEKDGIMFPLVESNCRYLQGAKYEDELLIKTWIKELTPVKAEFNYSVIRENDQKEIAKGSTLHAFVNNNFKIINLKKNHTELFKKLQSLI

SEQ ID NO: 10 - protein, 128 aa, Clostridium autoethanogenum
  MISC_FEATURE: putative thioesterase 3, AGY75999.1
MDFSKLFKVGSTYVSEYIVKPEDTANFIGNNGVVMLSTPAMIKYMEYTTLHIVDNVIPKNYRPVGTKIDVEHIKPIPANMKVVVKVTLISIEGKKLRYNVEAFNEKNCKVGFGIYEQQIVNLEQFLNR

SEQ ID NO: 11 - protein, 436 aa, Clostridium ljungdahlii; identical to SEQ ID NO: 8
  MISC_FEATURE: putative thioesterase 1, ADK15695.1

SEQ ID NO: 12 - protein, 137 aa, Clostridium ljungdahlii; identical to SEQ ID NO: 9
  MISC_FEATURE: putative thioesterase 2, ADK16655.1

SEQ ID NO: 13 - protein, 128 aa, Clostridium ljungdahlii; identical to SEQ ID NO: 10
  MISC_FEATURE: putative thioesterase 3, ADK16959.1

SEQ ID NO: 14 - protein, 246 aa, Clostridium beijerinckii
  MISC_FEATURE: Adc, WP_012059998.1
MLESEVSKQITTPLAAPAFPRGPYRFHNREYLNIIYRTDLDALRKIVPEPLELDRAYVRFEMMAMPDTTGLGSYTECGQAIPVKYNGVKGDYLHMMYLDNEPAIAVGRESSAYPKKLGYPKLFVDSDTLVGTLKYGTLPVATATMGYKHEPLDLKEAYAQIARPNFMLKIIQGYDGKPRICELICAENTDITIHGAWTGSARLQLFSHALAPLADLPVLEIVSASHILTDLTLGTPKVVHDYLSVK

SEQ ID NO: 15 - protein, 548 aa, Lactococcus lactis
  MISC_FEATURE: KivD
MYTVGDYLLDRLHELGIEEIFGVPGDYNLQFLDQIISHKDMKWVGNANELNASYMADGYARTKKAAAFLTTFGVGELSAVNGLAGSYAENLPVVEIVGSPTSKVQNEGKFVHHTLADGDFKHFMKMHEPVTAARTLLTAENATVEIDRVLSALLKERKPVYINLPVDVAAAKAEKPSLPLKKENSTSNTSDQEILNKIQESLKNAKKPIVITGHEIISFGLEKTVTQFISKTKLPITTLNFGKSSVDEALPSFLGIYNGTLSEPNLKEFVESADFILMLGVKLTDSSTGAFTHHLNENKMISLNIDEGKIFNERIQNFDFESLISSLLDLSEIEYKGKYIDKKQEDFVPSNALLSQDRLWQAVENLTQSNETIVAEQGTSFFGASSIFLKSKSHFIGQPLWGSIGYTFPAALGSQIADKESRHLLFIGDGSLQLTVQELGLAIREKINPICFIINNDGYTVEREIHGPNQSYNDIPMWNYSKLPESFGATEDRVVSKIVRTENEFVSVMKEAQADPNRMYWIELILAKEGAPKVLKKMGKLFAEQNKS

SEQ ID NO: 16 - protein, 351 aa, Clostridium autoethanogenum
  MISC_FEATURE: SecAdh, AGY74782.1
MKGFAMLGINKLGWIEKKNPVPGPYDAIVHPLAVSPCTSDIHTVFEGALGNRENMILGHEAVGEIAEVGSEVKDFKVGDRVIVPCTTPDWRSLEVQAGFQQHSNGMLAGWKFSNFKDGVFADYFHVNDADMNLAILPDEIPLESAVMMTDMMTTGFHGAELADIKMGSSVVVIGIGAVGLMGIAGSKLRGAGRIIGVGSRPVCVETAKFYGATDIVNYKNGDIVEQIMDLTHGKGVDRVIMAGGGAETLAQAVTMVKPGGVISNINYHGSGDTLPIPRVQWGCGMAHKTIRGGLCPGGRLRMEMLRDLVLYKRVDLSKLVTHVFDGAENIEKALLLMKNKPKDLIKSVVTF

SEQ ID NO: 17 - protein, 351 aa, Clostridium ljungdahlii; identical to SEQ ID NO: 16
  MISC_FEATURE: SecAdh, ADK15544.1

SEQ ID NO: 18 - protein, 351 aa, Clostridium ragsdalei; identical to SEQ ID NO: 16
  MISC_FEATURE: SecAdh, WP_013239134.1

SEQ ID NO: 19 - protein, 351 aa, Clostridium beijerinckii
  MISC_FEATURE: SecAdh, WP_026889046.1
MKGFAMLGINKLGWIEKERPVAGSYDAIVRPLAVSPCTSDIHTVFEGALGDRKNMILGHEAVGEVVEVGSEVKDFKPGDRVIVPCTTPDWRSLEVQAGFQQHSNGMLAGWKFSNFKDGVFGEYFHVNDADMNLAILPKDMPLENAVMITDMMTTGFHGAELADIQMGSSVVVIGIGAVGLMGIAGAKLRGAGRIIGVGSRPVCVETAKFYGATDILNYKNGHIVDQVMKLTNGKGVDRVIMAGGGSETLSQAVSMVKPGGIISNINYHGSGDALLIPRVEWGCGMAHKTIKGGLCPGGRLRAEMLRDMVVYNRVDLSKLVTHVYHGFDHIEEALLLMKDKPKDLIKAVVIL

SEQ ID NO: 20 - protein, 352 aa, Thermoanaerobacter brokii
  MISC_FEATURE: SecAdh, 3FSR_A
MKGFAMLSIGKVGWIEKEKPAPGPFDAIVRPLAVAPCTSDIHTVFEGAIGERHNMILGHEAVGEVVEVGSEVKDFKPGDRVVVPAITPDWRTSEVQRGYHQHSGGMLAGWKFSNVKDGVFGEFFHVNDADMNLAHLPKEIPLEAAVMIPDMMTTGFHGAELADIQMGSSVVVIGIGAVGLMGIAGAKLRGAGRIIGVGSRPICVEAAKFYGATDILNYKNGHIVDQVMKLTNGKGVDRVIMAGGGSETLSQAVSMVKPGGIISNINYHGSGDALLIPRVEWGCGMAHKTIKGGLCPGGRLRMERLIDLVFYKRVDPSKLVTHVFRGFDNIEKAFMLMKDKPKDLIKPVVILA

SEQ ID NO: 21 - protein, 520 aa, Mus musculus
  MISC_FEATURE: HMG-CoA synthase
MPGSLPLNAEACWPKDVGIVALEIYFPSQYVDQAELEKYDGVDAGKYTIGLGQARMGFCTDREDINSLCLTVVQKLMERHSLSYDCIGRLEVGTETIIDKSKSVKSKLMQLFEESGNTDIEGIDTTNACYGGTAAVFNAVNWVESSSWDGRYALVVAGDIAIYATGNARPTGGVGAVALLIGPNAPLIFDRGLRGTHMQHAYDFYKPDMLSEYPVVDGKLSIQCYLSALDRCYSVYRKKIRAQWQKEGKDKDFTLNDFGFMIFHSPYCKLVQKSLARMFLNDFLNDQNRDKNSIYSGLEAFGDVKLEDTYFDRDVEKAFMKASSELFNQKTKASLLVSNQNGNMYTSSVYGSLASVLAQYSPQQLAGKRVGVFSYGSGLAATLYSLKVTQDATPGSALDKITASLCDLKSRLDSRTCVAPDVFAENMKLREDTHHLANYIPQCSIDSLFEGTWYLVRVDEKHRRTYARRPFTNDHSLDEGMGLVHSNTATEHIPSPAKKVPRLPATSAESESAVISNGEH

SEQ ID NO: 22 - protein, 396 aa, Saccharomyces cerevisiae
  MISC_FEATURE: Mdd, CAA96324.1
MTVYTASVTAPVNIATLKYWGKRDTKLNLPTNSSISVTLSQDDLRTLTSAATAPEFERDTLWLNGEPHSIDNERTQNCLRDLRQLRKEMESKDASLPTLSQWKLHIVSENNFPTAAGLASSAAGFAALVSAIAKLYQLPQSTSEISRIARKGSGSACRSLFGGYVAWEMGKAEDGHDSMAVQIADSSDWPQMKACVLVVSDIKKDVSSTQGMQLTVATSELFKERIEHVVPKRFEVMRKAIVEKDFATFAKETMMDSNSFHATCLDSFPPIFYMNDTSKRIISWCHTINQFYGETIVAYTFDAGPNAVLYYLAENESKLFAFIYKLFGSVPGWDKKFTTEQLEAFNHQFESSNFTARELDLELQKDVARVILTQVGSGPQETNESLIDAKTGLPKE

SEQ ID NO: 23 - protein, 324 aa, Picrophilus torridus
  MISC_FEATURE: Mdd, WP_011178157.1
MENYNVKTRAFPTIGIILLGGISDKKNRIPLHTTAGIAYTGINNDVYTETKLYVSKDEKCYIDGKEIDLNSDRSPSKVIDKFKHEILMRVNLDDENNLSIDSRNFNILSGSSDSGAAALGECIESIFEYNINIFTFENDLQRISESVGRSLYGGLTVNYANGRESLTEPLLEPEAFNNFTIIGAHFNIDRKPSNEIHENIIKHENYRERIKSAERKAKKLEELSRNANIKGIFELAESDTVEYHKMLHDVGVDIINDRMENLIERVKEMKNNFWNSYIVTGGPNVFVITEKKDVDKAMEGLNDLCDDIRLLKVAGKPQVISKNF

SEQ ID NO: 24 - protein, 460 aa, Clostridium autoethanogenum
  MISC_FEATURE: CimA, AGY76958.1
MKKSSYEYKLNNVDSPNFYKNIFPYDEIPKINFNGVQIPKDLPENIYITDTTFRDGQQSMPPYTTEQIIRIFDYLHNLDNNSGIIKQTEFFLYTEKDRKAAQVCMERGYEFPEVTSWIRANKEDFKLVKQMGIKETGMLMSCSDYHIFKKLRKTRKETMDMYLGIVKEALDNGIRPRCHLEDITRADFYGFVVPLVNKLMELSKQSGIPIKIRACDTLGLGVSYSGVELPRSVQAIMYGLRNNCGVPSECIEWHGHNDFYAVVNNSTTAWLYGASAVNTSFLGIGERTGNCPLEAMIFEYGQIKGNTKNMKLEVITELSEYFKKEMEYAVPPRTPFVGKEFNVTRAGIHADGILKDEEIYNIFDTDKILGRPVVVAVNQYSGHAGIAAWINTYYRLKDEEKIDKWDTRIAKIKEWVDEQYKAGRTSIIGNDELELLVDKMLPDISQKKKKELARVDTRFI

SEQ ID NO: 25 - protein, 491 aa, Methanocaldococcus jannaschii
  MISC_FEATURE: CimA, NP_248395.1
MMVRIFDTTLRDGEQTPGVSLTPNDKLEIAKKLDELGVDVIEAGSAITSKGEREGIKLITKEGLNAEICSFVRALPVDIDAALECDVDSVHLVVPTSPIHMKYKLRKTEDEVLETALKAVEYAKEHGLIVELSAEDATRSDVNFLIKLFNEGEKVGADRVCVCDTVGVLTPQKSQELFKKITENVNLPVSVHCHNDFGMATANTCSAVLGGAVQCHVTVNGIGERAGNASLEEVVAALKILYGYDTKIKMEKLYEVSRIVSRLMKLPVPPNKAIVGDNAFAHEAGIHVDGLIKNTETYEPIKPEMVGNRRRIILGKHSGRKALKYKLDLMGINVSDEQLNKIYERVKEFGDLGKYISDADLLAIVREVTGKLVEEKIKLDELTVVSGNKITPIASVKLHYKGEDITLIETAYGVGPVDAAINAVRKAISGVADIKLVEYRVEAIGGGTDALIEVVVKLRKGTEIVEVRKSDADIIRASVDAVMEGINMLLN

SEQ ID NO: 26 - protein, 421 aa, Clostridium autoethanogenum
  MISC_FEATURE: LeuC, WP_023162955.1
MGMTMTQKILAHHAKMDEVKAGQLIKVKLDLVLGNDITTPVAINEFNKIGLNNVFDKNKIAIVPDHFTPNKDIKSAEQCKYVREFVKKMEIKNYFEVGRMGIEHALIPEKGLAVCGDVVIGADSHTCTYGALGAFSTGIGSTDMAAGMATGEAWFKVPEAIKFVLKGKLTKWVSGKDVILHIIGMIGVDGALYKSMEFTGEGVSSLTMDDRFTICNMAIEAGAKNGIFPVDENTINYVKEHSKKNYTVYEADSDAEYSQVIEIDLSKIRPTVAFPHIPENTKTIDEVGDIRIDQVVIGSCTNGRIGDLRAAASILKGRKVNENVRAIIFPATQAIYLQAMKEGLIEIFIEAGAVVSTPTCGPCLGGHMGILAEGERAVSTTNRNFVGRMGHVKSEVYLASPEVAAASAVTGKISSPEEVVK

SEQ ID NO: 27 - protein, 164 aa, Clostridium autoethanogenum
  MISC_FEATURE: LeuD, AGY77204.1
MIKGKAIKYGDNVDTDVIIPARYLNTSDHKELASHCMEDIDKDFSKKISKGDIMIAGKNFGCGSSREHAPIAIKASGISCIIAETFARIFFRNSINIGLPIMECEEAAKDIDEKDEVSVDTVSGVITNITKNKTYKAVPFPEFMHKIIKSEGLINYIKEEVENK

SEQ ID NO: 28 - protein, 466 aa, Escherichia coli
  MISC_FEATURE: LeuC, NP_414614.1
MAKTLYEKLFDAHVVYEAENETPLLYIDRHLVHEVTSPQAFDGLRAHGRPVRQPGKTFATMDHNVSTQTKDINACGEMARIQMQELIKNCKEFGVELYDLNHPYQGIVHVMGPEQGVTLPGMTIVCGDSHTATHGAFGALAFGIGTSEVEHVLATQTLKQGRAKTMKIEVQGKAAPGITAKDIVLAIIGKTGSAGGTGHVVEFCGEAIRDLSMEGRMTLCNMAIEMGAKAGLVAPDETTFNYVKGRLHAPKGKDFDDAVAYWKTLQTDEGATFDTVVTLQAEEISPQVTWGTNPGQVISVNDNIPDPASFADPVERASAEKALAYMGLKPGIPLTEVAIDKVFIGSCTNSRIEDLRAAAEIAKGRKVAPGVQALVVPGSGPVKAQAEAEGLDKIFIEAGFEWRLPGCSMCLAMNNDRLNPGERCASTSNRNFEGRQGRGGRTHLVSPAMAAAAAVTGHFADIRNIK

SEQ ID NO: 29 - protein, 201 aa, Escherichia coli
  MISC_FEATURE: LeuD, NP_414613.1
MAEKFIKHTGLVVPLDAANVDTDAIIPKQFLQKVTRTGFGAHLFNDWRFLDEKGQQPNPDFVLNFPQYQGASILLARENFGCGSSREHAPWALTDYGFKVVIAPSFADIFYGNSFNNQLLPVKLSDAEVDELFALVKANPGIHFDVDLEAQEVKAGEKTYRFTIDAFRRHCMMNGLDSIGLTLQHDDAIAAYEAKQPAFMN

SEQ ID NO: 30 - protein, 354 aa, Clostridium autoethanogenum
  MISC_FEATURE: LeuB, WP_023162957.1
MKIAIIPGDGIGKEIIEQAKKVLKAASAKYNFDFECEEVLLGGAAVDATGVPLPDKTVEVCKKSDAVLLGAVGGPKWDSLPSKLRPEAGLLGIRKALGVFANLRPAILFPELIAASNLKPEVLGGGLDIMIVRELIGGAYFGEKNRIDIEGGKKAWDTISYTSFEIDRITRKAFEIARKRSNRLTLVDKANVLESSKLWREVVGNIAKEYEDVEINYMYVDNASMQLIRDPKQFDVILTENMFGDILSDEASMLTGSLGMLPSASVRGDSFGLYEPVHGSAPDIAGQNKANPIGTIMSVAMMLKYSFDMEQAYVDIKNAISKVLKEGYRTGDIAKEDSKLVGTEEMGDLIVKNL

SEQ ID NO: 31 - protein, 363 aa, Escherichia coli
  MISC_FEATURE: LeuB, NP_414615.4
MSKNYHIAVLPGDGIGPEVMTQALKVLDAVRNRFAMRITTSHYDVGGAAIDNHGQPLPPATVEGCEQADAVLFGSVGGPKWEHLPPDQQPERGALLPLRKHFKLFSNLRPAKLYQGLEAFCPLRADIAANGFDILCVRELTGGIYFGQPKGREGSGQYEKAFDTEVYHRFEIERIARIAFESARKRRHKVTSIDKANVLQSSILWREIVNEIATEYPDVELAHMYIDNATMQLIKDPSQFDVLLCSNLFGDILSDECAMITGSMGMLPSASLNEQGFGLYEPAGGSAPDIAGKNIANPIAQILSLALLLRYSLDADDAACAIERAINRALEEGIRTGDLARGAAAVSTDEMGDIIARYVAEGV

SEQ ID NO: 32 - protein, 536 aa, Clostridium autoethanogenum
  MISC_FEATURE: IlvB, AGY74359.1
MKAAEAVIQCLKKENVNMVFGYPGAAVVPIYEALRKSDVKHILVRQEQAAGHSASGYARSTGEVGVCIVTSGPGATNLITAIAAAYMDSIPLVVITGQVKSTLIGRDVFQELDITGATESFTKYNFLVRDAKSIPKTIKEAFYIAETGRKGPVLVDIPMDIMEEDIDFEYPESVNIRGYKPTVKGHSGQIKKIIDRIKVSKRPLICAGGGVILANAQKELEQFVKKSHIPVVHTLMGKGCINENSDYYVGLIGTHGFAYANKVVQNADVLILIGARASDRTVSGVKSFAKDADIIHIDIDPAEIGKILNTYIPVVGDCGSVLSDLNKEIVAPQTEKWMEEIKNWKKDLYIERKPTDKVNPKYVLKTVSDTLGEEVILTADVGQNQLWCARNFRMTGNRKFLTSGGLGTMGYSLPAAIGAKIACPDKQVIAFAGDGGFQMSLFELGTIAENNLNIIIVLFNNSGLGMVREIQDNKYSGEFGVNFRTNPDFVKLAEAYGLKAKRVENDSEFNGVFREALDSSKAFLIECIVDPHERTF

SEQ ID NO: 33 - protein, 558 aa, Clostridium autoethanogenum
  MISC_FEATURE: IlvB, AGY74635.1
MKIKGAEVLLKCMMEQGVDTVFGYPGGAVLPIYDALYAAKGKITHISTSHEQGAAHAADGYARSTGKVGVVIATSGPGATNTVTAIATAYMDSVPIVVFTGQVARSLLGKDSFQEVNIKDITASITKKSCIVEKVEDLADTVREAFQIAVSGRPGPVVVDIPKDVQSAEVEYEPFRSKLSEIKEKKYFNLNEYGDSLNKAIDMINRSERPVIYSGGGTVTSGAQNELMELVEKIDSPITCSLMGIGAFPGNNEYYMGMVGMHGSRCSNYAVSNCDLLIAIGARFSDRVISKVSAFAPKARIIHIDIDPKEFGKNVDIDVAIKGDVKEVLQKINCKLEKADHRDWMEKIKQWKSEQCEPFKECKLSPKFIMDTLYNLTGGECIITTEVGQNQIWTAQYFKFLKPRTFVSSGGLGTMGFGLGASIGASMGNPGKKVINVAGDGSFKMNSTELATVAKYKLPIVQLLLNNRALGMVYQWQDMFYGKRFSNTELGPDVDFMKLGEAYGIKTFKIEDNSQVEKCLKEALDLNEPVIIECDIDRKEKVFPIVPPGAAISDLVEE

SEQ ID NO: 34 - protein, 158 aa, Clostridium autoethanogenum
  MISC_FEATURE: IlvN, AGY74360.1
MSVLVENHSGVLSKVAGLFSRRGYNIHSLTVGVTGDPEISRMTIVSIGDDYMFEQISKQLNKLIEVIKVIELNPDASVYRELSLIKVSAESNNKLLIMESVNTFRGKIVDMNEKSMIIEITGNEKKISAFIELMKPYGIKEIIRTGLTALQRGSKLED

SEQ ID NO: 35 - protein, 562 aa, Escherichia coli
  MISC_FEATURE: IlvB, NP_418127.1
MASSGTTSTRKRFTGAEFIVHFLEQQGIKIVTGIPGGSILPVYDALSQSTQIRHILARHEQGAGFIAQGMARTDGKPAVCMACSGPGATNLVTAIADARLDSIPLICITGQVPASMIGTDAFQEVDTYGISIPITKHNYLVRHIEELPQVMSDAFRIAQSGRPGPVWIDIPKDVQTAVFEIETQPAMAEKAAAPAFSEESIRDAAAMINAAKRPVLYLGGGVINAPARVRELAEKAQLPTTMTLMALGMLPKAHPLSLGMLGMHGVRSTNYILQEADLLIVLGARFDDRAIGKTEQFCPNAKIIHVDIDRAELGKIKQPHVAIQADVDDVLAQLIPLVEAQPRAEWHQLVADLQREFPCPIPKACDPLSHYGLINAVAACVDDNAIITTDVGQHQMWTAQAYPLNRPRQWLTSGGLGTMGFGLPAAIGAALANPDRKVLCFSGDGSLMMNIQEMATASENQLDVKIILMNNEALGLVHQQQSLFYEQGVFAATYPGKINFMQIAAGFGLETCDLNNEADPQASLQEIINRPGPALIHVRIDAEEKVYPMVPPGAANTEMVGE

SEQ ID NO: 36 - protein, 96 aa, Escherichia coli
  MISC_FEATURE: IlvN, NP_418126.1
MQNTTHDNVILELTVRNHPGVMTHVCGLFARRAFNVEGILCLPIQDSDKSHIWLLVNDDQRLEQMISQIDKLEDVVKVQRNQSDPTMFNKIAVFFQ

SEQ ID NO: 37 - protein, 337 aa, Clostridium autoethanogenum
  MISC_FEATURE: IlvC, WP_013238693.1
MEKLKVYYDEDADLNLLKGKKIAILGFGSQGHAHALNLKESGLDVIVGLYKGSKSWKKAEDYGFKVYEIAEAVKQADIITVLLPDEKQKQIYDESIKDNLSEGNALFFAHGFNIHFNQIVPPKFVDVLMIAPKGPGHIVRREYTLGNGVPCLYAVYQDYSGKGKEIALAYGKGIGGTRAGVMTTTFKVETETDLFGEQVVLCGGVAELIKAGFDTLVEAGYAPENAYFECLHEMKLIVDLIYEGGLARMRYSVSDTAEYGDYKIGKRIINDNTRAEMKKVLTEIQDGTFAREWLLENQTGRPGFTARRRMEKDAPIEKVGKELRSMMSWINENPDNE

SEQ ID NO: 38 - protein, 491 aa, Escherichia coli
  MISC_FEATURE: IlvC, NP_418222.1
MANYFNTLNLRQQLAQLGKCRFMGRDEFADGASYLQGKKVVIVGCGAQGLNQGLNMRDSGLDISYALRKEAIAEKRASWRKATENGFKVGTYEELIPQADLVINLTPDKQHSDVVRTVQPLMKDGAALGYSHGFNIVEVGEQIRKDITVVMVAPKCPGTEVREEYKRGFGVPTLIAVHPENDPKGEGMAIAKAWAAATGGHRAGVLESSFVAEVKSDLMGEQTILCGMLQAGSLLCFDKLVEEGTDPAYAEKLIQFGWETITEALKQGGITLMMDRLSNPAKLRAYALSEQLKEIMAPLFQKHMDDIISGEFSSGMMADWANDDKKLLTWREETGKTAFETAPQYEGKIGEQEYFDKGVLMIAMVKAGVELAFETMVDSGIIEESAYYESLHELPLIANTIARKRLYEMNVVISDTAEYGNYLFSYACVPLLKPFMAELQPGDLGKAIPEGAVDNGQLRDVNEAIRSHAIEQVGKKLRGYMTDMKRIAVAG

SEQ ID NO: 39 - protein, 552 aa, Clostridium autoethanogenum
  MISC_FEATURE: IlvD, WP_013238694.1
MKSDSVKKGIKAAPARALMYGMGYTKEEIERPLIGIVNSQNEIVAGHMHLDEIAKAAKLGVAMSGGTPIEFPAIAVCDGIAMGHVGMKYSLASRELIADSIEAMATAHGFDGLVLIPNCDKIVPGMLMAAARLNIPAVVVSGGPMRAGKLNNKALDFSTCIEKVAACSDGKVTEEELEEEAKRACPGCGSCSGLFTANSMNSLTEVLGMGLPLNGSALAQTGERNQLAKYAGMYVMDCVKNDRRPRDILTLDAFKNAITVDMAMAGSTNTVLHLPAIAHEAGIELNLDLFHEISKHTPCLTKLSPSGKHHMEDLHLAGGIPALMNELSKKGLINEDALTVTGKTVGETIKDFKVLDYEVIRSVDNAYSSEGGIAILRGNLAPDGAVVKESAVSKEMMVHEGPARVYNSEEAAVKAIFGNEINKGDVIVIRYEGPKGGPGMREMLSPTSAIAGMGLDKDVALLTDGRFSGATRGASIGHVSPEAMEGGLIGLVEEGDTIFVDITNKKLELKVSEEELEKRRKNYVKPEPKIKTGYLSRYAKLVTSANTGAVLK

SEQ ID NO: 40 - protein, 616 aa, Escherichia coli
  MISC_FEATURE: IlvD, YP_026248.1
MPKYRSATTTHGRNMAGARALWRATGMTDADFGKPIIAVVNSFTQFVPGHVHLRDLGKLVAEQIEAAGGVAKEFNTIAVDDGIAMGHGGMLYSLPSRELIADSVEYMVNAHCADAMVCISNCDKITPGMLMASLRLNIPVIFVSGGPMEAGKTKLSDQIIKLDLVDAMIQGADPKVSDSQSDQVERSACPTCGSCSGMFTANSMNCLTEALGLSQPGNGSLLATHADRKQLFLNAGKRIVELTKRYYEQNDESALPRNIASKAAFENAMTLDIAMGGSTNTVLHLLAAAQEAEIDFTMSDIDKLSRKVPQLCKVAPSTQKYHMEDVHRAGGVIGILGELDRAGLLNRDVKNVLGLTLPQTLEQYDVMLTQDDAVKNMFRAGPAGIRTTQAFSQDCRWDTLDDDRANGCIRSLEHAYSKDGGLAVLYGNFAENGCIVKTAGVDDSILKFTGPAKVYESQDDAVEAILGGKVVAGDVVVIRYEGPKGGPGMQEMLYPTSFLKSMGLGKACALITDGRFSGGTSGLSIGHVSPEAASGGSIGLIEDGDLIAIDIPNRGIQLQVSDAELAARREAQDARGDKAWTPKNRERQVSFALRAYASLATSADKGAVRDKSKLGG

SEQ ID NO: 41 - protein, 477 aa, Methanothermobacter thermautotrophicus
  MISC_FEATURE: VorA, WP_010876344.1
MTKKVIRKPDSLHDVFERKGGSAPTATHYCAGCGHGILHKLIGEAMDELGIQERAVMISPVGCAVFAYYYFDCGNVQVAHGRAPAVGTGISRAEDDAVVILYQGDGDLASIGLNETIQAANRGEKLAVFFVNNTVYGMTGGQMAPTTLVGEVTVTCPTGRDPRYAGYPLHMCELLDNLQAPVFIERVSLADPKRIRRARRAIKRALEIQRDGKGYAFVEVLSPCPTNLRQDAEGAERFLKEEMEKEFPVKNFRDRSAETEPLIRSESDFSRESLDRIFQIREDSVPDPVDDPEFPEVRVKIAGFGGQGVLSMGLTLAQAACSEGRHTSWYPAYGPEQRGGTSSCGVVISGERVGSPAVDTPDVLVALNQPSLDEFADDVADGGIILYDSTTASFSGGAVRAMGVPALEIARKHGTARAANTVMLGVMMALGLTGLDEESFREAIKFTFAGKEKIIDMNLRILEAGAEWARENIEGEL

SEQ ID NO: 42 - protein, 352 aa, Methanothermobacter thermautotrophicus
  MISC_FEATURE: VorB, WP_010876343.1
MATQMVKGNTAVIIGAMYAGCDCYFGYPITPASEILHEASRYFPMVGRKFVQAESEEAAINMVYGAAAAGHRVMTASSGPGISLKQEGISFLAGAELPAVIVDVMRAGPGLGNIGPEQGDYNQIVKGGGHGNYRNMVLAPSSVQEMCDLTMEAFELADKYRNPVVVLTDAVLGQMAEPLRFPEEAVEHRPDTSWAVCGNRETMKNLVTSIFLDFDELEEFNFYLQEKYARIEENEVRYEEYLVDDAEIVMVAYGISSRVARSAVETARAEGINVGLLRPITLFPFPSDRIRELADGGCRFISVEMSSGQMREDIRMASGCRDVELVNRMGGNLIELRDVLEKIREVAGDSSD

SEQ ID NO: 43 - protein, 79 aa, Methanothermobacter thermautotrophicus
  MISC_FEATURE: VorC, WP_010876342.1
MKKAYPVINSVECKACERCIIACPRKVLQMSSKINERGYHYVEYRGEGCNGCGNCYYTCPEINAIEVHIERCEDGNTDG

SEQ ID NO: 44 - protein, 124 aa, Methanothermobacter thermautotrophicus
  MISC_FEATURE: VorD, WP_010876341.1
MDEDGYMWFVGRTDDIIKSSGYRIGPFEVESAIISHPSVLECAVTGYPDPIRGQVVKATIVLARGYEPSEELKKEIQDHVKRVTAPYKYPRIVEFVDELPKTISGKIRRVEIREHDLEGDGENP

SEQ ID NO: 45 - protein, 394 aa, Pyrococcus furiosus
  MISC_FEATURE: VorA, WP_011012106.1
MEYKPIRKVVSGNYAAAYAALHARVQVVAAYPITPQTSIIEKIAEFIANGEADIQYIPVESEHSAMAACIGASATGARTFTATSAQGLALMHEMLHWAAGARLPIVMVDVNRAMAPPWSVWDDQTDSLSQRDTGWMQFYAENNQEVYDGVLMAYKVAETVNVPAMVVESAFILSHTYDVVEMIPQELVDEFLPPRKPLYSLANFDEPIAVGALATPNDYYEFRYKLAKAHEEAKKVIKEVGKEFGERFGRDYSQMIETGYIDDADFVFMGMGSLMGTVKEAVDLLRKEGYKVGYAKVRWFRPFPKEELVEIAESVKGIAVLDRNFSFGQEGILFTESKGALYNSSAHPLMKNYIVGLGGRDVTVKDIKAIADDMKKVIESGKVDKEVVWYHLKR

SEQ ID NO: 46 - protein, 311 aa, Pyrococcus furiosus
  MISC_FEATURE: VorB, WP_011012105.1
MEVPENIKKRVTIPFEEHFYAGHTACQGCGASLGLRYVLKAYGKKTILVIPACCSTIIAGPWPYSAIDANLFHTAFETTGAVISGIEAALKAMGYKVKGEDGIMVVGWAGDGGTADIGLQALSGFLERGHDAVYIMYDNEAYMNTGIQRSSSTPYGAWTTNTPGGRRHFLEKRHKKKVIDIVIAHRIPYAATASIAYPEDFIRKLKKAQKISGPSFIQLFAPCPTGWRAPTDKSIEIARLAVQTAYFPLFEYENGKYKINMPNPKKEPKPIEEFLKLQGRFKYMTKEDIETLQKWVLEEWERLKKLAEVFG

SEQ ID NO: 47 - protein, 185 aa, Pyrococcus furiosus
  MISC_FEATURE: VorC, WP_011012108.1
MIEVRFHGRGGQGAVTAANILAEAAFLEGKYVQAFPFFGVERRGAPVTAFTRIDNKPIRIKTQIYEPDVVVVLDPSLLDAVDVTAGLKDEGIVIVNTEKSKEEVLEKLKKKPKKLAIVDATTIALEILGLPITNTAILGAVAKATGLVKIESIEEAIKDTFSGELGEKNARAAREAYEKTEVFEL

SEQ ID NO: 48 - protein, 105 aa, Pyrococcus furiosus
  MISC_FEATURE: VorD, WP_011012107.1
MNTLFGKTKEEAKPIVLKSVDEYPEAPISLGTTLVNPTGDWRTFKPVVNEEKCVKCYICWKYCPEPAIYIKPDGYVAIDYDYCKGCGICANECPTKAITMIKEEK

SEQ ID NO: 49 - protein, 386 aa, Streptomyces avermitilis
  MISC_FEATURE: AcdH, AAD44196.1 or BAB69160.1
MDHRLTPELEELRRTVEEFAHDVVAPKIGDFYERHEFPYEIVREMGRMGLFGLPFPEEYGGMGGDYLALGIALEELARVDSSVAITLEAGVSLGAMPIHLFGTDAQKAEWLPRLCSGEILGAFGLTEPDGGSDAGATRTTARLDESTNEWVINGTKCFITNSGTDITGLVTVTAVTGRKPDGKPLISSIIVPSGTPGFTVAAPYSKVGWNASDTRELSFADVRVPAANLLGEQGRGYAQFLRILDEGRIAISALATGLAQGCVDESVKYAGERHAFGRNIGAYQAIQFKIADMEMKAHMARVGWRDAASRLVAGEPFKKEAAIAKLYSSTVAVDNAREATQIHGGYGFMNEYPVARMWRDSKILEIGEGTSEVQRMLIARELGLVG

SEQ ID NO: 50 - protein, 386 aa, Streptomyces coelicolor
  MISC_FEATURE: AcdH, AAD44195.1
MDHKLSPELEELRRTVEQFAHDVVAPKIGDFYERHEFPYEIVREMGRMGLFGLPFPEEYGGMGGDYFALGVALEELARVDSSVAITLEAGVSLGAMPLHLFGTEEQKREWLPRLCSGEILGAFGLTEPDGGSDAGATRTTARLDEATNEWVINGTKCFITNSGTDITGLVTVTAVTGRKPDGRPLISSIIVPSGTPGFTVAAPYSKVGWNASDTRELSFADVRVPAANLLGELGRGYAQFLRILDEGRVAIAALGTGLAQGCVDESVAYAKERHAFGRPIGANQAIQFKIADMEMKAHTARLAWRDAASRLVAGEPFKKEAALAKLYSSTVAVDNARDATQVHGGYGFMNEYPVARMWRDAKILEIGEGTSEVQRMLIARELGLVG

SEQ ID NO: 51 - protein, 261 aa, Clostridium beijerinckii
  MISC_FEATURE: Crt, ABR34202.1
MELKNVILEKEGHLAIVTINRPKALNALNSETLKDLDAVLEDLEKDSNMYTVIVTGAGEKSFVAGADISEMKDLNEEQGKEFGILGNNVFRRLERLDKPVIAAISGFALGGGCELAMSCDIRIASVKAKFGQPEAGLGITPGFGGTQRLARIVGPGKAKELIYTCDLINAEEAYRIGLVNKVVELEKLMEEAKAMANKIAANAPKAVAYCKDAIDRGMQVDIDAAILIEAEDFGKCFATEDQTEGMTAFLERRAEKNFQNK

SEQ ID NO: 52 - protein, 261 aa, Clostridium acetobutylicum
  MISC_FEATURE: Crt, NP_349318.1
MELNNVILEKEGKVAVVTINRPKALNALNSDTLKEMDYVIGEIENDSEVLAVILTGAGEKSFVAGADISEMKEMNTIEGRKFGILGNKVFRRLELLEKPVIAAVNGFALGGGCEIAMSCDIRIASSNARFGQPEVGLGITPGFGGTQRLSRLVGMGMAKQLIFTAQNIKADEALRIGLVNKVVEPSELMNTAKEIANKIVSNAPVAVKLSKQAINRGMQCDIDTALAFESEAFGECFSTEDQKDAMTAFIEKRKIEGFKNR

SEQ ID NO: 53 - protein, 397 aa, Treponema denticola
  MISC_FEATURE: Ccr, NP_971211.1
MIVKPMVRNNICLNAHPQGCKKGVEDQIEYTKKRITAEVKAGAKAPKNVLVLGCSNGYGLASRITAAFGYGAATIGVSFEKAGSETKYGTPGWYNNLAFDEAAKREGLYSVTIDGDAFSDEIKAQVIEEAKKKGIKFDLIVYSLASPVRTDPDTGIMHKSVLKPFGKTFTGKTVDPFTGELKEISAEPANDEEAAATVKVMGGEDWERWIKQLSKEGLLEEGCITLAYSYIGPEATQALYRKGTIGKAKEHLEATAHRLNKENPSIRAFVSVNKGLVTRASAVIPVIPLYLASLFKVMKEKGNHEGCIEQITRLYAERLYRKDGTIPVDEENRIRIDDWELEEDVQKAVSALMEKVTGENAESLTDLAGYRHDFLASNGFDVEGINYEAEVERFDRI

SEQ ID NO: 54 - protein, 539 aa, Euglena gracilis
  MISC_FEATURE: Ter, AAW66853.1
MSCPASPSAAVVSAGALCLCVATVLLATGSNPTALSTASTRSPTSLVRGVDRGLMRPTTAAALTTMREVPQMAEGFSGEATSAWAAAGPQWAAPLVAAASSALALWWWAARRSVRRPLAALAELPTAVTHLAPPMAMFTTTAKVIQPKIRGFICTTTHPIGCEKRVQEEIAYARAHPPTSPGPKRVLVIGCSTGYGLSTRITAAFGYQAATLGVFLAGPPTKGRPAAAGWYNTVAFEKAALEAGLYARSLNGDAFDSTTKARTVEAIKRDLGTVDLVVYSIAAPKRTDPATGVLHKACLKPIGATYTNRTVNTDKAEVTDVSIEPASPEEIADTVKVMGGEDWELWIQALSEAGVLAEGAKTVAYSYIGPEMTWPVYWSGTIGEAKKDVEKAAKRITQQYGCPAYPVVAKALVTQASSAIPVVPLYICLLYRVMKEKGTHEGCIEQMVRLLTTKLYPENGAPIVDEAGRVRVDDWEMAEDVQQAVKDLWSQVSTANLKDISDFAGYQTEFLRLFGFGIDGVDYDQPVDVEADLPSAAQQ

SEQ ID NO: 55 - protein, 282 aa, Clostridium beijerinckii
  MISC_FEATURE: Hbd, WP_011967675.1
MKKIFVLGAGTMGAGIVQAFAQKGCEVIVRDIKEEFVDRGIAGITKGLEKQVAKGKMSEEDKEAILSRISGTTDMKLAADCDLVVEAAIENMKIKKEIFAELDGICKPEAILASNTSSLSITEVASATKRPDKVIGMHFFNPAPVMKLVEIIKGIATSQETFDAVKELSVAIGKEPVEVAEAPGFVVNRILIPMINEASFILQEGIASVEDIDTAMKYGANHPMGPLALGDLIGLDVCLAIMDVLFTETGDNKYRASSILRKYVRAGWLGRKSGKGFYDYSK

SEQ ID NO: 56 - protein, 282 aa, Clostridium acetobutylicum
  MISC_FEATURE: Hbd, NP_349314.1
MKKVCVIGAGTMGSGIAQAFAAKGFEVVLRDIKDEFVDRGLDFINKNLSKLVKKGKIEEATKVEILTRISGTVDLNMAADCDLVIEAAVERMDIKKQIFADLDNICKPETILASNTSSLSITEVASATKRPDKVIGMHFFNPAPVMKLVEVIRGIATSQETFDAVKETSIAIGKDPVEVAEAPGFVVNRILIPMINEAVGILAEGIASVEDIDKAMKLGANHPMGPLELGDFIGLDICLAIMDVLYSETGDSKYRPHTLLKKYVRAGWLGRKSGKGFYDYSK

SEQ ID NO: 57 - protein, 282 aa, Clostridium kluyveri
  MISC_FEATURE: Hbd1, WP_011989027.1
MSIKSVAVLGSGTMSRGIVQAFAEAGIDVIIRGRTEGSIGKGLAAVKKAYDKKVSKGKISQEDADKIVGRVSTTTELEKLADCDLIIEAASEDMNIKKDYFGKLEEICKPETIFATNTSSLSITEVATATKRPDKFIGMHFFNPANVMKLVEIIRGMNTSQETFDIIKEASIKIGKTPVEVAEAPGFVVNKILVPMINEAVGILAEGIASAEDIDTAMKLGANHPMGPLALGDLIGLDVVLAVMDVLYSETGDSKYRAHTLLRKYVRAGWLGRKSGKGFFAY

SEQ ID NO: 58 - protein, 246 aa, Cupriavidus necator
  MISC_FEATURE: PhaB, WP_010810131.1
MTQRIAYVTGGMGGIGTAICQRLAKDGFRVVAGCGPNSPRREKWLEQQKALGFDFIASEGNVADWDSTKTAFDKVKSEVGEVDVLINNAGITRDVVFRKMTRADWDAVIDTNLTSLFNVTKQVIDGMADRGWGRIVNISSVNGQKGQFGQTNYSTAKAGLHGFTMALAQEVATKGVTVNTVSPGYIATDMVKAIRQDVLDKIVATIPVKRLGLPEEIASICAWLSSEESGFSTGADFSLNGGLHMG

SEQ ID NO: 59 - protein, 134 aa, Aeromonas caviae
  MISC_FEATURE: PhaJ, O32472
MSAQSLEVGQKARLSKRFGAAEVAAFAALSEDFNPLHLDPAFAATTAFERPIVHGMLLASLFSGLLGQQLPGKGSIYLGQSLSFKLPVFVGDEVTAEVEVTALREDKPIATLTTRIFTQGGALAVTGEAVVKLP

SEQ ID NO: 60 - protein, 260 aa, Ralstonia pickettii
  MISC_FEATURE: Bdh1, BAE72684.1
MQLKGKSAIVTGAASGIGKAIAELLAKEGAAVAIADLNLEAARAAAAGIEAAGGKAIAVAMDVTSEASVNQATDEVAQAFGNIDILVSNAGIQIVNPIQNYAFSDWKKMQAIHVDGAFLTTKAALKYMYRDKRGGTVIYMGSVHSHEASPLKSAYVAAKHALLGLARVLAKEGAEFNVRSHVICPGFVRTPLVDKQIPEQAKELGISEEEVVRRVMLGGTVDGVFTTVDDVARTALFLCAFPSAALTGQSFIVSHGWYMQ

SEQ ID NO: 61 - protein, 256 aa, Ralstonia pickettii
  MISC_FEATURE: Bdh2, BAE72685.1
MLQGKTALVTGSTCGIGLGIAQALAAQGANIIVNGFRRADGARQQIAAAGQVIRLGYHGADMSKASEIEDMMRYAEAEFAADILVNNAGIQHVASIEDFPPERWDAIIAINLTSAFHTTRLALPGMRQKNWGRVINIASTHGLVASAQKSAYVAAKHGIVGLTKVTALETAQNRVTANAICPGWVLTPLVQKQVQARPAHGISVEQAKRELVIEKQPSGQFVTPDELGALAVFLASEAGRQVRGAIWNMAGGWFAQ

SEQ ID NO: 62 - protein, 254 aa, Clostridium autoethanogenum
  MISC_FEATURE: Bdh, AGY75962
MRLENKVAIVTGSAMGIGKAIVRDFVNEGAKVIISDILEAEGQALEEELQKKGHSVYFFKTDVSSEKNIKELVKFTLEKFGTINILCNNAAVNIPGSVLELTEDIWNKTMDVNVKSHFLVSKHVIPVMQKAGGGSIVNTASANSFVAEPRLSAYVASKGAILMLTRAMALDFAKDNIRVNCICPGWVDTTFNDAHAELFGGREAVLKDLASVQPIGRPIAPMEIAKIATFLASDDSSCMTGSPVIADGGITAGV

SEQ ID NO: 63 - protein, 607 aa, Clostridium autoethanogenum
  MISC_FEATURE: AOR, WP_013238665.1
MYGYDGKVLRINLKERTCKSENLDLDKAKKFIGCRGLGVKTLFDEIDPKIDALSPENKFIIVTGPLTGAPVPTSGRFMVVTKAPLTGTIGISNSGGKWGVDLKKAGWDMIIVEDKADSPVYIEIVDDKVEIKDASQLWGKVTSETTKELEKITENKSKVLCIGPAGERLSLMAAVMNDVDRTAARGGVGAVMGSKNLKAITVKGTGKIALADKEKVKKVSVEKITTLKNDPVAGQGMPTYGTAILVNIINENGVHPVKNFQESYTNQADKISGETLTANQLVRKNPCYSCPIGCGRWVRLKDGTECGGPEYETLWCFGSDCGSYDLDAINEANMLCNEYGIDTITCGATIAAAMELYQRGYIKDEEIAGDNLSLKWGDTESMIGWIKRMVYSEGFGAKMTNGSYRLCEGYGAPEYSMTVKKQEIPAYDPRGIQGHGITYAVNNRGGCHIKGYMINPEILGYPEKLDRFALDGKAAYAKLFHDLTAVIDSLGLCIFTTFGLGIQDYVDMYNAVVGESTYDADSLLEAGDRIWTLEKLFNLAAGIDSSQDTLPKRLLEEPIPDGPSKGEVHRLDVLLPEYYSVRGWSKEGIPTEETLKKLGLDEYIGKF

SEQ ID NO: 64 - protein, 607 aa, Clostridium autoethanogenum
  MISC_FEATURE: AOR, WP_013238675.1
MYGYKGKVLRINLSSKTYIVEELKIDKAKKFIGARGLGVKTLFDEVDPKVDPLSPDNKFIIAAGPLTGAPVPTSGRFMVVTKSPLTGTIAIANSGGKWGAEFKAAGYDMIIVEGKSDKEVYVNIVDDKVEFRDASHVWGKLTEETTKMLQQETDSRAKVLCIGPAGEKLSLMAAVMNDVDRTAGRGGVGAVMGSKNLKAIVVKGSGKVKLFDEQKVKEVALEKTNILRKDPVAGGGLPTYGTAVLVNIINENGVHPVKNFQKSYTDQADKISGETLTKDCLVRKNPCYRCPIACGRWVKLDDGTECGGPEYETLWSFGSDCDVYDINAVNTANMLCNEYGLDTITAGCTIAAAMELYQRGYIKDEEIAADGLSLNWGDAKSMVEWVKKMGLREGFGDKMADGSYRLCDSYGVPEYSMTVKKQELPAYDPRGIQGHGITYAVNNRGGCHIKGYMVSPEILGYPEKLDRLAVEGKAGYARVFHDLTAVIDSLGLCIFTTFGLGAQDYVDMYNAVVGGELHDVNSLMLAGDRIWTLEKIFNLKAGIDSSQDTLPKRLLEEQIPEGPSKGEVHKLDVLLPEYYSVRGWDKNGIPTEETLKKLGLDEYVGKL

SEQ ID NO: 65 - protein, 607 aa, Clostridium ljungdahlii; identical to SEQ ID NO: 63
  MISC_FEATURE: AOR, ADK15073.1

SEQ ID NO: 66 - protein, 607 aa, Clostridium ljungdahlii; identical to SEQ ID NO: 64
  MISC_FEATURE: AOR, ADK15083.1

SEQ ID NO: 67 - protein, 405 aa, Clostridium autoethanogenum
  MISC_FEATURE: Adh, AGY76060.1
MKYMGIKIYGNKIRGIIMERFTLPRDIYFGEDALGALKTLKGKKAVVVVGGGSMKRFGFLDKVEEYLKEANIEVKLIEGVEPDPSVETVMKGAKIMTEFGPDWIVAIGGGSPIDAAKAMWLFYEYPDFTFKQAIVPFGLPELRQKAKFVAIASTSGTATEVTSFSVITDYKAKIKYPLADFNLTPDIAIVDPALAQTMPPKLTAHTGMDALTHALEAYVASARSDISDPLAIHSIIMTRDNLLKSYKGDKDARNKMHISQCLAGMAFSNALLGITHSLAHKTGAVWHIPHGCANAIYLPYVLDFNKKACSDRYANIAKILGLKGTTEDELVDSLVKMVQDMDKELNIPLTLKDYGISKDDFNSNVDFIAKNALLDACTGANPRPIDFDQMKKILQCIYDGKKVTF

SEQ ID NO: 68 - protein, 388 aa, Clostridium ljungdahlii
  MISC_FEATURE: Adh, ADK17019.1
MERFTLPRDIYFGEDALGALKTLKGKKAVVVVGGGSMKRFGFLDKVEEYLKEANIEVKLIEGVEPDPSVETVMKGAKIMTEFGPDWIVAIGGGSPIDAAKAMWLFYEYPDFTFKQAIVPFGLPELRQKAKFVAIASTSGTATEVTSFSVITDYKAKIKYPLADFNLTPDIAIVDPALAQTMPPKLTAHTGMDALTHALEAYVASARSDISDPLAIHSIIMTRDNLLKSYKGDKDARNKMHISQCLAGMAFSNALLGITHSLAHKTGAVWHIPHGCANAIYLPYVLDFNKKACSDRYANIAKILGLKGTTEDELVDSLVKMVQDMDKELNIPLTLKDYGISKDDFNSNVDFIAKNALLDACTGANPRPIDFDQMKKILQCIYDGKKVTF

SEQ ID NO: 69 - protein, 390 aa, Clostridium acetobutylicum
  MISC_FEATURE: BdhB, NP_349891.1
MVDFEYSIPTRIFFGKDKINVLGRELKKYGSKVLIVYGGGSIKRNGIYDKAVSILEKNSIKFYELAGVEPNPRVTTVEKGVKICRENGVEVVLAIGGGSAIDCAKVIAAACEYDGNPWDIVLDGSKIKRVLPIASILTIAATGSEMDTWAVINNMDTNEKLIAAHPDMAPKFSILDPTYTYTVPTNQTAAGTADIMSHIFEVYFSNTKTAYLQDRMAEALLRTCIKYGGIALEKPDDYEARANLMWASSLAINGLLTYGKDTNWSVHLMEHELSAYYDITHGVGLAILTPNWMEYILNNDTVYKFVEYGVNVWGIDKEKNHYDIAHQAIQKTRDYFVNVLGLPSRLRDVGIEEEKLDIMAKESVKLTGGTIGNLRPVNASEVLQIFKKSV

SEQ ID NO: 70 - protein, 387 aa, Clostridium beijerinckii
  MISC_FEATURE: Bdh, WP_041897187.1
MENFNYSIPTKVYFGKGQIKNLAAIIKEYGNKIFIAYGGGSIKKIGLYDEMIKILNDNSISYVELSGIEPNPRIETVRKGIKICKENNVEVVLAVGGGSTIDCAKVIAAGVKYEGDPWDLVTSPQKINEVLPIVTILTLSATGSEMDPHAVISDMTTNQKLGTGHENMKPKASILDPEYTYSVPKNQTAAGTADIMSHIFETYFNHTKGVDIQDSTAEGLLRACIKYGKIAIENPKDYDARANLMWASSWAINGLISYGTNSPWVVHPMEHELSAFYDITHGVGLAILTPHWMKYSLDDTTVFKFAQYGINVWGIDKNLDKFEIANKAIEKTSEFFKELGIPSTLREVGIEEEKLELMAKKAMNPYFKYAFKPLDENDILKIFKAAL

SEQ ID NO: 71 - protein, 388 aa, Clostridium ljungdahlii
  MISC_FEATURE: Bdh1, YP_003780648.1
MGRFTLPRDIYFGENALENLKNLDGNKAVVVVGGGSMKRFGFLAKVEKYLKETGMEVKLIEGVEPDPSVDTVMNGAKIMRDFNPDWIVSIGGGSPIDAAKAMWIFYEYPDFTFEKAVVPFGIPKLRQKAQFVAIPSTSGTATEVTSFSVITDYKAKIKYPLADFNLTPDIAIIDPSLAETMPKKLTAHTGMDALTHAIEAYVASLHSDFSDPLAMHAITMIHKYLLKSYEEDKEARGHMHIAQCLAGMAFSNALLGITHSIAHKTGAVFHIPHGCANAIYLPYVIDFNKKACSERYAKIAKKLHLSGNSEDELIDSLTEMIRTMNKKMDIPLTIKDYGISENDFNENLDFIAHNAMMDACTGSNPRAITEEEMKKLLQYMYNGQKVNF

SEQ ID NO: 72 - protein, 405 aa, Clostridium autoethanogenum; identical to SEQ ID NO: 67
  MISC_FEATURE: Bdh1, AGY76060.1

SEQ ID NO: 73 - protein, 388 aa, Clostridium ljungdahlii; identical to SEQ ID NO: 68
  MISC_FEATURE: Bdh2, YP_003782121.1

SEQ ID NO: 74 - protein, 388 aa, Clostridium autoethanogenum; identical to SEQ ID NO: 71
  MISC_FEATURE: Bdh2, AGY74784.1

SEQ ID NO: 75 - protein, 862 aa, Clostridium acetobutylicum
  MISC_FEATURE: AdhE1, NP_149325.1
MKVTTVKELDEKLKVIKEAQKKFSCYSQEMVDEIFRNAAMAAIDARIELAKAAVLETGMGLVEDKVIKNHFAGEYIYNKYKDEKTCGIIERNEPYGITKIAEPIGVVAAIIPVTNPTSTTIFKSLISLKTRNGIFFSPHPRAKKSTILAAKTILDAAVKSGAPENIIGWIDEPSIELTQYLMQKADITLATGGPSLVKSAYSSGKPAIGVGPGNTPVIIDESAHIKMAVSSIILSKTYDNGVICASEQSVIVLKSIYNKVKDEFQERGAYIIKKNELDKVREVIFKDGSVNPKIVGQSAYTIAAMAGIKVPKTTRILIGEVTSLGEEEPFAHEKLSPVLAMYEADNFDDALKKAVTLINLGGLGHTSGIYADEIKARDKIDRFSSAMKTVRTFVNIPTSQGASGDLYNFRIPPSFTLGCGFWGGNSVSENVGPKHLLNIKTVAERRENMLWFRVPHKVYFKFGCLQFALKDLKDLKKKRAFIVTDSDPYNLNYVDSIIKILEHLDIDFKVFNKVGREADLKTIKKATEEMSSFMPDTIIALGGTPEMSSAKLMWVLYEHPEVKFEDLAIKFMDIRKRIYTFPKLGKKAMLVAITTSAGSGSEVTPFALVTDNNTGNKYMLADYEMTPNMAIVDAELMMKMPKGLTAYSGIDALVNSIEAYTSVYASEYTNGLALEAIRLIFKYLPEAYKNGRTNEKAREKMAHASTMAGMASANAFLGLCHSMAIKLSSEHNIPSGIANALLIEEVIKFNAVDNPVKQAPCPQYKYPNTIFRYARIADYIKLGGNTDEEKVDLLINKIHELKKALNIPTSIKDAGVLEENFYSSLDRISELALDDQCTGANPRFPLTSEIKEMYINCFKKQP

SEQ ID NO: 76 - protein, 858 aa, Clostridium acetobutylicum
  MISC_FEATURE: AdhE2, NP_149199.1
MKVTNQKELKQKLNELREAQKKFATYTQEQVDKIFKQCAIAAAKERINLAKLAVEETGIGLVEDKIIKNHFAAEYIYNKYKNEKTCGIIDHDDSLGITKVAEPIGIVAAIVPTTNPTSTAIFKSLISLKTRNAIFFSPHPRAKKSTIAAAKLILDAAVKAGAPKNIIGWIDEPSIELSQDLMSEADIILATGGPSMVKAAYSSGKPAIGVGAGNTPAIIDESADIDMAVSSIILSKTYDNGVICASEQSILVMNSIYEKVKEEFVKRGSYILNQNEIAKIKETMFKNGAINADIVGKSAYIIAKMAGIEVPQTTKILIGEVQSVEKSELFSHEKLSPVLAMYKVKDFDEALKKAQRLIELGGSGHTSSLYIDSQNNKDKVKEFGLAMKTSRTFINMPSSQGASGDLYNFAIAPSFTLGCGTWGGNSVSQNVEPKHLLNIKSVAERRENMLWFKVPQKIYFKYGCLRFALKELKDMNKKRAFIVTDKDLFKLGYVNKITKVLDEIDIKYSIFTDIKSDPTIDSVKKGAKEMLNFEPDTIISIGGGSPMDAAKVMHLLYEYPEAEIENLAINFMDIRKRICNFPKLGTKAISVAIPTTAGTGSEATPFAVITNDETGMKYPLTSYELTPNMAIIDTELMLNMPRKLTAATGIDALVHAIEAYVSVMATDYTDELALRAIKMIFKYLPRAYKNGTNDIEAREKMAHASNIAGMAFANAFLGVCHSMAHKLGAMHHVPHGIACAVLIEEVIKYNATDCPTKQTAFPQYKSPNAKRKYAEIAEYLNLKGTSDTEKVTALIEAISKLKIDLSIPQNISAAGINKKDFYNTLDKMSELAFDDQCTTANPRYPLISELKDIYIKSF

SEQ ID NO: 77 - protein, 860 aa, Clostridium beijerinckii
  MISC_FEATURE: AdhE, WP_041893626.1
MRVTNPEELTKRIEQIREAQREFAKFSQEEVDEIFRQAAMAANDARITLAKMAVEESGMGIVEDKVIKNHFAAEYIYNQYKDTKTCGVIERDEMFGITHIAEPIGVIAAIVPTTNPTSTAIFKTLIALKTRNGIIISPHPRAKNSTIAAAKIVLEAAERAGAPKGIIGWIDEPSIELSRNVMSESDIILATGGPGMVRAAYSSGKPAIGVGAGNTPAIIDDTAHIKMAVNSILLSKTFDNGVVCASEQSIIAMESVYDEVRKELDERGAYILKGDEVDKVRSIILDPKGSLNSEIVGQSAYKIAKMAGVEVSEAVKVLIGEVESPELEEPFSHEKLSPILGMYKAKTFDDALRLASRMIELGGFGHTSILYTNQVESVDRIEKFGVAMKTARTLINMPASQGAIGDIYNFKLAPSLTLGCGSWGGNSISENVGPKHLINVKRIAERRENMLWFRVPDKIYFKFGCLPIALEELNAMKKKRAFIVTDRVLFDLGYTHKITDILSENHIEYKIFSDVEPDPTLKAAKLGADAMRDFNPDVIIAIGGGSPMDAAKIMWVMYEHPDVRFEDLAMRFMDIRKRVYEFPPMGERAILVAIPTSAGTGSEVTPFAVITDQQTGVKYPLADYALTPNMAIIDAELMMSMPKGLTAASGIDALVHAIEAYVSVLASEYTNGLALEAIRLTFKYLPDAYNGGTTNIKAREKMAHASSVAGMAFANAFLGICHSMAHKLGAFHHVPHGIANALLIDEVIRFNATDAPRKQAAFPQYKYPNAGWRYARIADYLNLGGNTEEEKVELLIKAIDDLKVKVRIPKSIKEFGVSEEKFYDSMDEMVEQAFDDQCTGANPRYPLMSEIKEMYIKSYN

SEQ ID NO: 78 - protein, 870 aa, Clostridium autoethanogenum
  MISC_FEATURE: AdhE1, WP_023163372.1
MKVTNVEELMKRLEEIKDAQKKFATYTQEQVDEIFRQAAMAANSARIELAKMAVEESGMGIVEDKVIKNHFASEYIYNKYKDEKTCGVLERDAGFGIVRIAEPVGVIAAVVPTTNPTSTAIFKSLIALKTRNGIIFSPHPRAKKSTIAAAKIVLDAAVKAGAPEGIIGWIDEPSIELSQVVMGEANLILATGGPGMVKAAYSSGKPAVGVGPGNTPAVIDESADIKMAVNSILLSKTFDNGMICASEQSVIVLDSIYEEVKKEFAYRGAYILSKDETDKVGKIILKNGALNAGIVGQPAFKIAQLAGVDVPEKAKVLIGEVESVELEEPFSHEKLSPVLAMYRARNFEDAIAKTDKLVRAGGFGHTSSLYINPMTEKAKVEKFSTMMKTSRTIINTPSSQGGIGDIYNFKLAPSLTLGCGSWGGNSVSENVGPKHLLNIKSVAERRENMLWFRVPEKVYFKYGSLGVALKELKVMNKKKVFIVTDKVLYQLGYVDKVTKVLEELKISYKVFTDVEPDPTLATAKKGAAELLSYEPDTIISVGGGSAMDAAKIMWVMYEHPEVKFEDLAMRFMDIRKRVYVFPKMGEKAMMISVATSAGTGSEVTPFAVITDEKTGAKYPLADYELTPDMAIVDAELMMGMPRGLTAASGIDALTHALEAYVSIMATEFTNGLALEAVKLIFEYLPKAYTEGTTNVKAREKMAHASCIAGMAFANAFLGVCHSMAHKLGAQHHIPHGIANALMIDEVIKFNAVDDPIKQAAFPQYEYPNARYRYAQIADCLNLGGNTEEEKVQLLINAIDDLKAKLNIPETIKEAGVSEDKFYATLDKMSELAFDDQCTGANPRYPLISEIKQMYINVFDKTEPIVEDEEK

SEQ ID NO: 79 - protein, 877 aa, Clostridium autoethanogenum
  MISC_FEATURE: AdhE2, WP_023163373.1
MKVTKVTNVEELMKKLDEVTAAQKKFSSYTQEQVDEIFRQAAMAANSARIDLAKMAVEESGMGIVEDKVIKNHFVAEYIYNKYKGEKTCGVLEQDEGFGMVRIAEPVGVIAAVVPTTNPTSTAIFKSLIALKTRNGIVFSPHPRAKKSTIAAAKIVLDAAVKAGAPEGIIGWIDEPSIELSQVVMKEADLILATGGPGMVKAAYSSGKPAIGVGPGNTPAVIDESADIKMAVNSILLSKTFDNGMICASEQSVIVASSIYDEVKKEFADRGAYILSKDETDKVGKTIMINGALNAGIVGQSAFKIAQMAGVSVPEDAKILIGEVKSVEPEEEPFAHEKLSPVLAMYKAKDFDEALLKAGRLVERGGIGHTSVLYVNSMTEKVKVEKFRETMKTGRTLINMPSAQGAIGDIYNFKLAPSLTLGCGSWGGNSVSENVGPKHLLNIKSVAERRENMLWFRVPEKVYFKYGSLGVALKELRIMEKKKAFIVTDKVLYQLGYVDKITKNLDELRVSYKIFTDVEPDPTLATAKKGAAELLSYEPDTIIAVGGGSAMDAAKIMWVMYEHPEVRFEDLAMRFMDIRKRVYVFPKMGEKAMMISVATSAGTGSEVTPFAVITDERTGAKYPLADYELTPNMAIVDAELMMGMPKGLTAASGIDALTHALEAYVSIMASEYTNGLALEATRLVFKYLPIAYTEGTINVKAREKMAHASCIAGMAFANAFLGVCHSMAHKLGAQHHIPHGIANALMIDEVIKFNAVEAPRKQAAFPQYKYPNVKRRYARIADYLNLGGSTDDEKVQLLINAIDDLKTKLNIPKTIKEAGVSEDKFYATLDTMSELAFDDQCTGANPRYPLIGEIKQMYINAFDTPKATVEKKTRKKK

SEQ ID NO: 80 - protein, 468 aa, Clostridium saccharoperbutylacetonicum
  MISC_FEATURE: Bld, AAP42563.1
MIKDTLVSITKDLKLKTNVENANLKNYKDDSSCFGVFENVENAISNAVHAQKILSLHYTKEQREKIITEIRKAALENKEILATMILEETHMGRYEDKILKHELVAKYTPGTEDLTTTAWSGDNGLTVVEMSPYGVIGAITPSTNPTETVICNSIGMIAAGNTVVFNGHPGAKKCVAFAVEMINKAIISCGGPENLVTTIKNPTMDSLDAIIKHPSIKLLCGTGGPGMVKTLLNSGKKAIGAGAGNPPVIVDDTADIEKAGKSIIEGCSFDNNLPCIAEKEVFVFENVADDLISNMLKNNAVIINEDQVSKLIDLVLQKNNETQEYSINKKWVGKDAKLFLDEIDVESPSSVKCIICEVSARHPFVMTELMMPILPIVRVKDIDEAIEYAKIAEQNRKHSAYIYSKNIDNLNRFEREIDTTIFVKNAKSFAGVGYEAEGFTTFTIAGSTGEGITSARNFTRQRRCVLAG

SEQ ID NO: 81 - protein, 562 aa, Aquincola tertiaricarbonis
  MISC_FEATURE: HcmAB, large subunit, AFK77668.1
MTWLEPQIKSQLQSERKDWEANEVGAFLKKAPERKEQFHTIGDFPVQRTYTAADIADTPLEDIGLPGRYPFTRGPYPTMYRSRTWTMRQIAGFGTGEDTNKRFKYLIAQGQTGISTDFDMPTLMGYDSDHPMSDGEVGREGVAIDTLADMEALLADIDLEKISVSFTINPSAWILLAMYVALGEKRGYDLNKLSGTVQADILKEYMAQKEYIYPIAPSVRIVRDIITYSAKNLKRYNPINISGYHISEAGSSPLQEAAFTLANLITYVNEVTKTGMHVDEFAPRLAFFFVSQGDFFEEVAKFRALRRCYAKIMKERFGARNPESMRLRFHCQTAAATLTKPQYMVNVVRTSLQALSAVLGGAQSLHTNGYDEAFAIPTEDAMKMALRTQQIIAEESGVADVIDPLGGSYYVEALTTEYEKKIFEILEEVEKRGGTIKLIEQGWFQKQIADFAYETALRKQSGQKPVIGVNRFVENEEDVKIEIHPYDNTTAERQISRTRRVRAERDEAKVQAMLDQLVAVAKDESQNLMPLTIELVKAGATMGDIVEKLKGIWGTYRETPVF

SEQ ID NO: 82 - protein, 136 aa, Aquincola tertiaricarbonis
  MISC_FEATURE: HcmAB, small subunit, AFK77665.1
MDQTPIRVLLAKVGLDGHDRGVKVVARALRDAGMDVIYSGLHRTPEEVVNTAIQEDVDVLGVSLLSGVQLTVFPKIFKLLDERGAGDLIVIAGGVMPDEDAAAIRKLGVREVLLQDTPPQAIIDSIRSLVAARGAR

SEQ ID NO: 83 - protein, 563 aa, Kyrpidia tusciae
  MISC_FEATURE: HcmAB, large subunit, WP_013074530.1
MADQEKLFNGDEIRRIRQEKERWYRETVKGNDGGNDYVTDSGIPVNLIYGPDDIADFDYLKESGFSGEPPYVRGVYPNMYRGRLFTIRQIAGFGTPEDTNRRFKFLLENGATGTSVVLDLPTIRGYDSDDPKAEGHVGAAGVAIDSLEDMEALYDGIPIDQVSSNIVTHLPSTTVVLMAMFVAMAEKRGLPLEKLSGTNQNDFLMETTIGSSLEILPPKASFRLQCDSIEYASKRLPRWNPVSYNGYNLREAGTTAVQEVGCAIANAIATTEELIRRGNDVDDFAKRLSFFWNLFNDFFEEIAKCRASRLVWYDVMKNRFGAKNPRSYLMRFHVQTGGITLTKVEPLNNIARSAIQGLAAVLGGAQSLHIDSYDEAYSAPTEQAALVSLRTQQIIQVETGVVNTVDPLAGSYYVEYLTREMAEHIRAYIDQIESRGGIIAVVESGWLHREIAEFAYRTQQDIETGKRKVVGLNYFPSKEAETKVEVFRYPEDAERMQKEKLAKLRARRDPVKVEQTLRVLREKCHEDVNILPYVKDAVEAYCTLGEIQNVFREEFGLWQFPLV

SEQ ID NO: 84 - protein, 132 aa, Kyrpidia tusciae
  MISC_FEATURE: HcmAB, small subunit, WP_013074531.1
MEKKIKVIMVKLGLDIHWRGALVVSKMLRDRGMEVVYLGNLFPEQIVQAAVQEGADVVGLSTLGGNHLTLGPKVVELLRAKGMEEVLVIMGGVIPEEDVPALKEAGIAEVFGPETPIDAIESFIRSRFPDRD

SEQ ID NO: 85 - protein, 327 aa, Aquincola tertiaricarbonis
  MISC_FEATURE: MeaB, AFK77667.1
MTYVPSSALLEQLRAGNTWALGRLISRAEAGVAEARPALAEVYRHAGSAHVIGLTGVPGSGKSTLVAKLTAALRKRGEKVGIVAIDPSSPYSGGAILGDRIRMTELANDSGVFIRSMATRGATGGMARAALDAVDLLDVAGYHTIILETVGVGQDEVEVAHASDTTVVVSAPGLGDEIQAIKAGVLEIADIHVVSKCDRDDANRTLTDLKQMLTLGTMVGPKRAWAIPVVGVSSYTGEGVDDLLGRIAAHRQATADTELGRERRRRVAEFRLQKTAETLLLERFTTGAQPFSPALADSLSNRASDPYAAARELIARTIRKEYSNDLA

SEQ ID NO: 86 - protein, 312 aa, Kyrpidia tusciae
  MISC_FEATURE: MeaB, WP_013074529.1
MQELLSRFDAGDPVALGKLLKEVENGTSSGKEALRCTASRQGRAHVVGITGPPGAGKSTLTAKLSKRWAEAGREVGIVCVDPTSPFSGGALLGDRIRMLELSSFPNVFIKSLATRGSLGGMAASTADIIQLMDAYGKEVVVVETVGVGQVEFDVMDLSDTVVLVNVPGLGDSIQALKAGILEIADIFVINQADRPGAEDSVRDLRQMLADRKETGWLWPVVKTVATRGEGIDRLAEAIESHRAYLKREQLWEEKRCRRNRQRLMQEMDRLFRQHVLTRIRTDPTARALFEEVEKGTQDPYSAARHLFQEIVN

SEQ ID NO: 87 - protein, 301 aa, Clostridium acetobutylicum
  MISC_FEATURE: Ptb, WP_010966357.1
MIKSFNEIIMKVKSKEMKKVAVAVAQDEPVLEAVRDAKKNGIADAILVGDHDEIVSIALKIGMDVNDFEIVNEPNVKKAALKAVELVSTGKADMVMKGLVNTATFLRSVLNKEVGLRTGKTMSHVAVFETEKFDRLLFLTDVAFNTYPELKEKIDIVNNSVKVAHAIGIENPKVAPICAVEVINPKMPSTLDAAMLSKMSDRGQIKGCVVDGPLALDIALSEEAAHHKGVTGEVAGKADIFLMPNIETGNVMYKTLTYTTDSKNGGILVGTSAPVVLTSRADSHETKMNSIALAALVAGNK

SEQ ID NO: 88 - protein, 302 aa, Clostridium beijerinckii
  MISC_FEATURE: Ptb
MSKNFDELLSRLKEVPTKKVAVAVAQDEPVLEAIKEATENNIAEAILVGDKQQIHEIAKKINLDLSDYEIMDIKDPKKATLEAVKLVSSGHADMLMKGLVDTATFLRSVLNKEVGLRTGKLMSHVAVFDVEGWDRLLFLTDAAFNTYPEFKDKVGMINNAVVVAHACGIDVPRIAPICPVEVVNTSMQSTVDAALLAKMSDRGQIKGCIIDGPFALDNAISEEAAHHKGVTGSVAGKADILLLPNIEAANVMYKTLTYFSKSRNGGLLVGTSAPVILTSRADSFETKVNSIALAALVAARNK

SEQ ID NO: 89 - protein, 302 aa, Clostridium beijerinckii
  MISC_FEATURE: Ptb, WP_041893500.1
MSKNFDELLSRLKEVPTKKVAVAVAQDEPVLEAIKEATENNIAQAILVGDKQQIHEIAKKINLDLSDYEIMDIKDPKKATLEAVKLVSSGHADMLMKGLVDTATFLRSVLNKEVGLRTGKLMSHVAVFDVEGWDRLLFLTDAAFNTYPEFKDKVGMINNAVVVAHACGIDVPRIAPICPVEVVNTSMQSTVDAALLAKMSDRGQIKGCVIDGPFALDNAISEEAAHHKGVTGSVAGKADILLLPNIEAANVMYKTLTYFSKSRNGGLLVGTSAPVILTSRADSFETKVNSIALAALVAARNK

SEQ ID NO: 90 - protein, 355 aa, Clostridium acetobutylicum
  MISC_FEATURE: Buk, WP_010966356.1
MYRLLIINPGSTSTKIGIYDDEKEIFEKTLRHSAEEIEKYNTIFDQFQFRKNVILDALKEANIEVSSLNAVVGRGGLLKPIVSGTYAVNQKMLEDLKVGVQGQHASNLGGIIANEIAKEINVPAYIVDPVVVDELDEVSRISGMADIPRKSIFHALNQKAVARRYAKEVGKKYEDLNLIVVHMGGGTSVGTHKDGRVIEVNNTLDGEGPFSPERSGGVPIGDLVRLCFSNKYTYEEVMKKINGKGGVVSYLNTIDFKAVVDKALEGDKKCALIYEAFTFQVAKEIGKCSTVLKGNVDAIILTGGIAYNEHVCNAIEDRVKFIAPVVRYGGEDELLALAEGGLRVLRGEEKAKEYK

SEQ ID NO: 91 - protein, 355 aa, Clostridium beijerinckii
  MISC_FEATURE: Buk, WP_011967556
MSYKLLIINPGSTSTKIGVYEGEKELFEETLRHTNEEIKRYDTIYDQFEFRKEVILNVLKEKNFDIKTLSAIVGRGGMLRPVEGGTYAVNDAMVEDLKVGVQGPHASNLGGIIAKSIGDELNIPSFIVDPVVTDELADVARLSGVPELPRKSKFHALNQKAVAKRYGKESGQGYENLNLVVVHMGGGVSVGAHNHGKVVDVNNALDGDGPFSPERAGSVPIGDLVKMCFSGKYSEAEVYGKAVGKGGFVGYLNTNDVKGVIDKMEEGDKECESIYKAFVYQISKAIGEMSVVLEGKVDQIIFTGGIAYSPTLVPDLKAKVEWIAPVTVYPGEDELLALAQGAIRVLDGEEQAKVY

SEQ ID NO: 92 - protein, 355 aa, Clostridium beijerinckii
  MISC_FEATURE: Buk, WP_017209677
MSYKLLIINPGSTSTKIGVYEGEKELFEETLRHTNEEIKRYDTIYDQFEFRKEVILNVLKEKNFDIKTLSAIVGRGGMLRPVEGGTYAVNDAMVEDLKVGVQGPHASNLGGIIAKSIGDELNIPSFIVDPVVTDELADVARLSGVPELPRKSKFHALNQKAVAKRYGKESGQGYENLNLVVVHMGGGVSVGAHNHGKVVDVNNALDGDGPFSPERAGSVPIGDLVKMCFSGKYSEAEVYGKVVGKGGFVGYLNTNDVKGVIDKMEEGDKECGSIYKAFVYQISKAIGEMSVVLEGKVDQIIFTGGIAYSPTLVPDLKAKVEWIAPVTVYPGEDELLALAQGAIRVLDGEEQAKVY

SEQ ID NO: 93 - protein, 355 aa, Clostridium beijerinckii
  MISC_FEATURE: Buk, WP_026886638
MSYKLLIINPGSTSTKIGVYEGEKELFEETLRHTNEEIKRYDTIYDQFEFRKEVILNVLKEKNFDIKTLSAIVGRGGMLRPVEGGTYAVNDAMVEDLKVGVQGPHASNLGGIIAKSIGDELNIPSFIVDPVVTDELADVARLSGVPELPRKSKFHALNQKAVAKRYGKESGQGYENLNLVVVHMGGGVSVGAHNHGKVVDVNNALDGDGPFSPERAGSVPIGDLVKMCFSGKYSEAEVYGKVVGKGGFVGYLNTNDVKGVIDNMESGDKECESIYKAFVYQISKAIGEMSVVLEGKVDQIIFTGGIAYSPTLVPDLKEKVEWIAPVTVYPGEDELLALAQGAIRVLDGEEQAKVY

SEQ ID NO: 94 - protein, 355 aa, Clostridium beijerinckii
  MISC_FEATURE: Buk, WP_041893502
MSYKLLIINPGSTSTKIGVYEGEKELFEETLRHTNEEIKRYDTIYDQFEFRKEVILNVLKEKNFDIKTLSAIVGRGGMLRPVEGGTYAVNDAMVEDLKVGVQGPHASNLGGIIAKSIGDELSIPSFIVDPVVTDELADVARLSGVPELPRKSKFHALNQKAVAKRYGKESGQGYENLNLVVVHMGGGVSVGAHNHGKVVDVNNALDGDGPFSPERAGSVPIGDLVKMCFSGKYSEAEVYGKVVGKGGFVGYLNTNDVKGVIDKMEEGDKECGSIYKAFVYQISKAIGEMSVVLEGKVDQIIFTGGIAYSPTLVPDLKAKVEWIAPVTVYPGEDELLALAQGAIRVLDGEEQAKVY

SEQ ID NO: 95 - DNA, 40 bp, Artificial sequence
  Synthetic polynucleotide
  misc_feature: pACYCDuet-ptb-buk - pACYC-ptb-R1, reverse
aagtttttactcatatgtatatctccttcttatacttaac

SEQ ID NO: 96 - DNA, 40 bp, Artificial sequence
  Synthetic polynucleotide
  misc_feature: pACYCDuet-ptb-buk - ptb-pACYC-F1, forward
agaaggagatatacatatgagtaaaaactttgatgagtta

SEQ ID NO: 97 - DNA, 38 bp, Artificial sequence
  Synthetic polynucleotide
  misc_feature: pACYCDuet-ptb-buk - buk-pACYC-R1, reverse
accagactcgagggtacctagtaaaccttagcttgttc

SEQ ID NO: 98 - DNA, 38 bp, Artificial sequence
  Synthetic polynucleotide
  misc_feature: pACYCDuet-ptb-buk - pACYC-buk-F1, forward
taaggtttactaggtaccctcgagtctggtaaagaaac

SEQ ID NO: 99 - DNA, 45 bp, Artificial sequence
  Synthetic polynucleotide
  misc_feature: pCOLADuet-thlA-adc - thlA-adc-R1, reverse
acatatgtatatctccttcttactagcacttttctagcaatattg

SEQ ID NO: 100 - DNA, 45 bp, Artificial sequence
  Synthetic polynucleotide
  misc_feature: pCOLADuet-thlA-adc - adc-ThlA-F1, forward
agtaagaaggagatatacatatgttagaaagtgaagtatctaaac

SEQ ID NO: 101 - DNA, 43 bp, Artificial sequence
  Synthetic polynucleotide
  misc_feature: pCOLADuet-thlA-adc - adc-pCOLA-R1, reverse
cagactcgagggtaccttattttactgaaagataatcatgtac

SEQ ID NO: 102 - DNA, 42 bp, Artificial sequence
  Synthetic polynucleotide
  misc_feature: pCOLADuet-thlA-adc - pCOLA-adc-F1, forward
tctttcagtaaaataaggtaccctcgagtctggtaaagaaac

SEQ ID NO: 103 - DNA, 40 bp, Artificial sequence
  Synthetic polynucleotide
  misc_feature: pCOLADuet-thlA-adc - thlA-pCOLA-F1, forward
gaaggagatatacatatgaaagaagttgtaatagctagtg

SEQ ID NO: 104 - DNA, 40 bp, Artificial sequence
  Synthetic polynucleotide
  misc_feature: pCOLADuet-thlA-adc - pCOLA-thlA-R1, reverse
acaacttctttcatatgtatatctccttcttatacttaac

SEQ ID NO: 105 - DNA, 5791 bp, Artificial sequence
  Synthetic polynucleotide
  misc_feature: pACYC-ptb-buk, plasmid
ggggaattgtgagcggataacaattcccctgtagaaataattttgtttaactttaataaggagatataccatgggcagcagccatcaccatcatcaccacagccaggatccgaattcgagctcggcgcgcctgcaggtcgacaagcttgcggccgcataatgcttaagtcgaacagaaagtaatcgtattgtacacggccgcataatcgaaattaatacgactcactataggggaattgtgagcggataacaattccccatcttagtatattagttaagtataagaaggagatatacatatgagtaaaaactttgatgagttattatcaagattaaaggaagttccaacaaaaaaagtggctgtagccgtagcacaagatgaaccagtattagaggctataaaagaagctacagaaaataacatcgcacaagcaatattggttggtgataaacaacaaatccatgaaatcgcaaagaaaataaacttggacttatctgattatgaaataatggatattaaagatccaaagaaagcaacattagaagcagtaaaattagtttctagtggtcatgcagatatgttaatgaaaggtctagttgatactgcaacattcctaagaagcgtattaaacaaagaggttggtcttagaacaggaaaattaatgtcccatgtagctgtgtttgatgtggaaggttgggatagactgttatttttaactgatgcagcatttaatacatatccagaatttaaggataaagttggaatgataaataatgcagttgtagttgctcatgcatgtggaatagatgttccaagagtagcacctatatgcccagttgaagttgtaaatacaagtatgcaatcaacagttgatgcagcattgttagctaaaatgagtgacagggggcaaattaaaggatgcgtaattgatggaccttttgccttagataatgcaatatcagaagaagcagctcatcataaaggtgttacaggatcagtagcaggtaaagctgatatattattattaccaaatatagaagcagcaaatgtaatgtataaaacattaacatatttctctaaatcaagaaatggtggacttttagtaggtacatcagcaccagtaattttaacttcaagagcagattcattcgaaactaaagttaattcaattgctcttgcagcattagttgcagcaagaaataagtaataaatcaatccataataattaatgcataattaatggagagatttatatggaatttgcaatgcactattagattctataataatttcttctgaaaattatgcattatgactgtatagaatgcattaaatttaagggggattcagaatgtcatataagctattaataatcaatccaggttcaacatcaacaaagattggtgtttacgaaggagaaaaggaactatttgaagaaactttgagacacacaaatgaagaaataaagagatatgatacaatatatgatcaatttgaatttagaaaagaagttatattaaatgttcttaaagaaaagaattttgatataaagactctaagtgctattgttggtagaggtggaatgcttagaccagttgaaggtggaacatatgcagtaaatgatgcaatggttgaagatttaaaagttggagttcaaggacctcatgcttctaaccttggcggaataattgccaagtcaattggagatgaattaaatattccatcatttatagtagatccagttgttacagatgagttagcagatgtagcaagactatctggagtaccagaactaccaagaaaaagtaaattccatgctttaaatcaaaaagcggtagctaaaagatatggaaaagaaagtggacaaggatatgaaaacctaaatcttgtagttgtacatatgggtggaggcgtttcagttggtgctcacaatcatgggaaagttgtcgatgtaaataatgcattagatggagatggcccattctcaccagaaagagctggatcagttccaattggtgatttagttaaaatgtgttttagtggaaaatatagtgaagcagaagtatatggcaaggctgtaggaaaaggtggatttgttggttatctaaacacaaatgatgtaaaaggtgttattgataagatggaagaaggagataaagaatgtgaatcaatatacaaagcatttgtttatcaaatttcaaaagcaatcggagaaatgtcagttgtattagaaggtaaagttgatcaaattatttttaccggaggaattgcatactcaccaacacttgttccagaccttaaagcaaaagttgaatggatagccccagttacagtttatcctggagaagatgaattacttgctctagctcaaggtgctataagagtacttgatggagaagaacaagctaaggtttactaggtaccctcgagtctggtaaagaaaccgctgctgcgaaatttgaacgccagcacatggactcgtctactagcgcagcttaattaacctaggctgctgccaccgctgagcaataactagcataaccccttggggcctctaaacgggtcttgaggggttttttgctgaaacctcaggcatttgagaagcacacggtcacactgcttccggtagtcaataaaccggtaaaccagcaatagacataagcggctatttaacgaccctgccctgaaccgacgacaagctgacgaccgggtctccgcaagtggcacttttcggggaaatgtgcgcggaacccctatttgtttatttttctaaatacattcaaatatgtatccgctcatgaattaattcttagaaaaactcatcgagcatcaaatgaaactgcaatttattcatatcaggattatcaataccatatttttgaaaaagccgtttctgtaatgaaggagaaaactcaccgaggcagttccataggatggcaagatcctggtatcggtctgcgattccgactcgtccaacatcaatacaacctattaatttcccctcgtcaaaaataaggttatcaagtgagaaatcaccatgagtgacgactgaatccggtgagaatggcaaaagtttatgcatttctttccagacttgttcaacaggccagccattacgctcgtcatcaaaatcactcgcatcaaccaaaccgttattcattcgtgattgcgcctgagcgagacgaaatacgcggtcgctgttaaaaggacaattacaaacaggaatcgaatgcaaccggcgcaggaacactgccagcgcatcaacaatattttcacctgaatcaggatattcttctaatacctggaatgctgttttcccggggatcgcagtggtgagtaaccatgcatcatcaggagtacggataaaatgcttgatggtcggaagaggcataaattccgtcagccagtttagtctgaccatctcatctgtaacatcattggcaacgctacctttgccatgtttcagaaacaactctggcgcatcgggcttcccatacaatcgatagattgtcgcacctgattgcccgacattatcgcgagcccatttatacccatataaatcagcatccatgttggaatttaatcgcggcctagagcaagacgtttcccgttgaatatggctcatactcttcctttttcaatattattgaagcatttatcagggttattgtctcatgagcggatacatatttgaatgtatttagaaaaataaacaaataggcatgctagcgcagaaacgtcctagaagatgccaggaggatacttagcagagagacaataaggccggagcgaagccgtttttccataggctccgcccccctgacgaacatcacgaaatctgacgctcaaatcagtggtggcgaaacccgacaggactataaagataccaggcgtttccccctgatggctccctcttgcgctctcctgttcccgtcctgcggcgtccgtgttgtggtggaggctttacccaaatcaccacgtcccgttccgtgtagacagttcgctccaagctgggctgtgtgcaagaaccccccgttcagcccgactgctgcgccttatccggtaactatcatcttgagtccaacccggaaagacacgacaaaacgccactggcagcagccattggtaactgagaattagtggatttagatatcgagagtcttgaagtggtggcctaacagaggctacactgaaaggacagtatttggtatctgcgctccactaaagccagttaccaggttaagcagttccccaactgacttaaccttcgatcaaaccgcctccccaggcggttttttcgtttacagagcaggagattacgacgatcgtaaaaggatctcaagaagatcctttacggattcccgacaccatcactctagatttcagtgcaatttatctcttcaaatgtagcacctgaagtcagccccatacgatataagttgtaattctcatgttagtcatgccccgcgcccaccggaaggagctgactgggttgaaggctctcaagggcatcggtcgagatcccggtgcctaatgagtgagctaacttacattaattgcgttgcgctcactgcccgctttccagtcgggaaacctgtcgtgccagctgcattaatgaatcggccaacgcgcggggagaggcggtttgcgtattgggcgccagggtggtttttcttttcaccagtgagacgggcaacagctgattgcccttcaccgcctggccctgagagagttgcagcaagcggtccacgctggtttgccccagcaggcgaaaatcctgtttgatggtggttaacggcgggatataacatgagctgtcttcggtatcgtcgtatcccactaccgagatgtccgcaccaacgcgcagcccggactcggtaatggcgcgcattgcgcccagcgccatctgatcgttggcaaccagcatcgcagtgggaacgatgccctcattcagcatttgcatggtttgttgaaaaccggacatggcactccagtcgccttcccgttccgctatcggctgaatttgattgcgagtgagatatttatgccagccagccagacgcagacgcgccgagacagaacttaatgggcccgctaacagcgcgatttgctggtgacccaatgcgaccagatgctccacgcccagtcgcgtaccgtcttcatgggagaaaataatactgttgatgggtgtctggtcagagacatcaagaaataacgccggaacattagtgcaggcagcttccacagcaatggcatcctggtcatccagcggatagttaatgatcagcccactgacgcgttgcgcgagaagattgtgcaccgccgctttacaggcttcgacgccgcttcgttctaccatcgacaccaccacgctggcacccagttgatcggcgcgagatttaatcgccgcgacaatttgcgacggcgcgtgcagggccagactggaggtggcaacgccaatcagcaacgactgtttgcccgccagttgttgtgccacgcggttgggaatgtaattcagctccgccatcgccgcttccactttttcccgcgttttcgcagaaacgtggctggcctggttcaccacgcgggaaacggtctgataagagacaccggcatactctgcgacatcgtataacgttactggtttcacattcaccaccctgaattgactctcttccgggcgctatcatgccataccgcgaaaggttttgcgccattcgatggtgtccgggatctcgacgctctcccttatgcgactcctgcattaggaaattaatacgactcactata

SEQ ID NO: 106 - DNA, 5609 bp, Artificial sequence
  Synthetic polynucleotide
  misc_feature: pCOLA-thlA-adc, plasmid
ggggaattgtgagcggataacaattcccctgtagaaataattttgtttaactttaataaggagatataccatgggcagcagccatcaccatcatcaccacagccaggatccgaattcgagctcggcgcgcctgcaggtcgacaagcttgcggccgcataatgcttaagtcgaacagaaagtaatcgtattgtacacggccgcataatcgaaattaatacgactcactataggggaattgtgagcggataacaattccccatcttagtatattagttaagtataagaaggagatatacatatgaaagaagttgtaatagctagtgcagtaagaacagcgattggatcttatggaaagtctcttaaggatgtaccagcagtagatttaggagctacagctataaaggaagcagttaaaaaagcaggaataaaaccagaggatgttaatgaagtcattttaggaaatgttcttcaagcaggtttaggacagaatccagcaagacaggcatcttttaaagcaggattaccagttgaaattccagctatgactattaataaggtttgtggttcaggacttagaacagttagcttagcagcacaaattataaaagcaggagatgctgacgtaataatagcaggtggtatggaaaatatgtctagagctccttacttagcgaataacgctagatggggatatagaatgggaaacgctaaatttgttgatgaaatgatcactgacggattgtgggatgcatttaatgattaccacatgggaataacagcagaaaacatagctgagagatggaacatttcaagagaagaacaagatgagtttgctcttgcatcacaaaaaaaagctgaagaagctataaaatcaggtcaatttaaagatgaaatagttcctgtagtaattaaaggcagaaagggagaaactgtagttgatacagatgagcaccctagatttggatcaactatagaaggacttgcaaaattaaaacctgccttcaaaaaagatggaacagttacagctggtaatgcatcaggattaaatgactgtgcagcagtacttgtaatcatgagtgcagaaaaagctaaagagcttggagtaaaaccacttgctaagatagtttcttatggttcagcaggagttgacccagcaataatgggatatggacctttctatgcaacaaaagcagctattgaaaaagcaggttggacagttgatgaattagatttaatagaatcaaatgaagcttttgcagctcaaagtttagcagtagcaaaagatttaaaatttgatatgaataaagtaaatgtaaatggaggagctattgcccttggtcatccaattggagcatcaggtgcaagaatactcgttactcttgtacacgcaatgcaaaaaagagatgcaaaaaaaggcttagcaactttatgtataggtggcggacaaggaacagcaatattgctagaaaagtgctagtaagaaggagatatacatatgttagaaagtgaagtatctaaacaaattacaactccacttgctgctccagcgtttcctagaggaccatataggtttcacaatagagaatatctaaacattatttatcgaactgatttagatgctcttcgaaaaatagtaccagagccacttgaattagatagagcatatgttagatttgaaatgatggctatgcctgatacaaccggactaggctcatatacagaatgtggtcaagctattccagtaaaatataatggtgttaagggtgactacttgcatatgatgtatctagataatgaacctgctattgctgttggaagagaaagtagcgcttatccaaaaaagcttggctatccaaagctatttgttgattcagatactttagttgggacacttaaatatggtacattaccagtagctactgcaacaatgggatataagcacgagcctctagatcttaaagaagcctatgctcaaattgcaagacccaattttatgctaaaaatcattcaaggttacgatggtaagccaagaatttgtgaactaatatgtgcagaaaatactgatataactattcacggtgcttggactggaagtgcacgtctacaattatttagccatgcactagctcctcttgctgatttacctgtattagagattgtatcagcatctcatatcctcacagatttaactcttggaacacctaaggttgtacatgattatctttcagtaaaataaggtaccctcgagtctggtaaagaaaccgctgctgcgaaatttgaacgccagcacatggactcgtctactagcgcagcttaattaacctaggctgctgccaccgctgagcaataactagcataaccccttggggcctctaaacgggtcttgaggggttttttgctgaaacctcaggcatttgagaagcacacggtcacactgcttccggtagtcaataaaccggtaaaccagcaatagacataagcggctatttaacgaccctgccctgaaccgacgacaagctgacgaccgggtctccgcaagtggcacttttcggggaaatgtgcgcggaacccctatttgtttatttttctaaatacattcaaatatgtatccgctcatgaattaattcttagaaaaactcatcgagcatcaaatgaaactgcaatttattcatatcaggattatcaataccatatttttgaaaaagccgtttctgtaatgaaggagaaaactcaccgaggcagttccataggatggcaagatcctggtatcggtctgcgattccgactcgtccaacatcaatacaacctattaatttcccctcgtcaaaaataaggttatcaagtgagaaatcaccatgagtgacgactgaatccggtgagaatggcaaaagtttatgcatttctttccagacttgttcaacaggccagccattacgctcgtcatcaaaatcactcgcatcaaccaaaccgttattcattcgtgattgcgcctgagcgagacgaaatacgcggtcgctgttaaaaggacaattacaaacaggaatcgaatgcaaccggcgcaggaacactgccagcgcatcaacaatattttcacctgaatcaggatattcttctaatacctggaatgctgttttcccggggatcgcagtggtgagtaaccatgcatcatcaggagtacggataaaatgcttgatggtcggaagaggcataaattccgtcagccagtttagtctgaccatctcatctgtaacatcattggcaacgctacctttgccatgtttcagaaacaactctggcgcatcgggcttcccatacaatcgatagattgtcgcacctgattgcccgacattatcgcgagcccatttatacccatataaatcagcatccatgttggaatttaatcgcggcctagagcaagacgtttcccgttgaatatggctcatactcttcctttttcaatattattgaagcatttatcagggttattgtctcatgagcggatacatatttgaatgtatttagaaaaataaacaaataggcatgctagcgcagaaacgtcctagaagatgccaggaggatacttagcagagagacaataaggccggagcgaagccgtttttccataggctccgcccccctgacgaacatcacgaaatctgacgctcaaatcagtggtggcgaaacccgacaggactataaagataccaggcgtttccccctgatggctccctcttgcgctctcctgttcccgtcctgcggcgtccgtgttgtggtggaggctttacccaaatcaccacgtcccgttccgtgtagacagttcgctccaagctgggctgtgtgcaagaaccccccgttcagcccgactgctgcgccttatccggtaactatcatcttgagtccaacccggaaagacacgacaaaacgccactggcagcagccattggtaactgagaattagtggatttagatatcgagagtcttgaagtggtggcctaacagaggctacactgaaaggacagtatttggtatctgcgctccactaaagccagttaccaggttaagcagttccccaactgacttaaccttcgatcaaaccgcctccccaggcggttttttcgtttacagagcaggagattacgacgatcgtaaaaggatctcaagaagatcctttacggattcccgacaccatcactctagatttcagtgcaatttatctcttcaaatgtagcacctgaagtcagccccatacgatataagttgtaattctcatgttagtcatgccccgcgcccaccggaaggagctgactgggttgaaggctctcaagggcatcggtcgagatcccggtgcctaatgagtgagctaacttacattaattgcgttgcgctcactgcccgctttccagtcgggaaacctgtcgtgccagctgcattaatgaatcggccaacgcgcggggagaggcggtttgcgtattgggcgccagggtggtttttcttttcaccagtgagacgggcaacagctgattgcccttcaccgcctggccctgagagagttgcagcaagcggtccacgctggtttgccccagcaggcgaaaatcctgtttgatggtggttaacggcgggatataacatgagctgtcttcggtatcgtcgtatcccactaccgagatgtccgcaccaacgcgcagcccggactcggtaatggcgcgcattgcgcccagcgccatctgatcgttggcaaccagcatcgcagtgggaacgatgccctcattcagcatttgcatggtttgttgaaaaccggacatggcactccagtcgccttcccgttccgctatcggctgaatttgattgcgagtgagatatttatgccagccagccagacgcagacgcgccgagacagaacttaatgggcccgctaacagcgcgatttgctggtgacccaatgcgaccagatgctccacgcccagtcgcgtaccgtcttcatgggagaaaataatactgttgatgggtgtctggtcagagacatcaagaaataacgccggaacattagtgcaggcagcttccacagcaatggcatcctggtcatccagcggatagttaatgatcagcccactgacgcgttgcgcgagaagattgtgcaccgccgctttacaggcttcgacgccgcttcgttctaccatcgacaccaccacgctggcacccagttgatcggcgcgagatttaatcgccgcgacaatttgcgacggcgcgtgcagggccagactggaggtggcaacgccaatcagcaacgactgtttgcccgccagttgttgtgccacgcggttgggaatgtaattcagctccgccatcgccgcttccactttttcccgcgttttcgcagaaacgtggctggcctggttcaccacgcgggaaacggtctgataagagacaccggcatactctgcgacatcgtataacgttactggtttcacattcaccaccctgaattgactctcttccgggcgctatcatgccataccgcgaaaggttttgcgccattcgatggtgtccgggatctcgacgctctcccttatgcgactcctgcattaggaaattaatacgactcactata

SEQ ID NO: 107 - DNA, 36 bp, Artificial sequence
  Synthetic polynucleotide
  misc_feature: thlA-ptb-R1, reverse
atttcctccctttctagcacttttctagcaatattg

SEQ ID NO: 108 - DNA, 36 bp, Artificial sequence
  Synthetic polynucleotide
  misc_feature: adc-buk-F1, forward
taaggtttactaaggaggttgttttatgttagaaag

SEQ ID NO: 109 - DNA, 36 bp, Artificial sequence
  Synthetic polynucleotide
  misc_feature: thlA-ptb-F1, forward
gctagaaaagtgctagaaagggaggaaatgaacatg

SEQ ID NO: 110 - DNA, 36 bp, Artificial sequence
  Synthetic polynucleotide
  misc_feature: Buk-adc-R1, reverse
aaaacaacctccttagtaaaccttagcttgttcttc

SEQ ID NO: 111 - DNA, 29 bp, Artificial sequence
  Synthetic polynucleotide
  misc_feature: pDuet-insert2-R1, forward
catatgtatatctccttcttatacttaac

SEQ ID NO: 112 - DNA, 29 bp, Artificial sequence
  Synthetic polynucleotide
  misc_feature: insert2-pDuet-F1, forward
gttaagtataagaaggagatatacatatg

SEQ ID NO: 113 - DNA, 21 bp, Artificial sequence
  Synthetic polynucleotide
  misc_feature: pDuet-insert2-F1, forward
cctcgagtctggtaaagaaac

SEQ ID NO: 114 - DNA, 21 bp, Artificial sequence
  Synthetic polynucleotide
  misc_feature: insert2-pDuet-R1, forward
gtttctttaccagactcgagg

SEQ ID NO: 115 - DNA, 36 bp, Artificial sequence
  Synthetic polynucleotide
  misc_feature: pCDF-phaB - pACYC-phaB-R1, forward
ctattctttgtgtcatggtatatctccttattaaag

SEQ ID NO: 116 - DNA, 36 bp, Artificial sequence
  Synthetic polynucleotide
  misc_feature: pCDF-phaB - phaB-pACYC-F1, forward
ataaggagatataccatgacacaaagaatagcatac

SEQ ID NO: 117 - DNA, 36 bp, Artificial sequence
  Synthetic polynucleotide
  misc_feature: pcdf-phab - pacyc-phab-f1, forward
tggtttacacatgggataagatccgaattcgagctc

SEQ ID NO: 118 - DNA, 36 bp, Artificial sequence
  Synthetic polynucleotide
  misc_feature: pCDF-phaB - phaB-pACYC-R1, forward
agctcgaattcggatcttatcccatgtgtaaaccac

SEQ ID NO: 119 - DNA, 4486 bp, Artificial sequence
  Synthetic polynucleotide
  misc_feature: pCDF-phaB, plasmid
ggggaattgtgagcggataacaattcccctgtagaaataattttgtttaactttaataaggagatataccatgacacaaagaatagcatacgtaacaggtggtatgggtggtataggaactgcaatatgtcaaagattagcaaaagatggatttagagttgtagctggatgcggaccaaatagtcctagaagagaaaagtggttagaacaacaaaaagcacttggatttgatttcatagcttctgaaggtaacgtagcagattgggactcaactaaaactgcttttgataaagttaaatctgaagttggtgaagttgatgtattaataaataatgcaggtattactagagatgtagtatttagaaagatgacaagagctgactgggatgcagtaatagatactaatcttactagtcttttcaatgtaactaagcaggtaattgatggtatggcagatagaggttggggtagaatagtaaatattagttcagttaatggacaaaaaggtcagtttggacagacaaattattctacagctaaagcaggtcttcatggttttacaatggctttagcacaggaagttgctacaaaaggtgttacagttaacactgttagtccaggatatattgctactgacatggtaaaggctataagacaagatgttcttgataaaattgttgctacaataccagtaaagagattaggacttcctgaagagatagcatctatttgtgcatggttatcaagtgaagaatcaggattctcaactggtgctgatttttcattaaacggtggtttacacatgggataagatccgaattcgagctcggcgcgcctgcaggtcgacaagcttgcggccgcataatgcttaagtcgaacagaaagtaatcgtattgtacacggccgcataatcgaaattaatacgactcactataggggaattgtgagcggataacaattccccatcttagtatattagttaagtataagaaggagatatacatatggcagatctcaattggatatcggccggccacgcgatcgctgacgtcggtaccctcgagtctggtaaagaaaccgctgctgcgaaatttgaacgccagcacatggactcgtctactagcgcagcttaattaacctaggctgctgccaccgctgagcaataactagcataaccccttggggcctctaaacgggtcttgaggggttttttgctgaaacctcaggcatttgagaagcacacggtcacactgcttccggtagtcaataaaccggtaaaccagcaatagacataagcggctatttaacgaccctgccctgaaccgacgaccgggtcatcgtggccggatcttgcggcccctcggcttgaacgaattgttagacattatttgccgactaccttggtgatctcgcctttcacgtagtggacaaattcttccaactgatctgcgcgcgaggccaagcgatcttcttcttgtccaagataagcctgtctagcttcaagtatgacgggctgatactgggccggcaggcgctccattgcccagtcggcagcgacatccttcggcgcgattttgccggttactgcgctgtaccaaatgcgggacaacgtaagcactacatttcgctcatcgccagcccagtcgggcggcgagttccatagcgttaaggtttcatttagcgcctcaaatagatcctgttcaggaaccggatcaaagagttcctccgccgctggacctaccaaggcaacgctatgttctcttgcttttgtcagcaagatagccagatcaatgtcgatcgtggctggctcgaagatacctgcaagaatgtcattgcgctgccattctccaaattgcagttcgcgcttagctggataacgccacggaatgatgtcgtcgtgcacaacaatggtgacttctacagcgcggagaatctcgctctctccaggggaagccgaagtttccaaaaggtcgttgatcaaagctcgccgcgttgtttcatcaagccttacggtcaccgtaaccagcaaatcaatatcactgtgtggcttcaggccgccatccactgcggagccgtacaaatgtacggccagcaacgtcggttcgagatggcgctcgatgacgccaactacctctgatagttgagtcgatacttcggcgatcaccgcttccctcatactcttcctttttcaatattattgaagcatttatcagggttattgtctcatgagcggatacatatttgaatgtatttagaaaaataaacaaatagctagctcactcggtcgctacgctccgggcgtgagactgcggcgggcgctgcggacacatacaaagttacccacagattccgtggataagcaggggactaacatgtgaggcaaaacagcagggccgcgccggtggcgtttttccataggctccgccctcctgccagagttcacataaacagacgcttttccggtgcatctgtgggagccgtgaggctcaaccatgaatctgacagtacgggcgaaacccgacaggacttaaagatccccaccgtttccggcgggtcgctccctcttgcgctctcctgttccgaccctgccgtttaccggatacctgttccgcctttctcccttacgggaagtgtggcgctttctcatagctcacacactggtatctcggctcggtgtaggtcgttcgctccaagctgggctgtaagcaagaactccccgttcagcccgactgctgcgccttatccggtaactgttcacttgagtccaacccggaaaagcacggtaaaacgccactggcagcagccattggtaactgggagttcgcagaggatttgtttagctaaacacgcggttgctcttgaagtgtgcgccaaagtccggctacactggaaggacagatttggttgctgtgctctgcgaaagccagttaccacggttaagcagttccccaactgacttaaccttcgatcaaaccacctccccaggtggttttttcgtttacagggcaaaagattacgcgcagaaaaaaaggatctcaagaagatcctttgatcttttctactgaaccgctctagatttcagtgcaatttatctcttcaaatgtagcacctgaagtcagccccatacgatataagttgtaattctcatgttagtcatgccccgcgcccaccggaaggagctgactgggttgaaggctctcaagggcatcggtcgagatcccggtgcctaatgagtgagctaacttacattaattgcgttgcgctcactgcccgctttccagtcgggaaacctgtcgtgccagctgcattaatgaatcggccaacgcgcggggagaggcggtttgcgtattgggcgccagggtggtttttcttttcaccagtgagacgggcaacagctgattgcccttcaccgcctggccctgagagagttgcagcaagcggtccacgctggtttgccccagcaggcgaaaatcctgtttgatggtggttaacggcgggatataacatgagctgtcttcggtatcgtcgtatcccactaccgagatgtccgcaccaacgcgcagcccggactcggtaatggcgcgcattgcgcccagcgccatctgatcgttggcaaccagcatcgcagtgggaacgatgccctcattcagcatttgcatggtttgttgaaaaccggacatggcactccagtcgccttcccgttccgctatcggctgaatttgattgcgagtgagatatttatgccagccagccagacgcagacgcgccgagacagaacttaatgggcccgctaacagcgcgatttgctggtgacccaatgcgaccagatgctccacgcccagtcgcgtaccgtcttcatgggagaaaataatactgttgatgggtgtctggtcagagacatcaagaaataacgccggaacattagtgcaggcagcttccacagcaatggcatcctggtcatccagcggatagttaatgatcagcccactgacgcgttgcgcgagaagattgtgcaccgccgctttacaggcttcgacgccgcttcgttctaccatcgacaccaccacgctggcacccagttgatcggcgcgagatttaatcgccgcgacaatttgcgacggcgcgtgcagggccagactggaggtggcaacgccaatcagcaacgactgtttgcccgccagttgttgtgccacgcggttgggaatgtaattcagctccgccatcgccgcttccactttttcccgcgttttcgcagaaacgtggctggcctggttcaccacgcgggaaacggtctgataagagacaccggcatactctgcgacatcgtataacgttactggtttcacattcaccaccctgaattgactctcttccgggcgctatcatgccataccgcgaaaggttttgcgccattcgatggtgtccgggatctcgacgctctcccttatgcgactcctgcattaggaaattaatacgactcactata

SEQ ID NO: 120 - DNA, 5221 bp, Artificial sequence
  Synthetic polynucleotide
  misc_feature: pCDF-phaB-bdh1, plasmid
ggggaattgtgagcggataacaattcccctgtagaaataattttgtttaactttaataaggagatataccatgacacaaagaatagcatacgtaacaggtggtatgggtggtataggaactgcaatatgtcaaagattagcaaaagatggatttagagttgtagctggatgcggaccaaatagtcctagaagagaaaagtggttagaacaacaaaaagcacttggatttgatttcatagcttctgaaggtaacgtagcagattgggactcaactaaaactgcttttgataaagttaaatctgaagttggtgaagttgatgtattaataaataatgcaggtattactagagatgtagtatttagaaagatgacaagagctgactgggatgcagtaatagatactaatcttactagtcttttcaatgtaactaagcaggtaattgatggtatggcagatagaggttggggtagaatagtaaatattagttcagttaatggacaaaaaggtcagtttggacagacaaattattctacagctaaagcaggtcttcatggttttacaatggctttagcacaggaagttgctacaaaaggtgttacagttaacactgttagtccaggatatattgctactgacatggtaaaggctataagacaagatgttcttgataaaattgttgctacaataccagtaaagagattaggacttcctgaagagatagcatctatttgtgcatggttatcaagtgaagaatcaggattctcaactggtgctgatttttcattaaacggtggtttacacatgggataagatccgaattcgagctcggcgcgcctgcaggtcgacaagcttgcggccgcataatgcttaagtcgaacagaaagtaatcgtattgtacacggccgcataatcgaaattaatacgactcactataggggaattgtgagcggataacaattccccatcttagtatattagttaagtataagaaggagatatacatatgcaattaaaaggtaaaagtgcaatagtaactggtgcagcaagtggaataggaaaagcaatagcagaattacttgcaaaagaaggtgcagcagtagcaatagctgatttaaatttagaagcagcaagagcagcagcagctggaatagaagcagctggcggaaaagctatagctgtagcaatggatgtaactagtgaagcaagtgtaaatcaagcaactgatgaagtagcacaagcatttggaaatatagatatattagtaagtaatgctggaatacaaatagtaaatcctatacaaaattatgcatttagtgattggaaaaaaatgcaagcaatacatgtagatggtgcatttttaactactaaagcagcattgaaatatatgtatagagataaaagaggtggaactgtaatatatatgggaagtgtacattctcatgaagcaagtcctttaaaaagtgcttatgtagcagcaaaacatgcattattaggattagcaagagtattagctaaagaaggtgctgaattcaacgtaagatctcacgttatatgtcctggatttgtaagaactcctttagtagataaacaaatacctgaacaagcaaaagaattaggaataagtgaagaagaagtagttagaagagtaatgttaggtggaacagtagacggtgtatttactactgtagatgatgtagcaagaactgcattatttttatgtgcatttcctagtgcagcattaactggacaaagttttatagtaagtcatggatggtatatgcaataaggtaccctcgagtctggtaaagaaaccgctgctgcgaaatttgaacgccagcacatggactcgtctactagcgcagcttaattaacctaggctgctgccaccgctgagcaataactagcataaccccttggggcctctaaacgggtcttgaggggttttttgctgaaacctcaggcatttgagaagcacacggtcacactgcttccggtagtcaataaaccggtaaaccagcaatagacataagcggctatttaacgaccctgccctgaaccgacgaccgggtcatcgtggccggatcttgcggcccctcggcttgaacgaattgttagacattatttgccgactaccttggtgatctcgcctttcacgtagtggacaaattcttccaactgatctgcgcgcgaggccaagcgatcttcttcttgtccaagataagcctgtctagcttcaagtatgacgggctgatactgggccggcaggcgctccattgcccagtcggcagcgacatccttcggcgcgattttgccggttactgcgctgtaccaaatgcgggacaacgtaagcactacatttcgctcatcgccagcccagtcgggcggcgagttccatagcgttaaggtttcatttagcgcctcaaatagatcctgttcaggaaccggatcaaagagttcctccgccgctggacctaccaaggcaacgctatgttctcttgcttttgtcagcaagatagccagatcaatgtcgatcgtggctggctcgaagatacctgcaagaatgtcattgcgctgccattctccaaattgcagttcgcgcttagctggataacgccacggaatgatgtcgtcgtgcacaacaatggtgacttctacagcgcggagaatctcgctctctccaggggaagccgaagtttccaaaaggtcgttgatcaaagctcgccgcgttgtttcatcaagccttacggtcaccgtaaccagcaaatcaatatcactgtgtggcttcaggccgccatccactgcggagccgtacaaatgtacggccagcaacgtcggttcgagatggcgctcgatgacgccaactacctctgatagttgagtcgatacttcggcgatcaccgcttccctcatactcttcctttttcaatattattgaagcatttatcagggttattgtctcatgagcggatacatatttgaatgtatttagaaaaataaacaaatagctagctcactcggtcgctacgctccgggcgtgagactgcggcgggcgctgcggacacatacaaagttacccacagattccgtggataagcaggggactaacatgtgaggcaaaacagcagggccgcgccggtggcgtttttccataggctccgccctcctgccagagttcacataaacagacgcttttccggtgcatctgtgggagccgtgaggctcaaccatgaatctgacagtacgggcgaaacccgacaggacttaaagatccccaccgtttccggcgggtcgctccctcttgcgctctcctgttccgaccctgccgtttaccggatacctgttccgcctttctcccttacgggaagtgtggcgctttctcatagctcacacactggtatctcggctcggtgtaggtcgttcgctccaagctgggctgtaagcaagaactccccgttcagcccgactgctgcgccttatccggtaactgttcacttgagtccaacccggaaaagcacggtaaaacgccactggcagcagccattggtaactgggagttcgcagaggatttgtttagctaaacacgcggttgctcttgaagtgtgcgccaaagtccggctacactggaaggacagatttggttgctgtgctctgcgaaagccagttaccacggttaagcagttccccaactgacttaaccttcgatcaaaccacctccccaggtggttttttcgtttacagggcaaaagattacgcgcagaaaaaaaggatctcaagaagatcctttgatcttttctactgaaccgctctagatttcagtgcaatttatctcttcaaatgtagcacctgaagtcagccccatacgatataagttgtaattctcatgttagtcatgccccgcgcccaccggaaggagctgactgggttgaaggctctcaagggcatcggtcgagatcccggtgcctaatgagtgagctaacttacattaattgcgttgcgctcactgcccgctttccagtcgggaaacctgtcgtgccagctgcattaatgaatcggccaacgcgcggggagaggcggtttgcgtattgggcgccagggtggtttttcttttcaccagtgagacgggcaacagctgattgcccttcaccgcctggccctgagagagttgcagcaagcggtccacgctggtttgccccagcaggcgaaaatcctgtttgatggtggttaacggcgggatataacatgagctgtcttcggtatcgtcgtatcccactaccgagatgtccgcaccaacgcgcagcccggactcggtaatggcgcgcattgcgcccagcgccatctgatcgttggcaaccagcatcgcagtgggaacgatgccctcattcagcatttgcatggtttgttgaaaaccggacatggcactccagtcgccttcccgttccgctatcggctgaatttgattgcgagtgagatatttatgccagccagccagacgcagacgcgccgagacagaacttaatgggcccgctaacagcgcgatttgctggtgacccaatgcgaccagatgctccacgcccagtcgcgtaccgtcttcatgggagaaaataatactgttgatgggtgtctggtcagagacatcaagaaataacgccggaacattagtgcaggcagcttccacagcaatggcatcctggtcatccagcggatagttaatgatcagcccactgacgcgttgcgcgagaagattgtgcaccgccgctttacaggcttcgacgccgcttcgttctaccatcgacaccaccacgctggcacccagttgatcggcgcgagatttaatcgccgcgacaatttgcgacggcgcgtgcagggccagactggaggtggcaacgccaatcagcaacgactgtttgcccgccagttgttgtgccacgcggttgggaatgtaattcagctccgccatcgccgcttccactttttcccgcgttttcgcagaaacgtggctggcctggttcaccacgcgggaaacggtctgataagagacaccggcatactctgcgacatcgtataacgttactggtttcacattcaccaccctgaattgactctcttccgggcgctatcatgccataccgcgaaaggttttgcgccattcgatggtgtccgggatctcgacgctctcccttatgcgactcctgcattaggaaattaatacgactcactata

SEQ ID NO: 121 - DNA, 10922 bp, Artificial sequence
  Synthetic polynucleotide
  misc_feature: pMTL8225-budA::thlA-phaB, plasmid
aaactcctttttgataatctcatgaccaaaatcccttaacgtgagttttcgttccactgagcgtcagaccccgtagaaaagatcaaaggatcttcttgagatcctttttttctgcgcgtaatctgctgcttgcaaacaaaaaaaccaccgctaccagcggtggtttgtttgccggatcaagagctaccaactctttttccgaaggtaactggcttcagcagagcgcagataccaaatactgttcttctagtgtagccgtagttaggccaccacttcaagaactctgtagcaccgcctacatacctcgctctgctaatcctgttaccagtggctgctgccagtggcgataagtcgtgtcttaccgggttggactcaagacgatagttaccggataaggcgcagcggtcgggctgaacggggggttcgtgcacacagcccagcttggagcgaacgacctacaccgaactgagatacctacagcgtgagctatgagaaagcgccacgcttcccgaagggagaaaggcggacaggtatccggtaagcggcagggtcggaacaggagagcgcacgagggagcttccagggggaaacgcctggtatctttatagtcctgtcgggtttcgccacctctgacttgagcgtcgatttttgtgatgctcgtcaggggggcggagcctatggaaaaacgccagcaacgcggcctttttacggttcctggccttttgctggccttttgctcacatgttctttcctgcgttatcccctgattctgtggataaccgtattaccgcctttgagtgagctgataccgctcgccgcagccgaacgaccgagcgcagcgagtcagtgagcgaggaagcggaagagcgcccaatacgcagggccccctgcttcggggtcattatagcgattttttcggtatatccatcctttttcgcacgatatacaggattttgccaaagggttcgtgtagactttccttggtgtatccaacggcgtcagccgggcaggataggtgaagtaggcccacccgcgagcgggtgttccttcttcactgtcccttattcgcacctggcggtgctcaacgggaatcctgctctgcgaggctggccggctaccgccggcgtaacagatgagggcaagcggatggctgatgaaaccaagccaaccaggaagggcagcccacctatcaaggtgtactgccttccagacgaacgaagagcgattgaggaaaaggcggcggcggccggcatgagcctgtcggcctacctgctggccgtcggccagggctacaaaatcacgggcgtcgtggactatgagcacgtccgcgagctggcccgcatcaatggcgacctgggccgcctgggcggcctgctgaaactctggctcaccgacgacccgcgcacggcgcggttcggtgatgccacgatcctcgccctgctggcgaagatcgaagagaagcaggacgagcttggcaaggtcatgatgggcgtggtccgcccgagggcagagccatgacttttttagccgctaaaacggccggggggtgcgcgtgattgccaagcacgtccccatgcgctccatcaagaagagcgacttcgcggagctggtgaagtacatcaccgacgagcaaggcaagaccgatcgggccccctgcaggataaaaaaattgtagataaattttataaaatagttttatctacaatttttttatcaggaaacagctatgaccgcggccgcggcgccaagcttagaaaaatataaataagaagtagctttaagagaattaaattattaagaaaagcaaaggtgtttaaaaaataaatttttaaacacctttgcttttcttaaattataaataagataaaaaagaatcctgaataaaataaaaaggggtgtctcaaaattttattttgagacgacccctttttattctatatgtcgatgctatagctgagatcgtggaattcttgttagctaccagattcacatttaagttgtttctctaaaccacagattatcaattcaagtccaaaaagaaatgctggttctgcgccttgatgatcaaataactctattgcttgtcttaacaatggaggcattgaatctgttgttggtgtttctctttcctcttttgcaacttgatgttcttgatcctccaatacgcaacctaaagtaaaatgtcctacagcacttagtgcgtataaggcattttctaaactaaaaccctgttgacataagaatgctaattgattttctaatgtttcatattgtttttcagttggtctagttcctaaatgtactttagccccatctctatgtgataatagagcacaacgaaaagatttagcgttattcctaagaaaatcttgccatgattcaccttctaaaggacaaaagtgagtgtgatgtctatctaacatttcaatagctaaggcgtcaagtaaagctctcttattcttcacatgccaatacaacgtaggttgttctactccaagtttctgagctaactttcttgtagttagtccttctattccaacttcatttagtaattccaatgcactattgataactttacttttatcaagtctagacatcatttaatatcctcctcttcaatatatttaagtcgactgatcggatcctgatcggagctcccatggcggccggtcgatatcgatgtgtagtagcctgtgaaataagtaaggaaaaaaaagaagtaagtgttatatatgatgattattttgtagatgtagataggataatagaatccatagaaaatataggttatacagttatataaaaattactttaaaatctatcattgatagggtaaaatataaatcgtataaagttgtgtaatttttaaggaggtgtgttacagacgtccgcgagagaccttaaatatattgaagaggaggaaatacatatggtttcaagatatgttccagatatgggagatttaatatgggttgattttgatccaacaaaaggatcagaacaagcaggacatagaccagcagttgttttatcaccatttatgtataataataaaacaggaatgtgtttatgtgttccatgtacaacacaatcaaaaggatatccatttgaagttgttttatcaggacaagaaagagatggagttgcattagcagatcaagttaaatcaatagcatggagagcaagaggagcaacaaaaaaaggaacagttgcaccagaagaattacaattaataaaagcaaaaataaatgttttaataggataatgttattaagctagcataaaaataagaagcctgcatttgcaggcttcttatttttatggcgcgccgttctgaatccttagctaatggttcaacaggtaactatgacgaagatagcaccctggataagtctgtaatggattctaaggcatttaatgaagacgtgtatataaaatgtgctaatgaaaaagaaaatgcgttaaaagagcctaaaatgagttcaaatggttttgaaattgattggtagtttaatttaatatattttttctattggctatctcgatacctatagaatcttctgttcacttttgtttttgaaatataaaaaggggctttttagccccttttttttaaaactccggaggagtttcttcattcttgatactatacgtaactattttcgatttgacttcattgtcaattaagctagtaaaatcaatggttaaaaaacaaaaaacttgcatttttctacctagtaatttataattttaagtgtcgagtttaaaagtataatttaccaggaaaggagcaagttttttaataaggaaaaatttttccttttaaaattctatttcgttatatgactaattataatcaaaaaaatgaaaataaacaagaggtaaaaactgctttagagaaatgtactgataaaaaaagaaaaaatcctagatttacgtcatacatagcacctttaactactaagaaaaatattgaaaggacttccacttgtggagattatttgtttatgttgagtgatgcagacttagaacattttaaattacataaaggtaatttttgcggtaatagattttgtccaatgtgtagttggcgacttgcttgtaaggatagtttagaaatatctattcttatggagcatttaagaaaagaagaaaataaagagtttatatttttaactcttacaactccaaatgtaaaaagttatgatcttaattattctattaaacaatataataaatcttttaaaaaattaatggagcgtaaggaagttaaggatataactaaaggttatataagaaaattagaagtaacttaccaaaaggaaaaatacataacaaaggatttatggaaaataaaaaaagattattatcaaaaaaaaggacttgaaattggtgatttagaacctaattttgatacttataatcctcattttcatgtagttattgcagttaataaaagttattttacagataaaaattattatataaatcgagaaagatggttggaattatggaagtttgctactaaggatgattctataactcaagttgatgttagaaaagcaaaaattaatgattataaagaggtttacgaacttgcgaaatattcagctaaagacactgattatttaatatcgaggccagtatttgaaattttttataaagcattaaaaggcaagcaggtattagtttttagtggattttttaaagatgcacacaaattgtacaagcaaggaaaacttgatgtttataaaaagaaagatgaaattaaatatgtctatatagtttattataattggtgcaaaaaacaatatgaaaaaactagaataagggaacttacggaagatgaaaaagaagaattaaatcaagatttaatagatgaaatagaaatagattaaagtgtaactatactttatatatatatgattaaaaaaataaaaaacaacagcctattaggttgttgttttttattttctttattaatttttttaatttttagtttttagttcttttttaaaataagtttcagcctctttttcaatattttttaaagaaggagtatttgcatgaattgccttttttctaacagacttaggaaatattttaacagtatcttcttgcgccggtgattttggaacttcataacttactaatttataattattattttcttttttaattgtaacagttgcaaaagaagctgaacctgttccttcaactagtttatcatcttcaatataatattcttgacctatatagtataaatatatttttattatatttttacttttttctgaatctattattttataatcataaaaagttttaccaccaaaagaaggttgtactccttctggtccaacatatttttttactatattatctaaataatttttgggaactggtgttgtaatttgattaatcgaacaaccagttatacttaaaggaattataactataaaaatatataggattatctttttaaatttcattattggcctcctttttattaaatttatgttaccataaaaaggacataacgggaatatgtagaatatttttaatgtagacaaaattttacataaatataaagaaaggaagtgtttgtttaaattttatagcaaactatcaaaaattagggggataaaaatttatgaaaaaaaggttttcgatgttatttttatgtttaactttaatagtttgtggtttatttacaaattcggccggcctacctcctcgtataaataagatgtttttgttttgcttgatactactttttcttcacaggaaaatatacttcagtaacaagatctttaggaatggtgacttggtgggggtcagttacatatacttcatatggtgggtttgtaagtttatatccttcattttctacccattccctcaacttagcatatacagagatgttaattctgaatatgagccccttaaaacagacttcgcacaaaggactccaggcaagtatcttgttccctttacaatctcctttatcggaatggcaagttctgtatcattgccagaaggattgtattcagcgctgtgataaatagttattggcttaccaagaaagtcaattacaaaaatatatataaagaaagcaaagctacatatattaaagcatttaaggtaaaactaaaaatattataaaaatgaaattattttttctcatagctaaagttacataatacgaggaggatttataatgaaaaaagtaataggaattataagtattgtactatttgtactcgtagcacttcaatcctgtgctgcaggagtaggaaatgcattaagtaataacaaagaagctagtggatctgctggattatttttatctgtatgtatgcttattgctggaataatagcaataatatcaaaatatagtaaaggtatgactataacagctatagtattttatttgttagcttttgttgtagggattgctaatgttgggcatttttcagatttgcaaatttggtcaatcattaacttgatatttgctggactattgatatttcatttgcttaaaaataagcaattatataatagcagtgggaaaaagtagaatcatatattgtaattatttttaattatgttggcaaaattgaaattgtcactgaaacacctctaaatgttttaaatacatatgtttaattattgtgacagattctaatagtagaaagtagaaatttgctatgttataatgacatagaggtgaatgtaatatgaaagaagttgtaatagctagtgcagtaagaacagcgattggatcttatggaaagtctcttaaggatgtaccagcagtagatttaggagctacagctataaaggaagcagttaaaaaagcaggaataaaaccagaggatgttaatgaagtcattttaggaaatgttcttcaagcaggtttaggacagaatccagcaagacaggcatcttttaaagcaggattaccagttgaaattccagctatgactattaataaggtttgtggttcaggacttagaacagttagcttagcagcacaaattataaaagcaggagatgctgacgtaataatagcaggtggtatggaaaatatgtctagagctccttacttagcgaataacgctagatggggatatagaatgggaaacgctaaatttgttgatgaaatgatcactgacggattgtgggatgcatttaatgattaccacatgggaataacagcagaaaacatagctgagagatggaacatttcaagagaagaacaagatgagtttgctcttgcatcacaaaaaaaagctgaagaagctataaaatcaggtcaatttaaagatgaaatagttcctgtagtaattaaaggcagaaagggagaaactgtagttgatacagatgagcaccctagatttggatcaactatagaaggacttgcaaaattaaaacctgccttcaaaaaagatggaacagttacagctggtaatgcatcaggattaaatgactgtgcagcagtacttgtaatcatgagtgcagaaaaagctaaagagcttggagtaaaaccacttgctaagatagtttcttatggttcagcaggagttgacccagcaataatgggatatggacctttctatgcaacaaaagcagctattgaaaaagcaggttggacagttgatgaattagatttaatagaatcaaatgaagcttttgcagctcaaagtttagcagtagcaaaagatttaaaatttgatatgaataaagtaaatgtaaatggaggagctattgcccttggtcatccaattggagcatcaggtgcaagaatactcgttactcttgtacacgcaatgcaaaaaagagatgcaaaaaaaggcttagcaactttatgtataggtggcggacaaggaacagcaatattgctagaaaagtgctaggaattcaggaggtatagcatatgacacaaagaatagcatacgtaacaggtggtatgggtggtataggaactgcaatatgtcaaagattagcaaaagatggatttagagttgtagctggatgcggaccaaatagtcctagaagagaaaagtggttagaacaacaaaaagcacttggatttgatttcatagcttctgaaggtaacgtagcagattgggactcaactaaaactgcttttgataaagttaaatctgaagttggtgaagttgatgtattaataaataatgcaggtattactagagatgtagtatttagaaagatgacaagagctgactgggatgcagtaatagatactaatcttactagtcttttcaatgtaactaagcaggtaattgatggtatggcagatagaggttggggtagaatagtaaatattagttcagttaatggacaaaaaggtcagtttggacagacaaattattctacagctaaagcaggtcttcatggttttacaatggctttagcacaggaagttgctacaaaaggtgttacagttaacactgttagtccaggatatattgctactgacatggtaaaggctataagacaagatgttcttgataaaattgttgctacaataccagtaaagagattaggacttcctgaagagatagcatctatttgtgcatggttatcaagtgaagaatcaggattctcaactggtgctgatttttcattaaacggtggtttacacatgggataataccgttcgtataatgtatgctatacgaagttatccttagaagcaaacttaagagtgtgttgatagtgcagtatcttaaaattttgtgtataataggaattgaagttaaattagatgctaaaaatttgtaattaagaaggagggattcgtcatgttggtattccaaatgcgtaatgtagataaaacatctactgttttgaaacagactaaaaacagtgattacgcagataaataaatacgttagattaattcctaccagtgactaatcttatgactttttaaacagataactaaaattacaaacaaatcgtttaacttctgtatttatttacagatgtaatcacttcaggagtaattacatgaacaaaaatataaaatattctcaaaactttttaacgagtgaaaaagtactcaaccaaataataaaacaattgaatttaaaagaaaccgataccgtttacgaaattggaacaggtaaagggcatttaacgacgaaactggctaaaataagtaaacaggtaacgtctattgaattagacagtcatctattcaacttatcgtcagaaaaattaaaactgaacattcgtgtcactttaattcaccaagatattctacagtttcaattccctaacaaacagaggtataaaattgttgggagtattccttaccatttaagcacacaaattattaaaaaagtggtttttgaaagccatgcgtctgacatctatctgattgttgaagaaggattctacaagcgtaccttggatattcaccgaacactagggttgctcttgcacactcaagtctcgattcagcaattgcttaagctgccagcggaatgctttcatcctaaaccaaaagtaaacagtgtcttaataaaacttacccgccataccacagatgttccagataaatattggaagctatatacgtactttgtttcaaaatgggtcaatcgagaatatcgtcaactgtttactaaaaatcagtttcatcaagcaatgaaacacgccaaagtaaacaatttaagtaccattacttatgagcaagtattgtctatttttaatagttatctattatttaacgggaggaaataattctatgagtcgcttttttaaatttggaaagttacacgttactaaagggaatggagataaattattagatatactactgacagcttccaagaagctaaagaggtcataacttcgtataatgtatgctatacgaacggtaagtattgatagaaaaaaacactagacagtgctaataacaatgtctagtgctttttatcttgctcaattttttcattgagttcatttaagtaagtccacctgtccatcttttcgtctagctctttttccagtgaattcttttcggataagagatcttcaagaagtgcataatcagatgaagcagcttccatttctattttcttttcagatatagatttttctagatgttcaattacctcatctattttgtcaaactccatttgttctgcataggtaaattttagaggcttttctttttgcaacttatagttgtttttagctgtatttttcttagagcttattttttcctctgatatttttgcagttttgtgaaaataggaatagtttcctgtatattgagtgattttaccgtttccttcaaaagaaaatattttatcaactgttttgtcaaggaagtacctgtcatgagatacagctataacagctccttcaaaatcgttaatataatcttctaggattgtaagtgtttctatatccagatcatttgttggttcgtccagcaaaagtacattagggtaattcatcagtatttttagaagatataatcttcttcgttctcctcctgaaagttttccaaggggagtccattgaactgaaggttcaaataaaaaattttcaagtacagcagaagcacttattttttcacccgatgaagttgacgcatattctgatgtcccacgtatgtattcaattaccctttcgttcatatccatatcagaaattccctgagaatagtatcctatctttactgtttcacctatatctatagtgccgctgtccggcagaattttttgaactaaaatattcataagagtggatttaccacttccattaggtccaataatacctattctgtcattatttagtatgttataagtgaaatttttaattaatgtcttttcaccaaaacttttgcttatgttatccaggtttatgactttttgttt

SEQ ID NO: 122 - DNA, 43 bp, Artificial sequence
  Synthetic polynucleotide
  misc_feature: SN01
atttacaaattcggccggcctacctcctcgtataaataagatg

SEQ ID NO: 123 - DNA, 43 bp, Artificial sequence
  Synthetic polynucleotide
  misc_feature: SN02
ctagctattacaacttctttcatattacattcacctctatgtc

SEQ ID NO: 124 - DNA, 43 bp, Artificial sequence
  Synthetic polynucleotide
  misc_feature: SN03
gacatagaggtgaatgtaatatgaaagaagttgtaatagctag

SEQ ID NO: 125 - DNA, 49 bp, Artificial sequence
  Synthetic polynucleotide
  misc_feature: SN04mod
gtatagcatacattatacgaacggtattatcccatgtgtaaaccaccgt

SEQ ID NO: 126 - DNA, 48 bp, Artificial sequence
  Synthetic polynucleotide
  misc_feature: SN05mod
ttcgtataatgtatgctatacgaagttatccttagaagcaaacttaag

SEQ ID NO: 127 - DNA, 46 bp, Artificial sequence
  Synthetic polynucleotide
  misc_feature: SN06
gtctagtgtttttttctatcaatactctagataccgttcgtatagc

SEQ ID NO: 128 - DNA, 46 bp, Artificial sequence
  Synthetic polynucleotide
  misc_feature: SN07
tgtatgctatacgaacggtaagtattgatagaaaaaaacactagac

SEQ ID NO: 129 - DNA, 40 bp, Artificial sequence
  Synthetic polynucleotide
  misc_feature: SN08
caaaaaggagtttaaacaaaaagtcataaacctggataac

SEQ ID NO: 130 - DNA, 25 bp, Artificial sequence
  Synthetic polynucleotide
  misc_feature: Og31f
ccgtttctcacaacaacaataccag

SEQ ID NO: 131 - DNA, 25 bp, Artificial sequence
  Synthetic polynucleotide
  misc_feature: Og32r
aaaccaccttgacgatgaaaccata

SEQ ID NO: 132 - DNA, 7951 bp, Artificial sequence
  Synthetic polynucleotide
  misc_feature: pMTL8315-Pfdx-thlA-phaB-bld, plasmid
cctgcaggataaaaaaattgtagataaattttataaaatagttttatctacaatttttttatcaggaaacagctatgaccgcggccgctcactatctgcggaacctgcctccttatctgataaaaaatattcgctgcatctttgacttgttattttctttcaaatgcctaaaattatcttttaaaattataacaaatgtgataaaatacaggggatgaaaacattatctaaaaattaaggaggtgttacatatgaaagaagttgtaatagctagtgcagtaagaacagcgattggatcttatggaaagtctcttaaggatgtaccagcagtagatttaggagctacagctataaaggaagcagttaaaaaagcaggaataaaaccagaggatgttaatgaagtcattttaggaaatgttcttcaagcaggtttaggacagaatccagcaagacaggcatcttttaaagcaggattaccagttgaaattccagctatgactattaataaggtttgtggttcaggacttagaacagttagcttagcagcacaaattataaaagcaggagatgctgacgtaataatagcaggtggtatggaaaatatgtctagagctccttacttagcgaataacgctagatggggatatagaatgggaaacgctaaatttgttgatgaaatgatcactgacggattgtgggatgcatttaatgattaccacatgggaataacagcagaaaacatagctgagagatggaacatttcaagagaagaacaagatgagtttgctcttgcatcacaaaaaaaagctgaagaagctataaaatcaggtcaatttaaagatgaaatagttcctgtagtaattaaaggcagaaagggagaaactgtagttgatacagatgagcaccctagatttggatcaactatagaaggacttgcaaaattaaaacctgccttcaaaaaagatggaacagttacagctggtaatgcatcaggattaaatgactgtgcagcagtacttgtaatcatgagtgcagaaaaagctaaagagcttggagtaaaaccacttgctaagatagtttcttatggttcagcaggagttgacccagcaataatgggatatggacctttctatgcaacaaaagcagctattgaaaaagcaggttggacagttgatgaattagatttaatagaatcaaatgaagcttttgcagctcaaagtttagcagtagcaaaagatttaaaatttgatatgaataaagtaaatgtaaatggaggagctattgcccttggtcatccaattggagcatcaggtgcaagaatactcgttactcttgtacacgcaatgcaaaaaagagatgcaaaaaaaggcttagcaactttatgtataggtggcggacaaggaacagcaatattgctagaaaagtgctaggaattcaggaggtatagcatatgacacaaagaatagcatacgtaacaggtggtatgggtggtataggaactgcaatatgtcaaagattagcaaaagatggatttagagttgtagctggatgcggaccaaatagtcctagaagagaaaagtggttagaacaacaaaaagcacttggatttgatttcatagcttctgaaggtaacgtagcagattgggactcaactaaaactgcttttgataaagttaaatctgaagttggtgaagttgatgtattaataaataatgcaggtattactagagatgtagtatttagaaagatgacaagagctgactgggatgcagtaatagatactaatcttactagtcttttcaatgtaactaagcaggtaattgatggtatggcagatagaggttggggtagaatagtaaatattagttcagttaatggacaaaaaggtcagtttggacagacaaattattctacagctaaagcaggtcttcatggttttacaatggctttagcacaggaagttgctacaaaaggtgttacagttaacactgttagtccaggatatattgctactgacatggtaaaggctataagacaagatgttcttgataaaattgttgctacaataccagtaaagagattaggacttcctgaagagatagcatctatttgtgcatggttatcaagtgaagaatcaggattctcaactggtgctgatttttcattaaacggtggtttacacatgggataagaaggagatatacatatgataaaagatacacttgttagtattacaaaagatttaaaacttaaaactaatgttgaaaatgcaaatcttaaaaattataaagatgatagttcttgttttggagtatttgaaaatgttgaaaatgcaataagtaatgcagtacatgctcaaaaaattttatctcttcattatacaaaagaacagagagaaaaaattataactgaaattagaaaagcagctttagaaaataaagaaatattagctacaatgattcttgaagaaactcacatgggaagatatgaagataaaatacttaaacatgaacttgtagcaaaatatacacctggaactgaagatttaactacaactgcttggtcaggtgataatggacttacagtagttgaaatgagtccttatggagttataggagcaattacaccttctactaatccaacagaaactgtaatatgtaattcaattggtatgattgcagctggaaatactgtagtttttaatggtcatcctggagctaaaaaatgtgtagcatttgctgttgaaatgattaataaagctataattagttgtggaggtcctgaaaatcttgttacaactataaaaaatccaacaatggattctcttgatgcaataattaaacatccttcaattaaacttctttgtggtacaggaggtccaggaatggtaaaaactcttcttaattctggtaaaaaagctataggagcaggtgctggaaatcctccagtaattgttgatgatacagcagatatagaaaaagctggtaaatcaattattgaaggatgtagttttgataataatttaccatgtatagcagaaaaagaagtatttgtttttgaaaatgttgctgatgatttaattagtaatatgcttaaaaataatgcagtaataattaatgaagatcaagtttctaaacttatagatttagtattacagaaaaataatgaaacacaggaatattctattaataaaaaatgggtaggaaaagatgcaaaattatttcttgatgaaatagatgtagaatcaccttcaagtgttaaatgtataatttgtgaagtttctgcttcacatccatttgtaatgactgaattaatgatgcctatacttccaattgtaagagttaaagatatagatgaagcaatagaatatgcaaaaattgctgaacagaatagaaaacatagtgcttatatttattctaaaaatatagataatttaaatagatttgaaagagaaatagatacaactatttttgttaaaaatgcaaaatcatttgctggtgtaggatatgaagcagaaggttttacaacttttacaatagctggaagtactggtgaaggtattacaagtgcaagaaattttacaagacagagaagatgtgttttagcaggttaatctagagtcgacgtcacgcgtccatggagatctcgaggcctgcagacatgcaagcttggcactggccgtcgttttacaacgtcgtgactgggaaaaccctggcgttacccaacttaatcgccttgcagcacatccccctttcgccagctggcgtaatagcgaagaggcccgcaccgatcgcccttcccaacagttgcgcagcctgaatggcgaatggcgctagcataaaaataagaagcctgcatttgcaggcttcttatttttatggcgcgccgccattatttttttgaacaattgacaattcatttcttattttttattaagtgatagtcaaaaggcataacagtgctgaatagaaagaaatttacagaaaagaaaattatagaatttagtatgattaattatactcatttatgaatgtttaattgaatacaaaaaaaaatacttgttatgtattcaattacgggttaaaatatagacaagttgaaaaatttaataaaaaaataagtcctcagctcttatatattaagctaccaacttagtatataagccaaaacttaaatgtgctaccaacacatcaagccgttagagaactctatctatagcaatatttcaaatgtaccgacatacaagagaaacattaactatatatattcaatttatgagattatcttaacagatataaatgtaaattgcaataagtaagatttagaagtttatagcctttgtgtattggaagcagtacgcaaaggcttttttatttgataaaaattagaagtatatttattttttcataattaatttatgaaaatgaaagggggtgagcaaagtgacagaggaaagcagtatcttatcaaataacaaggtattagcaatatcattattgactttagcagtaaacattatgacttttatagtgcttgtagctaagtagtacgaaagggggagctttaaaaagctccttggaatacatagaattcataaattaatttatgaaaagaagggcgtatatgaaaacttgtaaaaattgcaaagagtttattaaagatactgaaatatgcaaaatacattcgttgatgattcatgataaaacagtagcaacctattgcagtaaatacaatgagtcaagatgtttacataaagggaaagtccaatgtattaattgttcaaagatgaaccgatatggatggtgtgccataaaaatgagatgttttacagaggaagaacagaaaaaagaacgtacatgcattaaatattatgcaaggagctttaaaaaagctcatgtaaagaagagtaaaaagaaaaaataatttatttattaatttaatattgagagtgccgacacagtatgcactaaaaaatatatctgtggtgtagtgagccgatacaaaaggatagtcactcgcattttcataatacatcttatgttatgattatgtgtcggtgggacttcacgacgaaaacccacaataaaaaaagagttcggggtagggttaagcatagttgaggcaactaaacaatcaagctaggatatgcagtagcagaccgtaaggtcgttgtttaggtgtgttgtaatacatacgctattaagatgtaaaaatacggataccaatgaagggaaaagtataatttttggatgtagtttgtttgttcatctatgggcaaactacgtccaaagccgtttccaaatctgctaaaaagtatatcctttctaaaatcaaagtcaagtatgaaatcataaataaagtttaattttgaagttattatgatattatgtttttctattaaaataaattaagtatatagaatagtttaataatagtatatacttaatgtgataagtgtctgacagtgtcacagaaaggatgattgttatggattataagcggccggccagtgggcaagttgaaaaattcacaaaaatgtggtataatatctttgttcattagagcgataaacttgaatttgagagggaacttagatggtatttgaaaaaattgataaaaatagttggaacagaaaagagtattttgaccactactttgcaagtgtaccttgtacctacagcatgaccgttaaagtggatatcacacaaataaaggaaaagggaatgaaactatatcctgcaatgctttattatattgcaatgattgtaaaccgccattcagagtttaggacggcaatcaatcaagatggtgaattggggatatatgatgagatgataccaagctatacaatatttcacaatgatactgaaacattttccagcctttggactgagtgtaagtctgactttaaatcatttttagcagattatgaaagtgatacgcaacggtatggaaacaatcatagaatggaaggaaagccaaatgctccggaaaacatttttaatgtatctatgataccgtggtcaaccttcgatggctttaatctgaatttgcagaaaggatatgattatttgattcctatttttactatggggaaatattataaagaagataacaaaattatacttcctttggcaattcaagttcatcacgcagtatgtgacggatttcacatttgccgttttgtaaacgaattgcaggaattgataaatagttaacttcaggtttgtctgtaactaaaaacaagtatttaagcaaaaacatcgtagaaatacggtgttttttgttaccctaagtttaaactcctttttgataatctcatgaccaaaatcccttaacgtgagttttcgttccactgagcgtcagaccccgtagaaaagatcaaaggatcttcttgagatcctttttttctgcgcgtaatctgctgcttgcaaacaaaaaaaccaccgctaccagcggtggtttgtttgccggatcaagagctaccaactctttttccgaaggtaactggcttcagcagagcgcagataccaaatactgttcttctagtgtagccgtagttaggccaccacttcaagaactctgtagcaccgcctacatacctcgctctgctaatcctgttaccagtggctgctgccagtggcgataagtcgtgtcttaccgggttggactcaagacgatagttaccggataaggcgcagcggtcgggctgaacggggggttcgtgcacacagcccagcttggagcgaacgacctacaccgaactgagatacctacagcgtgagctatgagaaagcgccacgcttcccgaagggagaaaggcggacaggtatccggtaagcggcagggtcggaacaggagagcgcacgagggagcttccagggggaaacgcctggtatctttatagtcctgtcgggtttcgccacctctgacttgagcgtcgatttttgtgatgctcgtcaggggggcggagcctatggaaaaacgccagcaacgcggcctttttacggttcctggccttttgctggccttttgctcacatgttctttcctgcgttatcccctgattctgtggataaccgtattaccgcctttgagtgagctgataccgctcgccgcagccgaacgaccgagcgcagcgagtcagtgagcgaggaagcggaagagcgcccaatacgcagggccccctgcttcggggtcattatagcgattttttcggtatatccatcctttttcgcacgatatacaggattttgccaaagggttcgtgtagactttccttggtgtatccaacggcgtcagccgggcaggataggtgaagtaggcccacccgcgagcgggtgttccttcttcactgtcccttattcgcacctggcggtgctcaacgggaatcctgctctgcgaggctggccggctaccgccggcgtaacagatgagggcaagcggatggctgatgaaaccaagccaaccaggaagggcagcccacctatcaaggtgtactgccttccagacgaacgaagagcgattgaggaaaaggcggcggcggccggcatgagcctgtcggcctacctgctggccgtcggccagggctacaaaatcacgggcgtcgtggactatgagcacgtccgcgagctggcccgcatcaatggcgacctgggccgcctgggcggcctgctgaaactctggctcaccgacgacccgcgcacggcgcggttcggtgatgccacgatcctcgccctgctggcgaagatcgaagagaagcaggacgagcttggcaaggtcatgatgggcgtggtccgcccgagggcagagccatgacttttttagccgctaaaacggccggggggtgcgcgtgattgccaagcacgtccccatgcgctccatcaagaagagcgacttcgcggagctggtgaagtacatcaccgacgagcaaggcaagaccgatcgggccc

SEQ ID NO: 133 - DNA, 36 bp, Artificial sequence
  Synthetic polynucleotide
  misc_feature: bld-phaB-F1, forward
acatgggataagaaggagatatacatatgataaaag

SEQ ID NO: 134 - DNA, 36 bp, Artificial sequence
  Synthetic polynucleotide
  misc_feature: bld-pMTL-R1, forward
cgtcgactctagattaacctgctaaaacacatcttc

SEQ ID NO: 135 - DNA, 36 bp, Artificial sequence
  Synthetic polynucleotide
  misc_feature: pMTL-bld-F1, forward
gtgttttagcaggttaatctagagtcgacgtcacgc

SEQ ID NO: 136 - DNA, 1179 bp, Clostridium acetobutylicum
  misc_feature: thlA
atgaaagaagttgtaatagctagtgcagtaagaacagcgattggatcttatggaaagtctcttaaggatgtaccagcagtagatttaggagctacagctataaaggaagcagttaaaaaagcaggaataaaaccagaggatgttaatgaagtcattttaggaaatgttcttcaagcaggtttaggacagaatccagcaagacaggcatcttttaaagcaggattaccagttgaaattccagctatgactattaataaggtttgtggttcaggacttagaacagttagcttagcagcacaaattataaaagcaggagatgctgacgtaataatagcaggtggtatggaaaatatgtctagagctccttacttagcgaataacgctagatggggatatagaatgggaaacgctaaatttgttgatgaaatgatcactgacggattgtgggatgcatttaatgattaccacatgggaataacagcagaaaacatagctgagagatggaacatttcaagagaagaacaagatgagtttgctcttgcatcacaaaaaaaagctgaagaagctataaaatcaggtcaatttaaagatgaaatagttcctgtagtaattaaaggcagaaagggagaaactgtagttgatacagatgagcaccctagatttggatcaactatagaaggacttgcaaaattaaaacctgccttcaaaaaagatggaacagttacagctggtaatgcatcaggattaaatgactgtgcagcagtacttgtaatcatgagtgcagaaaaagctaaagagcttggagtaaaaccacttgctaagatagtttcttatggttcagcaggagttgacccagcaataatgggatatggacctttctatgcaacaaaagcagctattgaaaaagcaggttggacagttgatgaattagatttaatagaatcaaatgaagcttttgcagctcaaagtttagcagtagcaaaagatttaaaatttgatatgaataaagtaaatgtaaatggaggagctattgcccttggtcatccaattggagcatcaggtgcaagaatactcgttactcttgtacacgcaatgcaaaaaagagatgcaaaaaaaggcttagcaactttatgtataggtggcggacaaggaacagcaatattgctagaaaagtgctag

SEQ ID NO: 137 - DNA, 849 bp, Clostridium kluyveri
  misc_feature: hbd1
atgagtattaaaagtgtagcggttttaggtagtggaactatgtctcgtggaattgtgcaggcttttgcagaagcaggtatagatgtaattatccgtggaagaactgaaggtagtattggaaaaggtctagcagcagtaaagaaagcttatgataaaaaagtatcaaaggggaaaatttcccaggaagatgctgataaaatagttggaagagtaagtacaacaactgaacttgaaaaattggctgattgtgatcttataatagaagcagcatcagaggatatgaatataaagaaagactattttggaaaattagaagaaatatgcaagcctgaaacaatttttgctactaatacttcttcattatctataactgaagtagcaacagctacaaagagaccagataaattcataggaatgcatttctttaatccagcaaatgttatgaaattagttgaaatcataagaggtatgaatacttcacaagaaacttttgatattataaaagaagcttccattaaaataggaaaaactcctgtagaagttgcagaagctccaggatttgttgtaaacaagatattagtaccaatgatcaatgaagcagtaggaattttggcagaaggaatagcttcagcagaagatatcgatacagctatgaaattaggcgctaatcacccaatgggtcctttagcattaggagatcttattggacttgatgtagttcttgcagttatggatgtactttatagtgaaactggagattcaaaatatagagctcatacattacttagaaaatatgtaagagcaggatggcttggaagaaaatcaggaaaaggattcttcgcttattaa

SEQ ID NO: 138 - DNA, 176 bp, Clostridium autoethanogenum
  misc_feature: ferredoxin promoter
ggccgcgctcactatctgcggaacctgcctccttatctgataaaaaatattcgctgcatctttgacttgttattttctttcaaatgcctaaaattatcttttaaaattataacaaatgtgataaaatacaggggatgaaaacattatctaaaaattaaggaggtgttacagaattc

SEQ ID NO: 139 - DNA, 474 bp, Clostridium autoethanogenum
  misc_feature: pyruvate-ferredoxin oxidoreductase promoter
aaaatagttgataataatgcagagttataaacaaaggtgaaaagcattacttgtattcttttttatatattattataaattaaaatgaagctgtattagaaaaaatacacacctgtaatataaaattttaaattaatttttaattttttcaaaatgtattttacatgtttagaattttgatgtatattaaaatagtagaatacataagatacttaatttaattaaagatagttaagtacttttcaatgtgcttttttagatgtttaatacaaatctttaattgtaaaagaaatgctgtactatttactgtactagtgacgggattaaactgtattaattataaataaaaaataagtacagttgtttaaaattatattttgtattaaatctaatagtacgatgtaagttattttatactattgctagtttaataaaaagatttaattatatgcttgaaaaggagaggaattcata

SEQ ID NO: 140 - DNA, 22 bp, Artificial sequence
  Synthetic polynucleotide
  misc_feature: ribosome binding site rbs2
aaatagaaaggaggtgttacat

SEQ ID NO: 141 - DNA, 35 bp, Artificial sequence
  Synthetic polynucleotide
  misc_feature: Pfdx-F1, forward
aaaggtctccggccgcgctcactatctgcggaacc

SEQ ID NO: 142 - DNA, 38 bp, Artificial sequence
  Synthetic polynucleotide
  misc_feature: Pfdx-R1, reverse
tttggtctcgaattctgtaacacctccttaatttttag

SEQ ID NO: 143 - DNA, 40 bp, Artificial sequence
  Synthetic polynucleotide
  misc_feature: Ppfor-F1, forward
aaaggtctccggccgcaaaatagttgataataatgcagag

SEQ ID NO: 144 - DNA, 35 bp, Artificial sequence
  Synthetic polynucleotide
  misc_feature: Ppfor-R1, reverse
tttggtctcgaattcctctccttttcaagcatata

SEQ ID NO: 145 - DNA, 45 bp, Artificial sequence
  Synthetic polynucleotide
  misc_feature: hbd1-F1, forward
aaaggtctcgaattcaaagatctatgtctattaaatcagttgcag

SEQ ID NO: 146 - DNA, 47 bp, Artificial sequence
  Synthetic polynucleotide
  misc_feature: hbd1-R1, reverse
tttggtctccctcctttctatttctaatatgcgaaaaatcctttacc

SEQ ID NO: 147 - DNA, 49 bp, Artificial sequence
  Synthetic polynucleotide
  misc_feature: thlA-F1, forward
aaaggtctcaggaggtgttacatatgaaagaagttgtaatagctagtgc

SEQ ID NO: 148 - DNA, 48 bp, Artificial sequence
  Synthetic polynucleotide
  misc_feature: thlA-R1, reverse
tttggtctcctcgagtatggatccctagcacttttctagcaatattgc

SEQ ID NO: 149 - DNA, 30 bp, Artificial sequence
  Synthetic polynucleotide
  misc_feature: Ppfor-F2, forward
aaacagctatgaccgcggccgcaaaatagt

SEQ ID NO: 150 - DNA, 24 bp, Artificial sequence
  Synthetic polynucleotide
  misc_feature: Ppfor-R2, reverse
ttactcattggattcctctccttt

SEQ ID NO: 151 - DNA, 29 bp, Artificial sequence
  Synthetic polynucleotide
  misc_feature: Ptb-Buk-F2, forward
ggaatccaatgagtaaaaactttgatgag

SEQ ID NO: 152 - DNA, 37 bp, Artificial sequence
  Synthetic polynucleotide
  misc_feature: Ptb-Buk-F2, reverse
caggcctcgagatctcctagtaaaccttagcttgttc

SEQ ID NO: 153 - DNA, 7884 bp, Artificial sequence
  Synthetic polynucleotide
  misc_feature: pMTL82256-ptb-buk, plasmid
gagatctcgaggcctgcagacatgcaagcttggcactggccgtcgttttacaacgtcgtgactgggaaaaccctggcgttacccaacttaatcgccttgcagcacatccccctttcgccagctggcgtaatagcgaagaggcccgcaccgatcgcccttcccaacagttgcgcagcctgaatggcgaatggcgctagcataaaaataagaagcctgcatttgcaggcttcttatttttatggcgcgccgttctgaatccttagctaatggttcaacaggtaactatgacgaagatagcaccctggataagtctgtaatggattctaaggcatttaatgaagacgtgtatataaaatgtgctaatgaaaaagaaaatgcgttaaaagagcctaaaatgagttcaaatggttttgaaattgattggtagtttaatttaatatattttttctattggctatctcgatacctatagaatcttctgttcacttttgtttttgaaatataaaaaggggctttttagccccttttttttaaaactccggaggagtttcttcattcttgatactatacgtaactattttcgatttgacttcattgtcaattaagctagtaaaatcaatggttaaaaaacaaaaaacttgcatttttctacctagtaatttataattttaagtgtcgagtttaaaagtataatttaccaggaaaggagcaagttttttaataaggaaaaatttttccttttaaaattctatttcgttatatgactaattataatcaaaaaaatgaaaataaacaagaggtaaaaactgctttagagaaatgtactgataaaaaaagaaaaaatcctagatttacgtcatacatagcacctttaactactaagaaaaatattgaaaggacttccacttgtggagattatttgtttatgttgagtgatgcagacttagaacattttaaattacataaaggtaatttttgcggtaatagattttgtccaatgtgtagttggcgacttgcttgtaaggatagtttagaaatatctattcttatggagcatttaagaaaagaagaaaataaagagtttatatttttaactcttacaactccaaatgtaaaaagttatgatcttaattattctattaaacaatataataaatcttttaaaaaattaatggagcgtaaggaagttaaggatataactaaaggttatataagaaaattagaagtaacttaccaaaaggaaaaatacataacaaaggatttatggaaaataaaaaaagattattatcaaaaaaaaggacttgaaattggtgatttagaacctaattttgatacttataatcctcattttcatgtagttattgcagttaataaaagttattttacagataaaaattattatataaatcgagaaagatggttggaattatggaagtttgctactaaggatgattctataactcaagttgatgttagaaaagcaaaaattaatgattataaagaggtttacgaacttgcgaaatattcagctaaagacactgattatttaatatcgaggccagtatttgaaattttttataaagcattaaaaggcaagcaggtattagtttttagtggattttttaaagatgcacacaaattgtacaagcaaggaaaacttgatgtttataaaaagaaagatgaaattaaatatgtctatatagtttattataattggtgcaaaaaacaatatgaaaaaactagaataagggaacttacggaagatgaaaaagaagaattaaatcaagatttaatagatgaaatagaaatagattaaagtgtaactatactttatatatatatgattaaaaaaataaaaaacaacagcctattaggttgttgttttttattttctttattaatttttttaatttttagtttttagttcttttttaaaataagtttcagcctctttttcaatattttttaaagaaggagtatttgcatgaattgccttttttctaacagacttaggaaatattttaacagtatcttcttgcgccggtgattttggaacttcataacttactaatttataattattattttcttttttaattgtaacagttgcaaaagaagctgaacctgttccttcaactagtttatcatcttcaatataatattcttgacctatatagtataaatatatttttattatatttttacttttttctgaatctattattttataatcataaaaagttttaccaccaaaagaaggttgtactccttctggtccaacatatttttttactatattatctaaataatttttgggaactggtgttgtaatttgattaatcgaacaaccagttatacttaaaggaattataactataaaaatatataggattatctttttaaatttcattattggcctcctttttattaaatttatgttaccataaaaaggacataacgggaatatgtagaatatttttaatgtagacaaaattttacataaatataaagaaaggaagtgtttgtttaaattttatagcaaactatcaaaaattagggggataaaaatttatgaaaaaaaggttttcgatgttatttttatgtttaactttaatagtttgtggtttatttacaaattcggccggccgaagcaaacttaagagtgtgttgatagtgcagtatcttaaaattttgtataataggaattgaagttaaattagatgctaaaaatttgtaattaagaaggagtgattacatgaacaaaaatataaaatattctcaaaactttttaacgagtgaaaaagtactcaaccaaataataaaacaattgaatttaaaagaaaccgataccgtttacgaaattggaacaggtaaagggcatttaacgacgaaactggctaaaataagtaaacaggtaacgtctattgaattagacagtcatctattcaacttatcgtcagaaaaattaaaactgaatactcgtgtcactttaattcaccaagatattctacagtttcaattccctaacaaacagaggtataaaattgttgggagtattccttaccatttaagcacacaaattattaaaaaagtggtttttgaaagccatgcgtctgacatctatctgattgttgaagaaggattctacaagcgtaccttggatattcaccgaacactagggttgctcttgcacactcaagtctcgattcagcaattgcttaagctgccagcggaatgctttcatcctaaaccaaaagtaaacagtgtcttaataaaacttacccgccataccacagatgttccagataaatattggaagctatatacgtactttgtttcaaaatgggtcaatcgagaatatcgtcaactgtttactaaaaatcagtttcatcaagcaatgaaacacgccaaagtaaacaatttaagtaccgttacttatgagcaagtattgtctatttttaatagttatctattatttaacgggaggaaataattctatgagtcgcttttgtaaatttggaaagttacacgttactaaagggaatgtgtttaaactcctttttgataatctcatgaccaaaatcccttaacgtgagttttcgttccactgagcgtcagaccccgtagaaaagatcaaaggatcttcttgagatcctttttttctgcgcgtaatctgctgcttgcaaacaaaaaaaccaccgctaccagcggtggtttgtttgccggatcaagagctaccaactctttttccgaaggtaactggcttcagcagagcgcagataccaaatactgttcttctagtgtagccgtagttaggccaccacttcaagaactctgtagcaccgcctacatacctcgctctgctaatcctgttaccagtggctgctgccagtggcgataagtcgtgtcttaccgggttggactcaagacgatagttaccggataaggcgcagcggtcgggctgaacggggggttcgtgcacacagcccagcttggagcgaacgacctacaccgaactgagatacctacagcgtgagctatgagaaagcgccacgcttcccgaagggagaaaggcggacaggtatccggtaagcggcagggtcggaacaggagagcgcacgagggagcttccagggggaaacgcctggtatctttatagtcctgtcgggtttcgccacctctgacttgagcgtcgatttttgtgatgctcgtcaggggggcggagcctatggaaaaacgccagcaacgcggcctttttacggttcctggccttttgctggccttttgctcacatgttctttcctgcgttatcccctgattctgtggataaccgtattaccgcctttgagtgagctgataccgctcgccgcagccgaacgaccgagcgcagcgagtcagtgagcgaggaagcggaagagcgcccaatacgcagggccccctgcttcggggtcattatagcgattttttcggtatatccatcctttttcgcacgatatacaggattttgccaaagggttcgtgtagactttccttggtgtatccaacggcgtcagccgggcaggataggtgaagtaggcccacccgcgagcgggtgttccttcttcactgtcccttattcgcacctggcggtgctcaacgggaatcctgctctgcgaggctggccggctaccgccggcgtaacagatgagggcaagcggatggctgatgaaaccaagccaaccaggaagggcagcccacctatcaaggtgtactgccttccagacgaacgaagagcgattgaggaaaaggcggcggcggccggcatgagcctgtcggcctacctgctggccgtcggccagggctacaaaatcacgggcgtcgtggactatgagcacgtccgcgagctggcccgcatcaatggcgacctgggccgcctgggcggcctgctgaaactctggctcaccgacgacccgcgcacggcgcggttcggtgatgccacgatcctcgccctgctggcgaagatcgaagagaagcaggacgagcttggcaaggtcatgatgggcgtggtccgcccgagggcagagccatgacttttttagccgctaaaacggccggggggtgcgcgtgattgccaagcacgtccccatgcgctccatcaagaagagcgacttcgcggagctggtgaagtacatcaccgacgagcaaggcaagaccgatcgggccccctgcaggataaaaaaattgtagataaattttataaaatagttttatctacaatttttttatcaggaaacagctatgaccgcggccgcaaaatagttgataataatgcagagttataaacaaaggtgaaaagcattacttgtattcttttttatatattattataaattaaaatgaagctgtattagaaaaaatacacacctgtaatataaaattttaaattaatttttaattttttcaaaatgtattttacatgtttagaattttgatgtatattaaaatagtagaatacataagatacttaatttaattaaagatagttaagtacttttcaatgtgcttttttagatgtttaatacaaatctttaattgtaaaagaaatgctgtactatttactgtactagtgacgggattaaactgtattaattataaataaaaaataagtacagttgtttaaaattatattttgtattaaatctaatagtacgatgtaagttattttatactattgctagtttaataaaaagatttaattatatgcttgaaaaggagaggaatccaatgagtaaaaactttgatgagttattatcaagattaaaggaagttccaacaaaaaaagtggctgtagccgtagcacaagatgaaccagtattagaggctataaaagaagctacagaaaataacatcgcacaagcaatattggttggtgataaacaacaaatccatgaaatcgcaaagaaaataaacttggacttatctgattatgaaataatggatattaaagatccaaagaaagcaacattagaagcagtaaaattagtttctagtggtcatgcagatatgttaatgaaaggtctagttgatactgcaacattcctaagaagcgtattaaacaaagaggttggtcttagaacaggaaaattaatgtcccatgtagctgtgtttgatgtggaaggttgggatagactgttatttttaactgatgcagcatttaatacatatccagaatttaaggataaagttggaatgataaataatgcagttgtagttgctcatgcatgtggaatagatgttccaagagtagcacctatatgcccagttgaagttgtaaatacaagtatgcaatcaacagttgatgcagcattgttagctaaaatgagtgacagggggcaaattaaaggatgcgtaattgatggaccttttgccttagataatgcaatatcagaagaagcagctcatcataaaggtgttacaggatcagtagcaggtaaagctgatatattattattaccaaatatagaagcagcaaatgtaatgtataaaacattaacatatttctctaaatcaagaaatggtggacttttagtaggtacatcagcaccagtaattttaacttcaagagcagattcattcgaaactaaagttaattcaattgctcttgcagcattagttgcagcaagaaataagtaataaatcaatccataataattaatgcataattaatggagagatttatatggaatttgcaatgcactattagattctataataatttcttctgaaaattatgcattatgactgtatagaatgcattaaatttaagggggattcagaatgtcatataagctattaataatcaatccaggttcaacatcaacaaagattggtgtttacgaaggagaaaaggaactatttgaagaaactttgagacacacaaatgaagaaataaagagatatgatacaatatatgatcaatttgaatttagaaaagaagttatattaaatgttcttaaagaaaagaattttgatataaagactctaagtgctattgttggtagaggtggaatgcttagaccagttgaaggtggaacatatgcagtaaatgatgcaatggttgaagatttaaaagttggagttcaaggacctcatgcttctaaccttggcggaataattgccaagtcaattggagatgaattaaatattccatcatttatagtagatccagttgttacagatgagttagcagatgtagcaagactatctggagtaccagaactaccaagaaaaagtaaattccatgctttaaatcaaaaagcggtagctaaaagatatggaaaagaaagtggacaaggatatgaaaacctaaatcttgtagttgtacatatgggtggaggcgtttcagttggtgctcacaatcatgggaaagttgtcgatgtaaataatgcattagatggagatggcccattctcaccagaaagagctggatcagttccaattggtgatttagttaaaatgtgttttagtggaaaatatagtgaagcagaagtatatggcaaggctgtaggaaaaggtggatttgttggttatctaaacacaaatgatgtaaaaggtgttattgataagatggaagaaggagataaagaatgtgaatcaatatacaaagcatttgtttatcaaatttcaaaagcaatcggagaaatgtcagttgtattagaaggtaaagttgatcaaattatttttaccggaggaattgcatactcaccaacacttgttccagaccttaaagcaaaagttgaatggatagccccagttacagtttatcctggagaagatgaattacttgctctagctcaaggtgctataagagtacttgatggagaagaacaagctaaggtttactag

SEQ ID NO: 154 - protein, 436 aa, Clostridium autoethanogenum; identical to SEQ ID NO: 8
  MISC_FEATURE: thioesterase 1

SEQ ID NO: 155 - protein, 60 aa, Clostridium ljungdahlii
  MISC_FEATURE: thioesterase 2
MYINETKVVVRYAETDKMGIVHHSNYYIYFEEARTQFIKKTGISYSQMEKDGIMFPLVES

SEQ ID NO: 156 - protein, 128 aa, Clostridium autoethanogenum; identical to SEQ ID NO: 10
  MISC_FEATURE: thioesterase 3

SEQ ID NO: 157 - protein, 436 aa, Clostridium ljungdahlii; identical to SEQ ID NO: 8
  MISC_FEATURE: thioesterase 1

SEQ ID NO: 158 - protein, 137 aa, Clostridium autoethanogenum; identical to SEQ ID NO: 9
  MISC_FEATURE: thioesterase 2

SEQ ID NO: 159 - protein, 128 aa, Clostridium ljungdahlii; identical to SEQ ID NO: 10
  MISC_FEATURE: thioesterase 3

SEQ ID NO: 160 - DNA, 11184 bp, Artificial sequence
  Synthetic polynucleotide
  misc_feature: pMTL8225-pta-ack::ptb-buk, plasmid
aaactcctttttgataatctcatgaccaaaatcccttaacgtgagttttcgttccactgagcgtcagaccccgtagaaaagatcaaaggatcttcttgagatcctttttttctgcgcgtaatctgctgcttgcaaacaaaaaaaccaccgctaccagcggtggtttgtttgccggatcaagagctaccaactctttttccgaaggtaactggcttcagcagagcgcagataccaaatactgttcttctagtgtagccgtagttaggccaccacttcaagaactctgtagcaccgcctacatacctcgctctgctaatcctgttaccagtggctgctgccagtggcgataagtcgtgtcttaccgggttggactcaagacgatagttaccggataaggcgcagcggtcgggctgaacggggggttcgtgcacacagcccagcttggagcgaacgacctacaccgaactgagatacctacagcgtgagctatgagaaagcgccacgcttcccgaagggagaaaggcggacaggtatccggtaagcggcagggtcggaacaggagagcgcacgagggagcttccagggggaaacgcctggtatctttatagtcctgtcgggtttcgccacctctgacttgagcgtcgatttttgtgatgctcgtcaggggggcggagcctatggaaaaacgccagcaacgcggcctttttacggttcctggccttttgctggccttttgctcacatgttctttcctgcgttatcccctgattctgtggataaccgtattaccgcctttgagtgagctgataccgctcgccgcagccgaacgaccgagcgcagcgagtcagtgagcgaggaagcggaagagcgcccaatacgcagggccccctgcttcggggtcattatagcgattttttcggtatatccatcctttttcgcacgatatacaggattttgccaaagggttcgtgtagactttccttggtgtatccaacggcgtcagccgggcaggataggtgaagtaggcccacccgcgagcgggtgttccttcttcactgtcccttattcgcacctggcggtgctcaacgggaatcctgctctgcgaggctggccggctaccgccggcgtaacagatgagggcaagcggatggctgatgaaaccaagccaaccaggaagggcagcccacctatcaaggtgtactgccttccagacgaacgaagagcgattgaggaaaaggcggcggcggccggcatgagcctgtcggcctacctgctggccgtcggccagggctacaaaatcacgggcgtcgtggactatgagcacgtccgcgagctggcccgcatcaatggcgacctgggccgcctgggcggcctgctgaaactctggctcaccgacgacccgcgcacggcgcggttcggtgatgccacgatcctcgccctgctggcgaagatcgaagagaagcaggacgagcttggcaaggtcatgatgggcgtggtccgcccgagggcagagccatgacttttttagccgctaaaacggccggggggtgcgcgtgattgccaagcacgtccccatgcgctccatcaagaagagcgacttcgcggagctggtgaagtacatcaccgacgagcaaggcaagaccgatcgggccccctgcaggataaaaaaattgtagataaattttataaaatagttttatctacaatttttttatcaggaaacagctatgaccgcggccgcggcgccaagcttagaaaaatataaataagaagtagctttaagagaattaaattattaagaaaagcaaaggtgtttaaaaaataaatttttaaacacctttgcttttcttaaattataaataagataaaaaagaatcctgaataaaataaaaaggggtgtctcaaaattttattttgagacgacccctttttattctatatgtcgatgctatagctgagatcgtggaattcttgttagctaccagattcacatttaagttgtttctctaaaccacagattatcaattcaagtccaaaaagaaatgctggttctgcgccttgatgatcaaataactctattgcttgtcttaacaatggaggcattgaatctgttgttggtgtttctctttcctcttttgcaacttgatgttcttgatcctccaatacgcaacctaaagtaaaatgtcctacagcacttagtgcgtataaggcattttctaaactaaaaccctgttgacataagaatgctaattgattttctaatgtttcatattgtttttcagttggtctagttcctaaatgtactttagccccatctctatgtgataatagagcacaacgaaaagatttagcgttattcctaagaaaatcttgccatgattcaccttctaaaggacaaaagtgagtgtgatgtctatctaacatttcaatagctaaggcgtcaagtaaagctctcttattcttcacatgccaatacaacgtaggttgttctactccaagtttctgagctaactttcttgtagttagtccttctattccaacttcatttagtaattccaatgcactattgataactttacttttatcaagtctagacatcatttaatatcctcctcttcaatatatttaagtcgactgatcggatcctgatcggagctcccatggcggccggtcgatatcgatgtgtagtagcctgtgaaataagtaaggaaaaaaaagaagtaagtgttatatatgatgattattttgtagatgtagataggataatagaatccatagaaaatataggttatacagttatataaaaattactttaaaatctatcattgatagggtaaaatataaatcgtataaagttgtgtaatttttaaggaggtgtgttacagacgtccgcgagagaccttaaatatattgaagaggaggaaatacatatggtttcaagatatgttccagatatgggagatttaatatgggttgattttgatccaacaaaaggatcagaacaagcaggacatagaccagcagttgttttatcaccatttatgtataataataaaacaggaatgtgtttatgtgttccatgtacaacacaatcaaaaggatatccatttgaagttgttttatcaggacaagaaagagatggagttgcattagcagatcaagttaaatcaatagcatggagagcaagaggagcaacaaaaaaaggaacagttgcaccagaagaattacaattaataaaagcaaaaataaatgttttaataggataatgttattaagctagcataaaaataagaagcctgcatttgcaggcttcttatttttatggcgcgccgttctgaatccttagctaatggttcaacaggtaactatgacgaagatagcaccctggataagtctgtaatggattctaaggcatttaatgaagacgtgtatataaaatgtgctaatgaaaaagaaaatgcgttaaaagagcctaaaatgagttcaaatggttttgaaattgattggtagtttaatttaatatattttttctattggctatctcgatacctatagaatcttctgttcacttttgtttttgaaatataaaaaggggctttttagccccttttttttaaaactccggaggagtttcttcattcttgatactatacgtaactattttcgatttgacttcattgtcaattaagctagtaaaatcaatggttaaaaaacaaaaaacttgcatttttctacctagtaatttataattttaagtgtcgagtttaaaagtataatttaccaggaaaggagcaagttttttaataaggaaaaatttttccttttaaaattctatttcgttatatgactaattataatcaaaaaaatgaaaataaacaagaggtaaaaactgctttagagaaatgtactgataaaaaaagaaaaaatcctagatttacgtcatacatagcacctttaactactaagaaaaatattgaaaggacttccacttgtggagattatttgtttatgttgagtgatgcagacttagaacattttaaattacataaaggtaatttttgcggtaatagattttgtccaatgtgtagttggcgacttgcttgtaaggatagtttagaaatatctattcttatggagcatttaagaaaagaagaaaataaagagtttatatttttaactcttacaactccaaatgtaaaaagttatgatcttaattattctattaaacaatataataaatcttttaaaaaattaatggagcgtaaggaagttaaggatataactaaaggttatataagaaaattagaagtaacttaccaaaaggaaaaatacataacaaaggatttatggaaaataaaaaaagattattatcaaaaaaaaggacttgaaattggtgatttagaacctaattttgatacttataatcctcattttcatgtagttattgcagttaataaaagttattttacagataaaaattattatataaatcgagaaagatggttggaattatggaagtttgctactaaggatgattctataactcaagttgatgttagaaaagcaaaaattaatgattataaagaggtttacgaacttgcgaaatattcagctaaagacactgattatttaatatcgaggccagtatttgaaattttttataaagcattaaaaggcaagcaggtattagtttttagtggattttttaaagatgcacacaaattgtacaagcaaggaaaacttgatgtttataaaaagaaagatgaaattaaatatgtctatatagtttattataattggtgcaaaaaacaatatgaaaaaactagaataagggaacttacggaagatgaaaaagaagaattaaatcaagatttaatagatgaaatagaaatagattaaagtgtaactatactttatatatatatgattaaaaaaataaaaaacaacagcctattaggttgttgttttttattttctttattaatttttttaatttttagtttttagttcttttttaaaataagtttcagcctctttttcaatattttttaaagaaggagtatttgcatgaattgccttttttctaacagacttaggaaatattttaacagtatcttcttgcgccggtgattttggaacttcataacttactaatttataattattattttcttttttaattgtaacagttgcaaaagaagctgaacctgttccttcaactagtttatcatcttcaatataatattcttgacctatatagtataaatatatttttattatatttttacttttttctgaatctattattttataatcataaaaagttttaccaccaaaagaaggttgtactccttctggtccaacatatttttttactatattatctaaataatttttgggaactggtgttgtaatttgattaatcgaacaaccagttatacttaaaggaattataactataaaaatatataggattatctttttaaatttcattattggcctcctttttattaaatttatgttaccataaaaaggacataacgggaatatgtagaatatttttaatgtagacaaaattttacataaatataaagaaaggaagtgtttgtttaaattttatagcaaactatcaaaaattagggggataaaaatttatgaaaaaaaggttttcgatgttatttttatgtttaactttaatagtttgtggtttatttacaaattcggccggccaaagattgctctatgtttaagctattatatgaacttccaattctttttattgatatgggagtaatattgctttttattcttattaggttttttaaatattctatacctaaaatattgtttggagattgaagtatttcatctatattgtactttgtaagagaacttttagtatttaatagaaaattatttaaagcactatttcgtgcagaaggataggacataccctgtgacattttttcctttaaaaataatttaaattgggtaggctcttctgcaagaatttttgcaatagatttcagcaagtttatattactatattcgcttccaaaacaaagattttttactacacccaagttttctaagagacttacagcaccataggcaaaaaattcagcagaagatagactgtagataacaggaagttcaaataccaggtctactccatttagaagtgccattttggttttagtccatttgtcaactatagatggtgaacctctttgcacgaagttaccactcataactgctattacagcatcacattttgtagcagaacgagcactttcaatatgatatttatgtccattgtgaaagggattatattcaactattattccagttacgttcatagaaattttcctttctaaaatattttattccatgtcaagaactctgtttatttcattaaagaactataagtacaaagtataaggcatttgaaaaaataggctagtatattgattgattatttattttaaaatgcctaagtgaaatatatacatattataacaataaaataagtattagtgtaggatttttaaatagagtatctattttcagattaaatttttgattatttgatttacattatataatattgagtaaagtattgactagcaaaattttttgatactttaatttgtgaaatttcttatcaaaagttatatttttgaataatttttattgaaaaatacaactaaaaaggattatagtataagtgtgtgtaattttgtgttaaatttaaagggaggaaatgaacatgaaattgatgagtaaaaactttgatgagttattatcaagattaaaggaagttccaacaaaaaaagtggctgtagccgtagcacaagatgaaccagtattagaggctataaaagaagctacagaaaataacatcgcacaagcaatattggttggtgataaacaacaaatccatgaaatcgcaaagaaaataaacttggacttatctgattatgaaataatggatattaaagatccaaagaaagcaacattagaagcagtaaaattagtttctagtggtcatgcagatatgttaatgaaaggtctagttgatactgcaacattcctaagaagcgtattaaacaaagaggttggtcttagaacaggaaaattaatgtcccatgtagctgtgtttgatgtggaaggttgggatagactgttatttttaactgatgcagcatttaatacatatccagaatttaaggataaagttggaatgataaataatgcagttgtagttgctcatgcatgtggaatagatgttccaagagtagcacctatatgcccagttgaagttgtaaatacaagtatgcaatcaacagttgatgcagcattgttagctaaaatgagtgacagggggcaaattaaaggatgcgtaattgatggaccttttgccttagataatgcaatatcagaagaagcagctcatcataaaggtgttacaggatcagtagcaggtaaagctgatatattattattaccaaatatagaagcagcaaatgtaatgtataaaacattaacatatttctctaaatcaagaaatggtggacttttagtaggtacatcagcaccagtaattttaacttcaagagcagattcattcgaaactaaagttaattcaattgctcttgcagcattagttgcagcaagaaataagtaataaatcaatccataataattaatgcataattaatggagagatttatatggaatttgcaatgcactattagattctataataatttcttctgaaaattatgcattatgactgtatagaatgcattaaatttaagggggattcagaatgtcatataagctattaataatcaatccaggttcaacatcaacaaagattggtgtttacgaaggagaaaaggaactatttgaagaaactttgagacacacaaatgaagaaataaagagatatgatacaatatatgatcaatttgaatttagaaaagaagttatattaaatgttcttaaagaaaagaattttgatataaagactctaagtgctattgttggtagaggtggaatgcttagaccagttgaaggtggaacatatgcagtaaatgatgcaatggttgaagatttaaaagttggagttcaaggacctcatgcttctaaccttggcggaataattgccaagtcaattggagatgaattaaatattccatcatttatagtagatccagttgttacagatgagttagcagatgtagcaagactatctggagtaccagaactaccaagaaaaagtaaattccatgctttaaatcaaaaagcggtagctaaaagatatggaaaagaaagtggacaaggatatgaaaacctaaatcttgtagttgtacatatgggtggaggcgtttcagttggtgctcacaatcatgggaaagttgtcgatgtaaataatgcattagatggagatggcccattctcaccagaaagagctggatcagttccaattggtgatttagttaaaatgtgttttagtggaaaatatagtgaagcagaagtatatggcaaggctgtaggaaaaggtggatttgttggttatctaaacacaaatgatgtaaaaggtgttattgataagatggaagaaggagataaagaatgtgaatcaatatacaaagcatttgtttatcaaatttcaaaagcaatcggagaaatgtcagttgtattagaaggtaaagttgatcaaattatttttaccggaggaattgcatactcaccaacacttgttccagaccttaaagcaaaagttgaatggatagccccagttacagtttatcctggagaagatgaattacttgctctagctcaaggtgctataagagtacttgatggagaagaacaagctaaggtttactagtaccgttcgtataatgtatgctatacgaagttatccttagaagcaaacttaagagtgtgttgatagtgcagtatcttaaaattttgtgtataataggaattgaagttaaattagatgctaaaaatttgtaattaagaaggagggattcgtcatgttggtattccaaatgcgtaatgtagataaaacatctactgttttgaaacagactaaaaacagtgattacgcagataaataaatacgttagattaattcctaccagtgactaatcttatgactttttaaacagataactaaaattacaaacaaatcgtttaacttctgtatttatttacagatgtaatcacttcaggagtaattacatgaacaaaaatataaaatattctcaaaactttttaacgagtgaaaaagtactcaaccaaataataaaacaattgaatttaaaagaaaccgataccgtttacgaaattggaacaggtaaagggcatttaacgacgaaactggctaaaataagtaaacaggtaacgtctattgaattagacagtcatctattcaacttatcgtcagaaaaattaaaactgaacattcgtgtcactttaattcaccaagatattctacagtttcaattccctaacaaacagaggtataaaattgttgggagtattccttaccatttaagcacacaaattattaaaaaagtggtttttgaaagccatgcgtctgacatctatctgattgttgaagaaggattctacaagcgtaccttggatattcaccgaacactagggttgctcttgcacactcaagtctcgattcagcaattgcttaagctgccagcggaatgctttcatcctaaaccaaaagtaaacagtgtcttaataaaacttacccgccataccacagatgttccagataaatattggaagctatatacgtactttgtttcaaaatgggtcaatcgagaatatcgtcaactgtttactaaaaatcagtttcatcaagcaatgaaacacgccaaagtaaacaatttaagtaccattacttatgagcaagtattgtctatttttaatagttatctattatttaacgggaggaaataattctatgagtcgcttttttaaatttggaaagttacacgttactaaagggaatggagataaattattagatatactactgacagcttccaagaagctaaagaggtcataacttcgtataatgtatgctatacgaacggtagacttgacttttaatgctcatctctatataataggttgtggctaatatatagaggtgagtgatatgaaattaaatgtatcagatttactaagtgaagaagttgttacaaaggacataaatgttacagtagaagaaaagggattctatgatggaagtgaatacataaagttattagagcctctaaagtttagcggaactttaagtaaagaaggagatattcttctgttggaaggaagaattaatactttactagagctcacttgttcacgatgtctaggtaaattctcttatgctgtgaatgttgctattactgaaaaatttacaaataataacaaggaaaataaggatgatgaagccatctttatagatagtaatatcattgatattacggaaataatagaaaataacattatattaattttaccaattaagaggctttgcagcgagaattgtaaggggttatgccaacagtgcggcactaacttaaataattctaaatgtcagtgcaaaagcgatgatattgatccgagattggcaaagctaaaagatatgtttttcactgattaaggaggtgtttactgtgggaaatccagccagcagaatatcaaaagcaaaaagagactcaagaagagcacagacttttaaattaggtttaccaggtttagttgagtgtcctcagtgccatgaaatgaaacttgcacatagagtttgtaagaattgtggatattataagggtaaggaaatcatttcaactgaaaataaataaaagaaagtcatttgactttctttttttgttcatggggtctataaaagttagatcatattaagtaacaaaattaggtaacaaaggtccagattataggataggatgtgaaaatatgataattgctgtggatggtatgggaggagattttgcaccttgtgctgtagtggaaggtgtggtagaagcagttaaaaagcaaaacgtaaatataataataaccggccaaaaagagcaaattgaaaatgaattagctaaatataattatcctaaggacaaaatagatattt

SEQ ID NO: 161 - DNA, 42 bp, Artificial sequence
  Synthetic polynucleotide
  misc_feature: SN22f
tttacaaattcggccggccaaagattgctctatgtttaagct

SEQ ID NO: 162 - DNA, 43 bp, Artificial sequence
  Synthetic polynucleotide
  misc_feature: SN23r
catcaaagtttttactcatcaatttcatgttcatttcctccct

SEQ ID NO: 163 - DNA, 46 bp, Artificial sequence
  Synthetic polynucleotide
  misc_feature: SN24f
agggaggaaatgaacatgaaattgatgagtaaaaactttgatgagt

SEQ ID NO: 164 - DNA, 50 bp, Artificial sequence
  Synthetic polynucleotide
  misc_feature: SN25r
gtatagcatacattatacgaacggtactagtaaaccttagcttgttcttc

SEQ ID NO: 165 - DNA, 50 bp, Artificial sequence
  Synthetic polynucleotide
  misc_feature: SN26f
gaagaacaagctaaggtttactagtaccgttcgtataatgtatgctatac

SEQ ID NO: 166 - DNA, 45 bp, Artificial sequence
  Synthetic polynucleotide
  misc_feature: SN27r
agagatgagcattaaaagtcaagtctaccgttcgtatagcataca

SEQ ID NO: 167 - DNA, 45 bp, Artificial sequence
  Synthetic polynucleotide
  misc_feature: SN28f
tgtatgctatacgaacggtagacttgacttttaatgctcatctct

SEQ ID NO: 168 - DNA, 47 bp, Artificial sequence
  Synthetic polynucleotide
  misc_feature: SN29r
catgagattatcaaaaaggagtttaaatatctattttgtccttagga

SEQ ID NO: 169 - DNA, 47 bp, Artificial sequence
  Synthetic polynucleotide
  misc_feature: SN30f
tcctaaggacaaaatagatatttaaactcctttttgataatctcatg

SEQ ID NO: 170 - DNA, 42 bp, Artificial sequence
  Synthetic polynucleotide
  misc_feature: SN31r
agcttaaacatagagcaatctttggccggccgaatttgtaaa

SEQ ID NO: 171 - DNA, 25 bp, Artificial sequence
  Synthetic polynucleotide
  misc_feature: Og29f
agccacatccagtagattgaacttt

SEQ ID NO: 172 - DNA, 25 bp, Artificial sequence
  Synthetic polynucleotide
  misc_feature: Og30r
aattcgccctacgattaaagtggaa

SEQ ID NO: 173 - DNA, 35 bp, Artificial sequence; identical to SEQ ID NO: 141
  Synthetic polynucleotide
  misc_feature: Pfdx-F1, forward

SEQ ID NO: 174 - DNA, 38 bp, Artificial sequence; identical to SEQ ID NO: 142
  Synthetic polynucleotide
  misc_feature: Pfdx-R1, reverse

SEQ ID NO: 175 - DNA, 52 bp, Artificial sequence
  Synthetic polynucleotide
  misc_feature: aor1-F1, forward
aaaggtctcgaattcaaagatctatgtatggttatgatggtaaagtattaag

SEQ ID NO: 176 - DNA, 54 bp, Artificial sequence
  Synthetic polynucleotide
  misc_feature: aor1-R1, reverse
tttggtctcctcgagtatggatccctagaacttacctatatattcatctaatcc

SEQ ID NO: 177 - DNA, 37 bp, Artificial sequence
  Synthetic polynucleotide
  misc_feature: pETDuet-pta-ack - ack-DuetI2-R1
gggtaccttatttattttcaactatttcttttgtatc

SEQ ID NO: 178 - DNA, 36 bp, Artificial sequence
  Synthetic polynucleotide
  misc_feature: pETDuet-pta-ack - DuetI2-ack-F1
ttgaaaataaataaggtaccctcgagtctggtaaag

SEQ ID NO: 179 - DNA, 36 bp, Artificial sequence
  Synthetic polynucleotide
  misc_feature: pETDuet-pta-ack - DuetI2-pta-R1
ttttttccatatgtatatctccttcttatacttaac

SEQ ID NO: 180 - DNA, 36 bp, Artificial sequence
  Synthetic polynucleotide
  misc_feature: pETDuet-pta-ack - pta-DuetI2-F1
aggagatatacatatggaaaaaatttggagtaaggc

SEQ ID NO: 181 - DNA, 36 bp, Artificial sequence
  Synthetic polynucleotide
  misc_feature: pETDuet-tesB - DuetI2-tesB-F1
gaaatcataattaaggtaccctcgagtctggtaaag

SEQ ID NO: 182 - DNA, 36 bp, Artificial sequence
  Synthetic polynucleotide
  misc_feature: pETDuet-tesB - DuetI2-tesB-R1
cctgactcatatgtatatctccttcttatacttaac

SEQ ID NO: 183 - DNA, 36 bp, Artificial sequence
  Synthetic polynucleotide
  misc_feature: pETDuet-tesB - tesB-DuetI2-F1
aagaaggagatatacatatgagtcaggcacttaaaa

SEQ ID NO: 184 - DNA, 35 bp, Artificial sequence
  Synthetic polynucleotide
  misc_feature: pETDuet-tesB - testB-DuetI2-R1
agggtaccttaattatgatttctcataacaccttc

SEQ ID NO: 185 - DNA, 7606 bp, Artificial sequence
  Synthetic polynucleotide
  misc_feature: pDUET-pta-ack, plasmid
ggggaattgtgagcggataacaattcccctctagaaataattttgtttaactttaagaaggagatataccatgggcagcagccatcaccatcatcaccacagccaggatccgaattcgagctcggcgcgcctgcaggtcgacaagcttgcggccgcataatgcttaagtcgaacagaaagtaatcgtattgtacacggccgcataatcgaaattaatacgactcactataggggaattgtgagcggataacaattccccatcttagtatattagttaagtataagaaggagatatacatatggaaaaaatttggagtaaggcaaaggaagacaaaaaaaagattgtcttagctgaaggagaagaagaaagaactcttcaagcttgtgaaaaaataattaaagagggtattgcaaatttaatccttgtagggaatgaaaaggtaataaaagaaaaagcgtcaaaattaggtgtaagtttaaatggagcagaaatagtagatccagagatttcagataaactaaaggcatatgcagatgctttttatgaattgagaaagaagaagggaataacgccagaaaaagcggataaaatagtaagagatccaatatactttgctacaatgatggttaaacttggagatgcagatggattggtttcaggtgcggttcatactacaggcgatcttttgagaccaggacttcaaatagtaaagacagctccaggtacatcagtagtttccagtacatttataatggaagtaccaaattgtgagtatggtgacaatggtgtacttctatttgctgattgtgctgtaaatccatgcccagatagtgatcaattggcttcaattgcaataagtacagcagaaactgcaaagaacttatgtggaatggatccaaaagtagcaatgctttcattttctactaagggaagtgcaaaacacgaattagtagacaaagttagaaatgctgtagagattgcaaaaaaagctaaaccagatttaagtttagacggagaattacaattagatgcctctatcgtagaaaaggttgcaagtttaaaggctcctggaagtgaagtagcaggaaaagcaaatgtacttgtatttccagatctccaagcaggaaatataggctataaactcgttcaaagatttgcaaaagcagatgctataggacctgtatgccaaggatttgcaaaacctataaatgatttgtcaagaggatgtaattctgatgatatagtaaatgtagtagctgtaacagcagttcaagcacaagctcaaaagtaataacaaaaagcataaatgattcatttttaggaggaatattaaacatgaaaatattagtagtaaactgtggaagttcatctttaaaatatcaacttattgatatgcaagatgaaagtgttgtagcaaagggtcttgtagaaagaataggaatggacggttcaattttaacacacaaagttaatggagaaaagtttgttacagagcaaccaatggaagaccacaaagttgctatacaattagtattaaatgctcttgtagataaaaaacatggtgtaataaaagacatgtcagaaatatccgctgtaggacatagagttttgcacggtggaaagaaatatgcagcatccattcttattgacgaaaatgtaatgaaagcaatagaagaatgtatcccactaggaccactacataatccagctaatataatgggaatagatgcttgtaaaaaattaatgccaaatactccaatggtagcagtatttgatacagcatttcatcagacaatgccagattatgcttatacttatgcaataccttatgatatatctgaaaagtatgatatcagaaaatatggttttcatggaacttctcatagattcgtttcaattgaagcagctaaattattaaagaaagatccaaaagatcttaagttaataacttgtcatttaggaaatggagctagcatatgtgcagtaaaccaaggaaaagcagtagatacaactatgggacttactcctcttgcaggacttgtaatgggaactagatgcggtgatatagatccagctatagtaccatttgtaatgaaaagaacaggcatgtctgtagatgaagtggataccttaatgaataaaaagtcaggaatacttggagtatcaggagtaagcagtgattttagagatgtagaagaagctgcaaattcaggaaatgatagagcaaaacttgcattaaatatgtattatcacaaagttaaatctttcataggagcttatgttgcagttttaaatggagcagatgctataatatttacggcaggacttggagaaaattcagcaactagcagatctgctatatgtaatggattaagctattttggaattaaaatagatgaagaaaagaataagaaaaggggagaggcactagaaataagcacacctgattcaaagataaaagtattagtaattcctacaaatgaagaacttatgatagctagggatacaaaagaaatagttgaaaataaataaggtaccctcgagtctggtaaagaaaccgctgctgcgaaatttgaacgccagcacatggactcgtctactagcgcagcttaattaacctaggctgctgccaccgctgagcaataactagcataaccccttggggcctctaaacgggtcttgaggggttttttgctgaaaggaggaactatatccggattggcgaatgggacgcgccctgtagcggcgcattaagcgcggcgggtgtggtggttacgcgcagcgtgaccgctacacttgccagcgccctagcgcccgctcctttcgctttcttcccttcctttctcgccacgttcgccggctttccccgtcaagctctaaatcgggggctccctttagggttccgatttagtgctttacggcacctcgaccccaaaaaacttgattagggtgatggttcacgtagtgggccatcgccctgatagacggtttttcgccctttgacgttggagtccacgttctttaatagtggactcttgttccaaactggaacaacactcaaccctatctcggtctattcttttgatttataagggattttgccgatttcggcctattggttaaaaaatgagctgatttaacaaaaatttaacgcgaattttaacaaaatattaacgtttacaatttctggcggcacgatggcatgagattatcaaaaaggatcttcacctagatccttttaaattaaaaatgaagttttaaatcaatctaaagtatatatgagtaaacttggtctgacagttaccaatgcttaatcagtgaggcacctatctcagcgatctgtctatttcgttcatccatagttgcctgactccccgtcgtgtagataactacgatacgggagggcttaccatctggccccagtgctgcaatgataccgcgagacccacgctcaccggctccagatttatcagcaataaaccagccagccggaagggccgagcgcagaagtggtcctgcaactttatccgcctccatccagtctattaattgttgccgggaagctagagtaagtagttcgccagttaatagtttgcgcaacgttgttgccattgctacaggcatcgtggtgtcacgctcgtcgtttggtatggcttcattcagctccggttcccaacgatcaaggcgagttacatgatcccccatgttgtgcaaaaaagcggttagctccttcggtcctccgatcgttgtcagaagtaagttggccgcagtgttatcactcatggttatggcagcactgcataattctcttactgtcatgccatccgtaagatgcttttctgtgactggtgagtactcaaccaagtcattctgagaatagtgtatgcggcgaccgagttgctcttgcccggcgtcaatacgggataataccgcgccacatagcagaactttaaaagtgctcatcattggaaaacgttcttcggggcgaaaactctcaaggatcttaccgctgttgagatccagttcgatgtaacccactcgtgcacccaactgatcttcagcatcttttactttcaccagcgtttctgggtgagcaaaaacaggaaggcaaaatgccgcaaaaaagggaataagggcgacacggaaatgttgaatactcatactcttcctttttcaatcatgattgaagcatttatcagggttattgtctcatgagcggatacatatttgaatgtatttagaaaaataaacaaataggtcatgaccaaaatcccttaacgtgagttttcgttccactgagcgtcagaccccgtagaaaagatcaaaggatcttcttgagatcctttttttctgcgcgtaatctgctgcttgcaaacaaaaaaaccaccgctaccagcggtggtttgtttgccggatcaagagctaccaactctttttccgaaggtaactggcttcagcagagcgcagataccaaatactgtccttctagtgtagccgtagttaggccaccacttcaagaactctgtagcaccgcctacatacctcgctctgctaatcctgttaccagtggctgctgccagtggcgataagtcgtgtcttaccgggttggactcaagacgatagttaccggataaggcgcagcggtcgggctgaacggggggttcgtgcacacagcccagcttggagcgaacgacctacaccgaactgagatacctacagcgtgagctatgagaaagcgccacgcttcccgaagggagaaaggcggacaggtatccggtaagcggcagggtcggaacaggagagcgcacgagggagcttccagggggaaacgcctggtatctttatagtcctgtcgggtttcgccacctctgacttgagcgtcgatttttgtgatgctcgtcaggggggcggagcctatggaaaaacgccagcaacgcggcctttttacggttcctggccttttgctggccttttgctcacatgttctttcctgcgttatcccctgattctgtggataaccgtattaccgcctttgagtgagctgataccgctcgccgcagccgaacgaccgagcgcagcgagtcagtgagcgaggaagcggaagagcgcctgatgcggtattttctccttacgcatctgtgcggtatttcacaccgcatatatggtgcactctcagtacaatctgctctgatgccgcatagttaagccagtatacactccgctatcgctacgtgactgggtcatggctgcgccccgacacccgccaacacccgctgacgcgccctgacgggcttgtctgctcccggcatccgcttacagacaagctgtgaccgtctccgggagctgcatgtgtcagaggttttcaccgtcatcaccgaaacgcgcgaggcagctgcggtaaagctcatcagcgtggtcgtgaagcgattcacagatgtctgcctgttcatccgcgtccagctcgttgagtttctccagaagcgttaatgtctggcttctgataaagcgggccatgttaagggcggttttttcctgtttggtcactgatgcctccgtgtaagggggatttctgttcatgggggtaatgataccgatgaaacgagagaggatgctcacgatacgggttactgatgatgaacatgcccggttactggaacgttgtgagggtaaacaactggcggtatggatgcggcgggaccagagaaaaatcactcagggtcaatgccagcgcttcgttaatacagatgtaggtgttccacagggtagccagcagcatcctgcgatgcagatccggaacataatggtgcagggcgctgacttccgcgtttccagactttacgaaacacggaaaccgaagaccattcatgttgttgctcaggtcgcagacgttttgcagcagcagtcgcttcacgttcgctcgcgtatcggtgattcattctgctaaccagtaaggcaaccccgccagcctagccgggtcctcaacgacaggagcacgatcatgctagtcatgccccgcgcccaccggaaggagctgactgggttgaaggctctcaagggcatcggtcgagatcccggtgcctaatgagtgagctaacttacattaattgcgttgcgctcactgcccgctttccagtcgggaaacctgtcgtgccagctgcattaatgaatcggccaacgcgcggggagaggcggtttgcgtattgggcgccagggtggtttttcttttcaccagtgagacgggcaacagctgattgcccttcaccgcctggccctgagagagttgcagcaagcggtccacgctggtttgccccagcaggcgaaaatcctgtttgatggtggttaacggcgggatataacatgagctgtcttcggtatcgtcgtatcccactaccgagatgtccgcaccaacgcgcagcccggactcggtaatggcgcgcattgcgcccagcgccatctgatcgttggcaaccagcatcgcagtgggaacgatgccctcattcagcatttgcatggtttgttgaaaaccggacatggcactccagtcgccttcccgttccgctatcggctgaatttgattgcgagtgagatatttatgccagccagccagacgcagacgcgccgagacagaacttaatgggcccgctaacagcgcgatttgctggtgacccaatgcgaccagatgctccacgcccagtcgcgtaccgtcttcatgggagaaaataatactgttgatgggtgtctggtcagagacatcaagaaataacgccggaacattagtgcaggcagcttccacagcaatggcatcctggtcatccagcggatagttaatgatcagcccactgacgcgttgcgcgagaagattgtgcaccgccgctttacaggcttcgacgccgcttcgttctaccatcgacaccaccacgctggcacccagttgatcggcgcgagatttaatcgccgcgacaatttgcgacggcgcgtgcagggccagactggaggtggcaacgccaatcagcaacgactgtttgcccgccagttgttgtgccacgcggttgggaatgtaattcagctccgccatcgccgcttccactttttcccgcgttttcgcagaaacgtggctggcctggttcaccacgcgggaaacggtctgataagagacaccggcatactctgcgacatcgtataacgttactggtttcacattcaccaccctgaattgactctcttccgggcgctatcatgccataccgcgaaaggttttgcgccattcgatggtgtccgggatctcgacgctctcccttatgcgactcctgcattaggaagcagcccagtagtaggttgaggccgttgagcaccgccgccgcaaggaatggtgcatgcaaggagatggcgcccaacagtcccccggccacggggcctgccaccatacccacgccgaaacaagcgctcatgagcccgaagtggcgagcccgatcttccccatcggtgatgtcggcgatataggcgccagcaaccgcacctgtggcgccggtgatgccggccacgatgcgtccggcgtagaggatcgagatcgatctcgatcccgcgaaattaatacgactcactata

SEQ ID NO: 186 - DNA, 7492 bp, Artificial sequence
  Synthetic polynucleotide
  misc_feature: pDUET-ptb-buk, plasmid
ggggaattgtgagcggataacaattcccctctagaaataattttgtttaactttaagaaggagatataccatgggcagcagccatcaccatcatcaccacagccaggatccgaattcgagctcggcgcgcctgcaggtcgacaagcttgcggccgcataatgcttaagtcgaacagaaagtaatcgtattgtacacggccgcataatcgaaattaatacgactcactataggggaattgtgagcggataacaattccccatcttagtatattagttaagtataagaaggagatatacatatgagtaaaaactttgatgagttattatcaagattaaaggaagttccaacaaaaaaagtggctgtagccgtagcacaagatgaaccagtattagaggctataaaagaagctacagaaaataacatcgcacaagcaatattggttggtgataaacaacaaatccatgaaatcgcaaagaaaataaacttggacttatctgattatgaaataatggatattaaagatccaaagaaagcaacattagaagcagtaaaattagtttctagtggtcatgcagatatgttaatgaaaggtctagttgatactgcaacattcctaagaagcgtattaaacaaagaggttggtcttagaacaggaaaattaatgtcccatgtagctgtgtttgatgtggaaggttgggatagactgttatttttaactgatgcagcatttaatacatatccagaatttaaggataaagttggaatgataaataatgcagttgtagttgctcatgcatgtggaatagatgttccaagagtagcacctatatgcccagttgaagttgtaaatacaagtatgcaatcaacagttgatgcagcattgttagctaaaatgagtgacagggggcaaattaaaggatgcgtaattgatggaccttttgccttagataatgcaatatcagaagaagcagctcatcataaaggtgttacaggatcagtagcaggtaaagctgatatattattattaccaaatatagaagcagcaaatgtaatgtataaaacattaacatatttctctaaatcaagaaatggtggacttttagtaggtacatcagcaccagtaattttaacttcaagagcagattcattcgaaactaaagttaattcaattgctcttgcagcattagttgcagcaagaaataagtaataaatcaatccataataattaatgcataattaatggagagatttatatggaatttgcaatgcactattagattctataataatttcttctgaaaattatgcattatgactgtatagaatgcattaaatttaagggggattcagaatgtcatataagctattaataatcaatccaggttcaacatcaacaaagattggtgtttacgaaggagaaaaggaactatttgaagaaactttgagacacacaaatgaagaaataaagagatatgatacaatatatgatcaatttgaatttagaaaagaagttatattaaatgttcttaaagaaaagaattttgatataaagactctaagtgctattgttggtagaggtggaatgcttagaccagttgaaggtggaacatatgcagtaaatgatgcaatggttgaagatttaaaagttggagttcaaggacctcatgcttctaaccttggcggaataattgccaagtcaattggagatgaattaaatattccatcatttatagtagatccagttgttacagatgagttagcagatgtagcaagactatctggagtaccagaactaccaagaaaaagtaaattccatgctttaaatcaaaaagcggtagctaaaagatatggaaaagaaagtggacaaggatatgaaaacctaaatcttgtagttgtacatatgggtggaggcgtttcagttggtgctcacaatcatgggaaagttgtcgatgtaaataatgcattagatggagatggcccattctcaccagaaagagctggatcagttccaattggtgatttagttaaaatgtgttttagtggaaaatatagtgaagcagaagtatatggcaaggctgtaggaaaaggtggatttgttggttatctaaacacaaatgatgtaaaaggtgttattgataagatggaagaaggagataaagaatgtgaatcaatatacaaagcatttgtttatcaaatttcaaaagcaatcggagaaatgtcagttgtattagaaggtaaagttgatcaaattatttttaccggaggaattgcatactcaccaacacttgttccagaccttaaagcaaaagttgaatggatagccccagttacagtttatcctggagaagatgaattacttgctctagctcaaggtgctataagagtacttgatggagaagaacaagctaaggtttactaggtaccctcgagtctggtaaagaaaccgctgctgcgaaatttgaacgccagcacatggactcgtctactagcgcagcttaattaacctaggctgctgccaccgctgagcaataactagcataaccccttggggcctctaaacgggtcttgaggggttttttgctgaaaggaggaactatatccggattggcgaatgggacgcgccctgtagcggcgcattaagcgcggcgggtgtggtggttacgcgcagcgtgaccgctacacttgccagcgccctagcgcccgctcctttcgctttcttcccttcctttctcgccacgttcgccggctttccccgtcaagctctaaatcgggggctccctttagggttccgatttagtgctttacggcacctcgaccccaaaaaacttgattagggtgatggttcacgtagtgggccatcgccctgatagacggtttttcgccctttgacgttggagtccacgttctttaatagtggactcttgttccaaactggaacaacactcaaccctatctcggtctattcttttgatttataagggattttgccgatttcggcctattggttaaaaaatgagctgatttaacaaaaatttaacgcgaattttaacaaaatattaacgtttacaatttctggcggcacgatggcatgagattatcaaaaaggatcttcacctagatccttttaaattaaaaatgaagttttaaatcaatctaaagtatatatgagtaaacttggtctgacagttaccaatgcttaatcagtgaggcacctatctcagcgatctgtctatttcgttcatccatagttgcctgactccccgtcgtgtagataactacgatacgggagggcttaccatctggccccagtgctgcaatgataccgcgagacccacgctcaccggctccagatttatcagcaataaaccagccagccggaagggccgagcgcagaagtggtcctgcaactttatccgcctccatccagtctattaattgttgccgggaagctagagtaagtagttcgccagttaatagtttgcgcaacgttgttgccattgctacaggcatcgtggtgtcacgctcgtcgtttggtatggcttcattcagctccggttcccaacgatcaaggcgagttacatgatcccccatgttgtgcaaaaaagcggttagctccttcggtcctccgatcgttgtcagaagtaagttggccgcagtgttatcactcatggttatggcagcactgcataattctcttactgtcatgccatccgtaagatgcttttctgtgactggtgagtactcaaccaagtcattctgagaatagtgtatgcggcgaccgagttgctcttgcccggcgtcaatacgggataataccgcgccacatagcagaactttaaaagtgctcatcattggaaaacgttcttcggggcgaaaactctcaaggatcttaccgctgttgagatccagttcgatgtaacccactcgtgcacccaactgatcttcagcatcttttactttcaccagcgtttctgggtgagcaaaaacaggaaggcaaaatgccgcaaaaaagggaataagggcgacacggaaatgttgaatactcatactcttcctttttcaatcatgattgaagcatttatcagggttattgtctcatgagcggatacatatttgaatgtatttagaaaaataaacaaataggtcatgaccaaaatcccttaacgtgagttttcgttccactgagcgtcagaccccgtagaaaagatcaaaggatcttcttgagatcctttttttctgcgcgtaatctgctgcttgcaaacaaaaaaaccaccgctaccagcggtggtttgtttgccggatcaagagctaccaactctttttccgaaggtaactggcttcagcagagcgcagataccaaatactgtccttctagtgtagccgtagttaggccaccacttcaagaactctgtagcaccgcctacatacctcgctctgctaatcctgttaccagtggctgctgccagtggcgataagtcgtgtcttaccgggttggactcaagacgatagttaccggataaggcgcagcggtcgggctgaacggggggttcgtgcacacagcccagcttggagcgaacgacctacaccgaactgagatacctacagcgtgagctatgagaaagcgccacgcttcccgaagggagaaaggcggacaggtatccggtaagcggcagggtcggaacaggagagcgcacgagggagcttccagggggaaacgcctggtatctttatagtcctgtcgggtttcgccacctctgacttgagcgtcgatttttgtgatgctcgtcaggggggcggagcctatggaaaaacgccagcaacgcggcctttttacggttcctggccttttgctggccttttgctcacatgttctttcctgcgttatcccctgattctgtggataaccgtattaccgcctttgagtgagctgataccgctcgccgcagccgaacgaccgagcgcagcgagtcagtgagcgaggaagcggaagagcgcctgatgcggtattttctccttacgcatctgtgcggtatttcacaccgcatatatggtgcactctcagtacaatctgctctgatgccgcatagttaagccagtatacactccgctatcgctacgtgactgggtcatggctgcgccccgacacccgccaacacccgctgacgcgccctgacgggcttgtctgctcccggcatccgcttacagacaagctgtgaccgtctccgggagctgcatgtgtcagaggttttcaccgtcatcaccgaaacgcgcgaggcagctgcggtaaagctcatcagcgtggtcgtgaagcgattcacagatgtctgcctgttcatccgcgtccagctcgttgagtttctccagaagcgttaatgtctggcttctgataaagcgggccatgttaagggcggttttttcctgtttggtcactgatgcctccgtgtaagggggatttctgttcatgggggtaatgataccgatgaaacgagagaggatgctcacgatacgggttactgatgatgaacatgcccggttactggaacgttgtgagggtaaacaactggcggtatggatgcggcgggaccagagaaaaatcactcagggtcaatgccagcgcttcgttaatacagatgtaggtgttccacagggtagccagcagcatcctgcgatgcagatccggaacataatggtgcagggcgctgacttccgcgtttccagactttacgaaacacggaaaccgaagaccattcatgttgttgctcaggtcgcagacgttttgcagcagcagtcgcttcacgttcgctcgcgtatcggtgattcattctgctaaccagtaaggcaaccccgccagcctagccgggtcctcaacgacaggagcacgatcatgctagtcatgccccgcgcccaccggaaggagctgactgggttgaaggctctcaagggcatcggtcgagatcccggtgcctaatgagtgagctaacttacattaattgcgttgcgctcactgcccgctttccagtcgggaaacctgtcgtgccagctgcattaatgaatcggccaacgcgcggggagaggcggtttgcgtattgggcgccagggtggtttttcttttcaccagtgagacgggcaacagctgattgcccttcaccgcctggccctgagagagttgcagcaagcggtccacgctggtttgccccagcaggcgaaaatcctgtttgatggtggttaacggcgggatataacatgagctgtcttcggtatcgtcgtatcccactaccgagatgtccgcaccaacgcgcagcccggactcggtaatggcgcgcattgcgcccagcgccatctgatcgttggcaaccagcatcgcagtgggaacgatgccctcattcagcatttgcatggtttgttgaaaaccggacatggcactccagtcgccttcccgttccgctatcggctgaatttgattgcgagtgagatatttatgccagccagccagacgcagacgcgccgagacagaacttaatgggcccgctaacagcgcgatttgctggtgacccaatgcgaccagatgctccacgcccagtcgcgtaccgtcttcatgggagaaaataatactgttgatgggtgtctggtcagagacatcaagaaataacgccggaacattagtgcaggcagcttccacagcaatggcatcctggtcatccagcggatagttaatgatcagcccactgacgcgttgcgcgagaagattgtgcaccgccgctttacaggcttcgacgccgcttcgttctaccatcgacaccaccacgctggcacccagttgatcggcgcgagatttaatcgccgcgacaatttgcgacggcgcgtgcagggccagactggaggtggcaacgccaatcagcaacgactgtttgcccgccagttgttgtgccacgcggttgggaatgtaattcagctccgccatcgccgcttccactttttcccgcgttttcgcagaaacgtggctggcctggttcaccacgcgggaaacggtctgataagagacaccggcatactctgcgacatcgtataacgttactggtttcacattcaccaccctgaattgactctcttccgggcgctatcatgccataccgcgaaaggttttgcgccattcgatggtgtccgggatctcgacgctctcccttatgcgactcctgcattaggaagcagcccagtagtaggttgaggccgttgagcaccgccgccgcaaggaatggtgcatgcaaggagatggcgcccaacagtcccccggccacggggcctgccaccatacccacgccgaaacaagcgctcatgagcccgaagtggcgagcccgatcttccccatcggtgatgtcggcgatataggcgccagcaaccgcacctgtggcgccggtgatgccggccacgatgcgtccggcgtagaggatcgagatcgatctcgatcccgcgaaattaatacgactcactata

SEQ ID NO: 187 - DNA, 6233 bp, Artificial sequence
  Synthetic polynucleotide
  misc_feature: pDUET-tesB, plasmid
ggggaattgtgagcggataacaattcccctctagaaataattttgtttaactttaagaaggagatataccatgggcagcagccatcaccatcatcaccacagccaggatccgaattcgagctcggcgcgcctgcaggtcgacaagcttgcggccgcataatgcttaagtcgaacagaaagtaatcgtattgtacacggccgcataatcgaaattaatacgactcactataggggaattgtgagcggataacaattccccatcttagtatattagttaagtataagaaggagatatacatatgagtcaggcacttaaaaatttacttactttacttaatcttgaaaaaatagaagaaggtttatttagaggacagtcagaagatttaggattaagacaagtatttggaggtcaagtagttggtcaggcactttatgcagctaaagaaactgtacctgaagaaagacttgttcatagttttcattcttattttcttagacctggagattctaaaaaaccaattatatatgatgtagaaactcttagagatggaaattcatttagtgcaagaagagttgcagctattcaaaatggtaaacctatattttacatgacagcttcttttcaagcaccagaagctggatttgaacatcagaaaactatgccttcagcacctgctccagatggattaccatcagaaacacaaatagcacagagtttagctcatttacttcctccagtacttaaagataaatttatttgtgatagacctttagaagttagaccagttgaatttcataatcctcttaaaggacatgtagcagaaccacatagacaagtttggataagagctaatggaagtgtaccagatgatcttagagttcatcagtatcttcttggttatgcatctgatttaaattttcttcctgtagctttacaaccacatggaataggttttcttgaacctggaatacagatagcaactatagatcattcaatgtggtttcatagaccatttaatcttaatgaatggcttctttatagtgtagaatctacatcagcaagttctgctagaggatttgttaggggtgaattttatactcaagatggagtacttgttgctagtacagtacaggaaggtgttatgagaaatcataattaaggtaccctcgagtctggtaaagaaaccgctgctgcgaaatttgaacgccagcacatggactcgtctactagcgcagcttaattaacctaggctgctgccaccgctgagcaataactagcataaccccttggggcctctaaacgggtcttgaggggttttttgctgaaaggaggaactatatccggattggcgaatgggacgcgccctgtagcggcgcattaagcgcggcgggtgtggtggttacgcgcagcgtgaccgctacacttgccagcgccctagcgcccgctcctttcgctttcttcccttcctttctcgccacgttcgccggctttccccgtcaagctctaaatcgggggctccctttagggttccgatttagtgctttacggcacctcgaccccaaaaaacttgattagggtgatggttcacgtagtgggccatcgccctgatagacggtttttcgccctttgacgttggagtccacgttctttaatagtggactcttgttccaaactggaacaacactcaaccctatctcggtctattcttttgatttataagggattttgccgatttcggcctattggttaaaaaatgagctgatttaacaaaaatttaacgcgaattttaacaaaatattaacgtttacaatttctggcggcacgatggcatgagattatcaaaaaggatcttcacctagatccttttaaattaaaaatgaagttttaaatcaatctaaagtatatatgagtaaacttggtctgacagttaccaatgcttaatcagtgaggcacctatctcagcgatctgtctatttcgttcatccatagttgcctgactccccgtcgtgtagataactacgatacgggagggcttaccatctggccccagtgctgcaatgataccgcgagacccacgctcaccggctccagatttatcagcaataaaccagccagccggaagggccgagcgcagaagtggtcctgcaactttatccgcctccatccagtctattaattgttgccgggaagctagagtaagtagttcgccagttaatagtttgcgcaacgttgttgccattgctacaggcatcgtggtgtcacgctcgtcgtttggtatggcttcattcagctccggttcccaacgatcaaggcgagttacatgatcccccatgttgtgcaaaaaagcggttagctccttcggtcctccgatcgttgtcagaagtaagttggccgcagtgttatcactcatggttatggcagcactgcataattctcttactgtcatgccatccgtaagatgcttttctgtgactggtgagtactcaaccaagtcattctgagaatagtgtatgcggcgaccgagttgctcttgcccggcgtcaatacgggataataccgcgccacatagcagaactttaaaagtgctcatcattggaaaacgttcttcggggcgaaaactctcaaggatcttaccgctgttgagatccagttcgatgtaacccactcgtgcacccaactgatcttcagcatcttttactttcaccagcgtttctgggtgagcaaaaacaggaaggcaaaatgccgcaaaaaagggaataagggcgacacggaaatgttgaatactcatactcttcctttttcaatcatgattgaagcatttatcagggttattgtctcatgagcggatacatatttgaatgtatttagaaaaataaacaaataggtcatgaccaaaatcccttaacgtgagttttcgttccactgagcgtcagaccccgtagaaaagatcaaaggatcttcttgagatcctttttttctgcgcgtaatctgctgcttgcaaacaaaaaaaccaccgctaccagcggtggtttgtttgccggatcaagagctaccaactctttttccgaaggtaactggcttcagcagagcgcagataccaaatactgtccttctagtgtagccgtagttaggccaccacttcaagaactctgtagcaccgcctacatacctcgctctgctaatcctgttaccagtggctgctgccagtggcgataagtcgtgtcttaccgggttggactcaagacgatagttaccggataaggcgcagcggtcgggctgaacggggggttcgtgcacacagcccagcttggagcgaacgacctacaccgaactgagatacctacagcgtgagctatgagaaagcgccacgcttcccgaagggagaaaggcggacaggtatccggtaagcggcagggtcggaacaggagagcgcacgagggagcttccagggggaaacgcctggtatctttatagtcctgtcgggtttcgccacctctgacttgagcgtcgatttttgtgatgctcgtcaggggggcggagcctatggaaaaacgccagcaacgcggcctttttacggttcctggccttttgctggccttttgctcacatgttctttcctgcgttatcccctgattctgtggataaccgtattaccgcctttgagtgagctgataccgctcgccgcagccgaacgaccgagcgcagcgagtcagtgagcgaggaagcggaagagcgcctgatgcggtattttctccttacgcatctgtgcggtatttcacaccgcatatatggtgcactctcagtacaatctgctctgatgccgcatagttaagccagtatacactccgctatcgctacgtgactgggtcatggctgcgccccgacacccgccaacacccgctgacgcgccctgacgggcttgtctgctcccggcatccgcttacagacaagctgtgaccgtctccgggagctgcatgtgtcagaggttttcaccgtcatcaccgaaacgcgcgaggcagctgcggtaaagctcatcagcgtggtcgtgaagcgattcacagatgtctgcctgttcatccgcgtccagctcgttgagtttctccagaagcgttaatgtctggcttctgataaagcgggccatgttaagggcggttttttcctgtttggtcactgatgcctccgtgtaagggggatttctgttcatgggggtaatgataccgatgaaacgagagaggatgctcacgatacgggttactgatgatgaacatgcccggttactggaacgttgtgagggtaaacaactggcggtatggatgcggcgggaccagagaaaaatcactcagggtcaatgccagcgcttcgttaatacagatgtaggtgttccacagggtagccagcagcatcctgcgatgcagatccggaacataatggtgcagggcgctgacttccgcgtttccagactttacgaaacacggaaaccgaagaccattcatgttgttgctcaggtcgcagacgttttgcagcagcagtcgcttcacgttcgctcgcgtatcggtgattcattctgctaaccagtaaggcaaccccgccagcctagccgggtcctcaacgacaggagcacgatcatgctagtcatgccccgcgcccaccggaaggagctgactgggttgaaggctctcaagggcatcggtcgagatcccggtgcctaatgagtgagctaacttacattaattgcgttgcgctcactgcccgctttccagtcgggaaacctgtcgtgccagctgcattaatgaatcggccaacgcgcggggagaggcggtttgcgtattgggcgccagggtggtttttcttttcaccagtgagacgggcaacagctgattgcccttcaccgcctggccctgagagagttgcagcaagcggtccacgctggtttgccccagcaggcgaaaatcctgtttgatggtggttaacggcgggatataacatgagctgtcttcggtatcgtcgtatcccactaccgagatgtccgcaccaacgcgcagcccggactcggtaatggcgcgcattgcgcccagcgccatctgatcgttggcaaccagcatcgcagtgggaacgatgccctcattcagcatttgcatggtttgttgaaaaccggacatggcactccagtcgccttcccgttccgctatcggctgaatttgattgcgagtgagatatttatgccagccagccagacgcagacgcgccgagacagaacttaatgggcccgctaacagcgcgatttgctggtgacccaatgcgaccagatgctccacgcccagtcgcgtaccgtcttcatgggagaaaataatactgttgatgggtgtctggtcagagacatcaagaaataacgccggaacattagtgcaggcagcttccacagcaatggcatcctggtcatccagcggatagttaatgatcagcccactgacgcgttgcgcgagaagattgtgcaccgccgctttacaggcttcgacgccgcttcgttctaccatcgacaccaccacgctggcacccagttgatcggcgcgagatttaatcgccgcgacaatttgcgacggcgcgtgcagggccagactggaggtggcaacgccaatcagcaacgactgtttgcccgccagttgttgtgccacgcggttgggaatgtaattcagctccgccatcgccgcttccactttttcccgcgttttcgcagaaacgtggctggcctggttcaccacgcgggaaacggtctgataagagacaccggcatactctgcgacatcgtataacgttactggtttcacattcaccaccctgaattgactctcttccgggcgctatcatgccataccgcgaaaggttttgcgccattcgatggtgtccgggatctcgacgctctcccttatgcgactcctgcattaggaagcagcccagtagtaggttgaggccgttgagcaccgccgccgcaaggaatggtgcatgcaaggagatggcgcccaacagtcccccggccacggggcctgccaccatacccacgccgaaacaagcgctcatgagcccgaagtggcgagcccgatcttccccatcggtgatgtcggcgatataggcgccagcaaccgcacctgtggcgccggtgatgccggccacgatgcgtccggcgtagaggatcgagatcgatctcgatcccgcgaaattaatacgactcactata

SEQ ID NO: 188 - DNA, 3120 bp, Artificial sequence
  Synthetic polynucleotide
  misc_feature: codon optimized gene cassette containing the Wood-Ljungdahl promoter in front of the genes meaB, hcmA and hcmB
atgacttatgtaccatcatcagcacttttagaacaacttagagcaggaaatacttgggctttaggaagacttatatcaagagcagaagctggagttgcagaagctagacctgcacttgctgaagtatatagacatgcaggttcagctcatgttataggtttaacaggagtaccaggatctggtaaatcaactcttgtagcaaaacttacagcagctcttagaaaaagaggagaaaaagttggtatagtagctattgatcctagttctccatatagtggaggagcaatacttggagatagaattagaatgactgaattagcaaatgattcaggagtatttataagaagtatggcaactagaggtgctactggaggaatggctagagcagctcttgatgcagttgatttacttgatgtagctggatatcatactattattttagaaacagttggagtaggtcaagatgaagttgaagtagcacatgcttctgatactacagtagttgtatcagcacctggacttggtgatgaaatacaggcaattaaagctggagttttagaaattgctgatattcatgttgtaagtaaatgtgatagagatgatgcaaatagaactcttacagatcttaaacaaatgcttactttaggaacaatggtaggacctaaaagagcatgggctataccagttgtaggagtttcaagttatacaggagaaggtgtagatgatttacttggtagaattgcagctcatagacaagcaactgctgatacagaacttggaagagaaagaagaagaagagtagctgaatttagacttcaaaaaactgcagaaacattacttttagaaagatttactacaggagcacagcctttttcaccagcattagctgatagtctttctaatagagctagtgatccttatgcagctgcaagagaattaatagctagaactataagaaaagaatattctaatgatcttgcatgtgctaaacttactataacatggttagaaccacaaattaaaagtcaacttcagtctgaaagaaaagattgggaagcaaatgaagttggagcatttcttaaaaaagcacctgaaagaaaagaacaatttcatacaattggagattttccagtacagagaacttatacagctgcagatatagcagatactcctcttgaagatattggtttacctggaagatatccatttactagaggaccttatccaacaatgtatagaagtagaacttggacaatgagacaaatagctggatttggtactggagaagatacaaataaaagatttaaatatcttatagcacagggtcagactggaatatcaacagattttgatatgcctacattaatgggatatgattcagatcatccaatgagtgatggtgaagttggaagagaaggtgtagctatagatacacttgcagatatggaagcacttcttgctgatattgatttagaaaaaatttcagttagttttactataaatccaagtgcatggattcttttagcaatgtatgtagctttaggtgaaaaaagaggttatgatcttaataaactttctggaacagtacaagctgatatacttaaagaatatatggcacagaaagaatatatttatcctatagctccaagtgttagaattgtaagagatataattacttattctgcaaaaaatcttaaaagatataatcctattaatatttctggatatcatatatcagaagctggttcttcaccattacaagaagctgcatttactcttgcaaatcttattacttatgtaaatgaagtaactaaaacaggaatgcatgtagatgaatttgcacctagattagcatttttctttgttagtcaaggagatttctttgaagaagtagcaaaatttagagctttaagaagatgttatgctaaaataatgaaagaaagatttggagcaagaaatcctgaatctatgagacttagatttcattgtcaaactgctgcagctactcttacaaaaccacagtatatggttaatgttgtaagaacaagtcttcaagcattatctgctgtattgggaggagcacaaagtcttcatactaatggatatgatgaagcatttgctatacctactgaagatgcaatgaaaatggctcttagaacacaacagattatagctgaagaatctggagttgcagatgtaatagatcctcttggaggaagttattatgttgaagcattaactacagaatatgaaaagaaaatatttgaaattcttgaagaagtagaaaaaagaggtggaactattaaacttattgaacaaggatggtttcaaaaacagatagcagattttgcttatgaaactgcacttagaaaacaatcaggacagaaacctgttataggtgtaaatagatttgttgaaaatgaagaagatgtaaaaattgaaatacatccttatgataatactacagctgaaagacaaatatcaagaactagaagagttagagcagaaagagatgaagcaaaagtacaagctatgcttgatcagttagttgcagtagctaaagatgaaagtcagaatcttatgcctcttactattgaattagtaaaagcaggagctacaatgggtgatattgtagaaaaacttaaaggtatttggggaacttatagagaaacaccagtattttaagcactagttggagagcttcccacgatggatcagattcctattagagtattattagcaaaagtaggtttagatggacatgatagaggtgtaaaagttgtagcaagagcattaagagatgctggaatggatgtaatatatagtggtcttcatagaactcctgaagaagtagttaatacagcaattcaagaagatgtagatgttttaggagttagtttactttctggtgtacagcttactgtttttcctaaaatttttaaattacttgatgaaagaggagctggtgatttaatagtaattgctggaggagtaatgccagatgaagatgcagctgcaataagaaaacttggagtaagagaagttttacttcaagatacaccaccacaggcaataatagattcaataagaagtttagtagcagcaagaggagcaagataa

SEQ ID NO: 189 - protein, 894 aa, Artificial sequence
  Synthetic polypeptide
  MISC_FEATURE: hcmA and meaB fusion
MTYVPSSALLEQLRAGNTWALGRLISRAEAGVAEARPALAEVYRHAGSAHVIGLTGVPGSGKSTLVAKLTAALRKRGEKVGIVAIDPSSPYSGGAILGDRIRMTELANDSGVFIRSMATRGATGGMARAALDAVDLLDVAGYHTIILETVGVGQDEVEVAHASDTTVVVSAPGLGDEIQAIKAGVLEIADIHVVSKCDRDDANRTLTDLKQMLTLGTMVGPKRAWAIPVVGVSSYTGEGVDDLLGRIAAHRQATADTELGRERRRRVAEFRLQKTAETLLLERFTTGAQPFSPALADSLSNRASDPYAAARELIARTIRKEYSNDLACAKLTITWLEPQIKSQLQSERKDWEANEVGAFLKKAPERKEQFHTIGDFPVQRTYTAADIADTPLEDIGLPGRYPFTRGPYPTMYRSRTWTMRQIAGFGTGEDTNKRFKYLIAQGQTGISTDFDMPTLMGYDSDHPMSDGEVGREGVAIDTLADMEALLADIDLEKISVSFTINPSAWILLAMYVALGEKRGYDLNKLSGTVQADILKEYMAQKEYIYPIAPSVRIVRDIITYSAKNLKRYNPINISGYHISEAGSSPLQEAAFTLANLITYVNEVTKTGMHVDEFAPRLAFFFVSQGDFFEEVAKFRALRRCYAKIMKERFGARNPESMRLRFHCQTAAATLTKPQYMVNVVRTSLQALSAVLGGAQSLHTNGYDEAFAIPTEDAMKMALRTQQIIAEESGVADVIDPLGGSYYVEALTTEYEKKIFEILEEVEKRGGTIKLIEQGWFQKQIADFAYETALRKQSGQKPVIGVNRFVENEEDVKIEIHPYDNTTAERQISRTRRVRAERDEAKVQAMLDQLVAVAKDESQNLMPLTIELVKAGATMGDIVEKLKGIWGTYRETPVF

SEQ ID NO: 190 - DNA, 849 bp, Clostridium acetobutylicum; identical to SEQ ID NO: 137
  misc_feature: hbd

SEQ ID NO: 191 - DNA, 10647 bp, Artificial sequence
  Synthetic polynucleotide
  misc_feature: pMTL83155-thlA-hbd-Pwl-meaBhcmA-hcmB
cctgcaggataaaaaaattgtagataaattttataaaatagttttatctacaatttttttatcaggaaacagctatgaccgcggccgcaatatgatatttatgtccattgtgaaagggattatattcaactattattccagttacgttcatagaaattttcctttctaaaatattttattccatgtcaagaactctgtttatttcattaaagaactataagtacaaagtataaggcatttgaaaaaataggctagtatattgattgattatttattttaaaatgcctaagtgaaatatatacatattataacaataaaataagtattagtgtaggatttttaaatagagtatctattttcagattaaatttttgattatttgatttacattatataatattgagtaaagtattgactagcaaaattttttgatactttaatttgtgaaatttcttatcaaaagttatatttttgaataatttttattgaaaaatacaactaaaaaggattatagtataagtgtgtgtaattttgtgttaaatttaaagggaggaaatgaacatgaaacatatgaaagaagttgtaatagctagtgcagtaagaacagcgattggatcttatggaaagtctcttaaggatgtaccagcagtagatttaggagctacagctataaaggaagcagttaaaaaagcaggaataaaaccagaggatgttaatgaagtcattttaggaaatgttcttcaagcaggtttaggacagaatccagcaagacaggcatcttttaaagcaggattaccagttgaaattccagctatgactattaataaggtttgtggttcaggacttagaacagttagcttagcagcacaaattataaaagcaggagatgctgacgtaataatagcaggtggtatggaaaatatgtctagagctccttacttagcgaataacgctagatggggatatagaatgggaaacgctaaatttgttgatgaaatgatcactgacggattgtgggatgcatttaatgattaccacatgggaataacagcagaaaacatagctgagagatggaacatttcaagagaagaacaagatgagtttgctcttgcatcacaaaaaaaagctgaagaagctataaaatcaggtcaatttaaagatgaaatagttcctgtagtaattaaaggcagaaagggagaaactgtagttgatacagatgagcaccctagatttggatcaactatagaaggacttgcaaaattaaaacctgccttcaaaaaagatggaacagttacagctggtaatgcatcaggattaaatgactgtgcagcagtacttgtaatcatgagtgcagaaaaagctaaagagcttggagtaaaaccacttgctaagatagtttcttatggttcagcaggagttgacccagcaataatgggatatggacctttctatgcaacaaaagcagctattgaaaaagcaggttggacagttgatgaattagatttaatagaatcaaatgaagcttttgcagctcaaagtttagcagtagcaaaagatttaaaatttgatatgaataaagtaaatgtaaatggaggagctattgcccttggtcatccaattggagcatcaggtgcaagaatactcgttactcttgtacacgcaatgcaaaaaagagatgcaaaaaaaggcttagcaactttatgtataggtggcggacaaggaacagcaatattgctagaaaagtgctaggaattctcaaaaattcggttaaataaaataattaggaggttcaatcatgtctattaaatcagttgcagttttaggttcaggtacaatgtcaagaggtattgttcaagcatttgctgaagcaggtatagatgtaataattagaggtagaacagaaggatcaataggaaaaggacttgctgctgttaagaaagcatacgataaaaaggtaagtaaaggaaagatatcacaagaagatgctgataaaatagttggtagagtatctactactacagaattagaaaaattagcagattgcgaccttataattgaggctgcatcagaagatatgaacataaagaaagattattttggaaaacttgaagaaatatgtaaaccagaaactatttttgctactaatacatcaagtttaagtattacagaagtagcaacagcaactaaaagaccagataagttcataggaatgcacttctttaatcctgctaatgtaatgaagcttgtagagattataagaggtatgaatacttctcaggaaacatttgatataattaaggaagcaagtattaaaataggaaaaactcctgtagaagtagcagaagcaccaggatttgttgttaataagatacttgttcctatgataaatgaggctgtaggtatacttgctgaaggtattgctagtgctgaagacatagacactgctatgaagttaggtgcaaaccatcctatgggaccattagcattaggtgatcttattggattagatgttgttttagcagtaatggatgtactttattctgagacaggtgattctaaatatagagctcatacacttcttagaaagtatgtaagagctggttggttaggtagaaagtctggtaaaggatttttcgcatattaaggtaccgcagatagtcataatagttccagaatagttcaatttagaaattagactaaacttcaaaatgtttgttaaatatataccaaactagtatagatattttttaaatactggacttaaacagtagtaatttgcctaaaaaattttttcaattttttttaaaaaatccttttcaagttgtacattgttatggtaatatgtaattgaagaagttatgtagtaatattgtaaacgtttcttgatttttttacatccatgtagtgcttaaaaaaccaaaatatgtcacatgcaattgtatatttcaaataacaatatttattttctcgttaaattcacaaataatttattaataatatcaataaccaagattatacttaaatggatgtttattttttaacacttttatagtaaatatatttattttatgtagtaaaaaggttataattataattgtatttattacaattaattaaaataaaaaatagggttttaggtaaaattaagttattttaagaagtaattacaataaaaattgaagttatttctttaaggagggaattattcatatgacttatgtaccatcatcagcacttttagaacaacttagagcaggaaatacttgggctttaggaagacttatatcaagagcagaagctggagttgcagaagctagacctgcacttgctgaagtatatagacatgcaggttcagctcatgttataggtttaacaggagtaccaggatctggtaaatcaactcttgtagcaaaacttacagcagctcttagaaaaagaggagaaaaagttggtatagtagctattgatcctagttctccatatagtggaggagcaatacttggagatagaattagaatgactgaattagcaaatgattcaggagtatttataagaagtatggcaactagaggtgctactggaggaatggctagagcagctcttgatgcagttgatttacttgatgtagctggatatcatactattattttagaaacagttggagtaggtcaagatgaagttgaagtagcacatgcttctgatactacagtagttgtatcagcacctggacttggtgatgaaatacaggcaattaaagctggagttttagaaattgctgatattcatgttgtaagtaaatgtgatagagatgatgcaaatagaactcttacagatcttaaacaaatgcttactttaggaacaatggtaggacctaaaagagcatgggctataccagttgtaggagtttcaagttatacaggagaaggtgtagatgatttacttggtagaattgcagctcatagacaagcaactgctgatacagaacttggaagagaaagaagaagaagagtagctgaatttagacttcaaaaaactgcagaaacattacttttagaaagatttactacaggagcacagcctttttcaccagcattagctgatagtctttctaatagagctagtgatccttatgcagctgcaagagaattaatagctagaactataagaaaagaatattctaatgatcttgcatgtgctaaacttactataacatggttagaaccacaaattaaaagtcaacttcagtctgaaagaaaagattgggaagcaaatgaagttggagcatttcttaaaaaagcacctgaaagaaaagaacaatttcatacaattggagattttccagtacagagaacttatacagctgcagatatagcagatactcctcttgaagatattggtttacctggaagatatccatttactagaggaccttatccaacaatgtatagaagtagaacttggacaatgagacaaatagctggatttggtactggagaagatacaaataaaagatttaaatatcttatagcacagggtcagactggaatatcaacagattttgatatgcctacattaatgggatatgattcagatcatccaatgagtgatggtgaagttggaagagaaggtgtagctatagatacacttgcagatatggaagcacttcttgctgatattgatttagaaaaaatttcagttagttttactataaatccaagtgcatggattcttttagcaatgtatgtagctttaggtgaaaaaagaggttatgatcttaataaactttctggaacagtacaagctgatatacttaaagaatatatggcacagaaagaatatatttatcctatagctccaagtgttagaattgtaagagatataattacttattctgcaaaaaatcttaaaagatataatcctattaatatttctggatatcatatatcagaagctggttcttcaccattacaagaagctgcatttactcttgcaaatcttattacttatgtaaatgaagtaactaaaacaggaatgcatgtagatgaatttgcacctagattagcatttttctttgttagtcaaggagatttctttgaagaagtagcaaaatttagagctttaagaagatgttatgctaaaataatgaaagaaagatttggagcaagaaatcctgaatctatgagacttagatttcattgtcaaactgctgcagctactcttacaaaaccacagtatatggttaatgttgtaagaacaagtcttcaagcattatctgctgtattgggaggagcacaaagtcttcatactaatggatatgatgaagcatttgctatacctactgaagatgcaatgaaaatggctcttagaacacaacagattatagctgaagaatctggagttgcagatgtaatagatcctcttggaggaagttattatgttgaagcattaactacagaatatgaaaagaaaatatttgaaattcttgaagaagtagaaaaaagaggtggaactattaaacttattgaacaaggatggtttcaaaaacagatagcagattttgcttatgaaactgcacttagaaaacaatcaggacagaaacctgttataggtgtaaatagatttgttgaaaatgaagaagatgtaaaaattgaaatacatccttatgataatactacagctgaaagacaaatatcaagaactagaagagttagagcagaaagagatgaagcaaaagtacaagctatgcttgatcagttagttgcagtagctaaagatgaaagtcagaatcttatgcctcttactattgaattagtaaaagcaggagctacaatgggtgatattgtagaaaaacttaaaggtatttggggaacttatagagaaacaccagtattttaagcactagttggagagcttcccacgatggatcagattcctattagagtattattagcaaaagtaggtttagatggacatgatagaggtgtaaaagttgtagcaagagcattaagagatgctggaatggatgtaatatatagtggtcttcatagaactcctgaagaagtagttaatacagcaattcaagaagatgtagatgttttaggagttagtttactttctggtgtacagcttactgtttttcctaaaatttttaaattacttgatgaaagaggagctggtgatttaatagtaattgctggaggagtaatgccagatgaagatgcagctgcaataagaaaacttggagtaagagaagttttacttcaagatacaccaccacaggcaataatagattcaataagaagtttagtagcagcaagaggagcaagataaccatggagatctcgaggcctgcagacatgcaagcttggcactggccgtcgttttacaacgtcgtgactgggaaaaccctggcgttacccaacttaatcgccttgcagcacatccccctttcgccagctggcgtaatagcgaagaggcccgcaccgatcgcccttcccaacagttgcgcagcctgaatggcgaatggcgctagcataaaaataagaagcctgcatttgcaggcttcttatttttatggcgcgccgccattatttttttgaacaattgacaattcatttcttattttttattaagtgatagtcaaaaggcataacagtgctgaatagaaagaaatttacagaaaagaaaattatagaatttagtatgattaattatactcatttatgaatgtttaattgaatacaaaaaaaaatacttgttatgtattcaattacgggttaaaatatagacaagttgaaaaatttaataaaaaaataagtcctcagctcttatatattaagctaccaacttagtatataagccaaaacttaaatgtgctaccaacacatcaagccgttagagaactctatctatagcaatatttcaaatgtaccgacatacaagagaaacattaactatatatattcaatttatgagattatcttaacagatataaatgtaaattgcaataagtaagatttagaagtttatagcctttgtgtattggaagcagtacgcaaaggcttttttatttgataaaaattagaagtatatttattttttcataattaatttatgaaaatgaaagggggtgagcaaagtgacagaggaaagcagtatcttatcaaataacaaggtattagcaatatcattattgactttagcagtaaacattatgacttttatagtgcttgtagctaagtagtacgaaagggggagctttaaaaagctccttggaatacatagaattcataaattaatttatgaaaagaagggcgtatatgaaaacttgtaaaaattgcaaagagtttattaaagatactgaaatatgcaaaatacattcgttgatgattcatgataaaacagtagcaacctattgcagtaaatacaatgagtcaagatgtttacataaagggaaagtccaatgtattaattgttcaaagatgaaccgatatggatggtgtgccataaaaatgagatgttttacagaggaagaacagaaaaaagaacgtacatgcattaaatattatgcaaggagctttaaaaaagctcatgtaaagaagagtaaaaagaaaaaataatttatttattaatttaatattgagagtgccgacacagtatgcactaaaaaatatatctgtggtgtagtgagccgatacaaaaggatagtcactcgcattttcataatacatcttatgttatgattatgtgtcggtgggacttcacgacgaaaacccacaataaaaaaagagttcggggtagggttaagcatagttgaggcaactaaacaatcaagctaggatatgcagtagcagaccgtaaggtcgttgtttaggtgtgttgtaatacatacgctattaagatgtaaaaatacggataccaatgaagggaaaagtataatttttggatgtagtttgtttgttcatctatgggcaaactacgtccaaagccgtttccaaatctgctaaaaagtatatcctttctaaaatcaaagtcaagtatgaaatcataaataaagtttaattttgaagttattatgatattatgtttttctattaaaataaattaagtatatagaatagtttaataatagtatatacttaatgtgataagtgtctgacagtgtcacagaaaggatgattgttatggattataagcggccggccagtgggcaagttgaaaaattcacaaaaatgtggtataatatctttgttcattagagcgataaacttgaatttgagagggaacttagatggtatttgaaaaaattgataaaaatagttggaacagaaaagagtattttgaccactactttgcaagtgtaccttgtacctacagcatgaccgttaaagtggatatcacacaaataaaggaaaagggaatgaaactatatcctgcaatgctttattatattgcaatgattgtaaaccgccattcagagtttaggacggcaatcaatcaagatggtgaattggggatatatgatgagatgataccaagctatacaatatttcacaatgatactgaaacattttccagcctttggactgagtgtaagtctgactttaaatcatttttagcagattatgaaagtgatacgcaacggtatggaaacaatcatagaatggaaggaaagccaaatgctccggaaaacatttttaatgtatctatgataccgtggtcaaccttcgatggctttaatctgaatttgcagaaaggatatgattatttgattcctatttttactatggggaaatattataaagaagataacaaaattatacttcctttggcaattcaagttcatcacgcagtatgtgacggatttcacatttgccgttttgtaaacgaattgcaggaattgataaatagttaacttcaggtttgtctgtaactaaaaacaagtatttaagcaaaaacatcgtagaaatacggtgttttttgttaccctaagtttaaactcctttttgataatctcatgaccaaaatcccttaacgtgagttttcgttccactgagcgtcagaccccgtagaaaagatcaaaggatcttcttgagatcctttttttctgcgcgtaatctgctgcttgcaaacaaaaaaaccaccgctaccagcggtggtttgtttgccggatcaagagctaccaactctttttccgaaggtaactggcttcagcagagcgcagataccaaatactgttcttctagtgtagccgtagttaggccaccacttcaagaactctgtagcaccgcctacatacctcgctctgctaatcctgttaccagtggctgctgccagtggcgataagtcgtgtcttaccgggttggactcaagacgatagttaccggataaggcgcagcggtcgggctgaacggggggttcgtgcacacagcccagcttggagcgaacgacctacaccgaactgagatacctacagcgtgagctatgagaaagcgccacgcttcccgaagggagaaaggcggacaggtatccggtaagcggcagggtcggaacaggagagcgcacgagggagcttccagggggaaacgcctggtatctttatagtcctgtcgggtttcgccacctctgacttgagcgtcgatttttgtgatgctcgtcaggggggcggagcctatggaaaaacgccagcaacgcggcctttttacggttcctggccttttgctggccttttgctcacatgttctttcctgcgttatcccctgattctgtggataaccgtattaccgcctttgagtgagctgataccgctcgccgcagccgaacgaccgagcgcagcgagtcagtgagcgaggaagcggaagagcgcccaatacgcagggccccctgcttcggggtcattatagcgattttttcggtatatccatcctttttcgcacgatatacaggattttgccaaagggttcgtgtagactttccttggtgtatccaacggcgtcagccgggcaggataggtgaagtaggcccacccgcgagcgggtgttccttcttcactgtcccttattcgcacctggcggtgctcaacgggaatcctgctctgcgaggctggccggctaccgccggcgtaacagatgagggcaagcggatggctgatgaaaccaagccaaccaggaagggcagcccacctatcaaggtgtactgccttccagacgaacgaagagcgattgaggaaaaggcggcggcggccggcatgagcctgtcggcctacctgctggccgtcggccagggctacaaaatcacgggcgtcgtggactatgagcacgtccgcgagctggcccgcatcaatggcgacctgggccgcctgggcggcctgctgaaactctggctcaccgacgacccgcgcacggcgcggttcggtgatgccacgatcctcgccctgctggcgaagatcgaagagaagcaggacgagcttggcaaggtcatgatgggcgtggtccgcccgagggcagagccatgacttttttagccgctaaaacggccggggggtgcgcgtgattgccaagcacgtccccatgcgctccatcaagaagagcgacttcgcggagctggtgaagtacatcaccgacgagcaaggcaagaccgatcgggccc

SEQ ID NO: 192 - DNA, 10539 bp, Artificial sequence
  Synthetic polynucleotide
  misc_feature: pMTL83155-thlA-phaB-Pwl-meaBhcmA-hcmB
cctgcaggataaaaaaattgtagataaattttataaaatagttttatctacaatttttttatcaggaaacagctatgaccgcggccgcaatatgatatttatgtccattgtgaaagggattatattcaactattattccagttacgttcatagaaattttcctttctaaaatattttattccatgtcaagaactctgtttatttcattaaagaactataagtacaaagtataaggcatttgaaaaaataggctagtatattgattgattatttattttaaaatgcctaagtgaaatatatacatattataacaataaaataagtattagtgtaggatttttaaatagagtatctattttcagattaaatttttgattatttgatttacattatataatattgagtaaagtattgactagcaaaattttttgatactttaatttgtgaaatttcttatcaaaagttatatttttgaataatttttattgaaaaatacaactaaaaaggattatagtataagtgtgtgtaattttgtgttaaatttaaagggaggaaatgaacatgaaacatatgaaagaagttgtaatagctagtgcagtaagaacagcgattggatcttatggaaagtctcttaaggatgtaccagcagtagatttaggagctacagctataaaggaagcagttaaaaaagcaggaataaaaccagaggatgttaatgaagtcattttaggaaatgttcttcaagcaggtttaggacagaatccagcaagacaggcatcttttaaagcaggattaccagttgaaattccagctatgactattaataaggtttgtggttcaggacttagaacagttagcttagcagcacaaattataaaagcaggagatgctgacgtaataatagcaggtggtatggaaaatatgtctagagctccttacttagcgaataacgctagatggggatatagaatgggaaacgctaaatttgttgatgaaatgatcactgacggattgtgggatgcatttaatgattaccacatgggaataacagcagaaaacatagctgagagatggaacatttcaagagaagaacaagatgagtttgctcttgcatcacaaaaaaaagctgaagaagctataaaatcaggtcaatttaaagatgaaatagttcctgtagtaattaaaggcagaaagggagaaactgtagttgatacagatgagcaccctagatttggatcaactatagaaggacttgcaaaattaaaacctgccttcaaaaaagatggaacagttacagctggtaatgcatcaggattaaatgactgtgcagcagtacttgtaatcatgagtgcagaaaaagctaaagagcttggagtaaaaccacttgctaagatagtttcttatggttcagcaggagttgacccagcaataatgggatatggacctttctatgcaacaaaagcagctattgaaaaagcaggttggacagttgatgaattagatttaatagaatcaaatgaagcttttgcagctcaaagtttagcagtagcaaaagatttaaaatttgatatgaataaagtaaatgtaaatggaggagctattgcccttggtcatccaattggagcatcaggtgcaagaatactcgttactcttgtacacgcaatgcaaaaaagagatgcaaaaaaaggcttagcaactttatgtataggtggcggacaaggaacagcaatattgctagaaaagtgctaggaattctcaaaaattcggttaaataaaataattaggaggttcaatcatgactcagcgcattgcgtatgtgaccggcggcatgggtggtatcggaaccgccatttgccagcggctggccaaggatggctttcgtgtggtggccggttgcggccccaactcgccgcgccgcgaaaagtggctggagcagcagaaggccctgggcttcgatttcattgcctcggaaggcaatgtggctgactgggactcgaccaagaccgcattcgacaaggtcaagtccgaggtcggcgaggttgatgtgctgatcaacaacgccggtatcacccgcgacgtggtgttccgcaagatgacccgcgccgactgggatgcggtgatcgacaccaacctgacctcgctgttcaacgtcaccaagcaggtgatcgacggcatggccgaccgtggctggggccgcatcgtcaacatctcgtcggtgaacgggcagaagggccagttcggccagaccaactactccaccgccaaggccggcctgcatggcttcaccatggcactggcgcaggaagtggcgaccaagggcgtgaccgtcaacacggtctctccgggctatatcgccaccgacatggtcaaggcgatccgccaggacgtgctcgacaagatcgtcgcgacgatcccggtcaagcgcctgggcctgccggaagagatcgcctcgatctgcgcctggttgtcgtcggaggagtccggtttctcgaccggcgccgacttctcgctcaacggcggcctgcatatgggctgaggtaccgcagatagtcataatagttccagaatagttcaatttagaaattagactaaacttcaaaatgtttgttaaatatataccaaactagtatagatattttttaaatactggacttaaacagtagtaatttgcctaaaaaattttttcaattttttttaaaaaatccttttcaagttgtacattgttatggtaatatgtaattgaagaagttatgtagtaatattgtaaacgtttcttgatttttttacatccatgtagtgcttaaaaaaccaaaatatgtcacatgcaattgtatatttcaaataacaatatttattttctcgttaaattcacaaataatttattaataatatcaataaccaagattatacttaaatggatgtttattttttaacacttttatagtaaatatatttattttatgtagtaaaaaggttataattataattgtatttattacaattaattaaaataaaaaatagggttttaggtaaaattaagttattttaagaagtaattacaataaaaattgaagttatttctttaaggagggaattattcatatgacttatgtaccatcatcagcacttttagaacaacttagagcaggaaatacttgggctttaggaagacttatatcaagagcagaagctggagttgcagaagctagacctgcacttgctgaagtatatagacatgcaggttcagctcatgttataggtttaacaggagtaccaggatctggtaaatcaactcttgtagcaaaacttacagcagctcttagaaaaagaggagaaaaagttggtatagtagctattgatcctagttctccatatagtggaggagcaatacttggagatagaattagaatgactgaattagcaaatgattcaggagtatttataagaagtatggcaactagaggtgctactggaggaatggctagagcagctcttgatgcagttgatttacttgatgtagctggatatcatactattattttagaaacagttggagtaggtcaagatgaagttgaagtagcacatgcttctgatactacagtagttgtatcagcacctggacttggtgatgaaatacaggcaattaaagctggagttttagaaattgctgatattcatgttgtaagtaaatgtgatagagatgatgcaaatagaactcttacagatcttaaacaaatgcttactttaggaacaatggtaggacctaaaagagcatgggctataccagttgtaggagtttcaagttatacaggagaaggtgtagatgatttacttggtagaattgcagctcatagacaagcaactgctgatacagaacttggaagagaaagaagaagaagagtagctgaatttagacttcaaaaaactgcagaaacattacttttagaaagatttactacaggagcacagcctttttcaccagcattagctgatagtctttctaatagagctagtgatccttatgcagctgcaagagaattaatagctagaactataagaaaagaatattctaatgatcttgcatgtgctaaacttactataacatggttagaaccacaaattaaaagtcaacttcagtctgaaagaaaagattgggaagcaaatgaagttggagcatttcttaaaaaagcacctgaaagaaaagaacaatttcatacaattggagattttccagtacagagaacttatacagctgcagatatagcagatactcctcttgaagatattggtttacctggaagatatccatttactagaggaccttatccaacaatgtatagaagtagaacttggacaatgagacaaatagctggatttggtactggagaagatacaaataaaagatttaaatatcttatagcacagggtcagactggaatatcaacagattttgatatgcctacattaatgggatatgattcagatcatccaatgagtgatggtgaagttggaagagaaggtgtagctatagatacacttgcagatatggaagcacttcttgctgatattgatttagaaaaaatttcagttagttttactataaatccaagtgcatggattcttttagcaatgtatgtagctttaggtgaaaaaagaggttatgatcttaataaactttctggaacagtacaagctgatatacttaaagaatatatggcacagaaagaatatatttatcctatagctccaagtgttagaattgtaagagatataattacttattctgcaaaaaatcttaaaagatataatcctattaatatttctggatatcatatatcagaagctggttcttcaccattacaagaagctgcatttactcttgcaaatcttattacttatgtaaatgaagtaactaaaacaggaatgcatgtagatgaatttgcacctagattagcatttttctttgttagtcaaggagatttctttgaagaagtagcaaaatttagagctttaagaagatgttatgctaaaataatgaaagaaagatttggagcaagaaatcctgaatctatgagacttagatttcattgtcaaactgctgcagctactcttacaaaaccacagtatatggttaatgttgtaagaacaagtcttcaagcattatctgctgtattgggaggagcacaaagtcttcatactaatggatatgatgaagcatttgctatacctactgaagatgcaatgaaaatggctcttagaacacaacagattatagctgaagaatctggagttgcagatgtaatagatcctcttggaggaagttattatgttgaagcattaactacagaatatgaaaagaaaatatttgaaattcttgaagaagtagaaaaaagaggtggaactattaaacttattgaacaaggatggtttcaaaaacagatagcagattttgcttatgaaactgcacttagaaaacaatcaggacagaaacctgttataggtgtaaatagatttgttgaaaatgaagaagatgtaaaaattgaaatacatccttatgataatactacagctgaaagacaaatatcaagaactagaagagttagagcagaaagagatgaagcaaaagtacaagctatgcttgatcagttagttgcagtagctaaagatgaaagtcagaatcttatgcctcttactattgaattagtaaaagcaggagctacaatgggtgatattgtagaaaaacttaaaggtatttggggaacttatagagaaacaccagtattttaagcactagttggagagcttcccacgatggatcagattcctattagagtattattagcaaaagtaggtttagatggacatgatagaggtgtaaaagttgtagcaagagcattaagagatgctggaatggatgtaatatatagtggtcttcatagaactcctgaagaagtagttaatacagcaattcaagaagatgtagatgttttaggagttagtttactttctggtgtacagcttactgtttttcctaaaatttttaaattacttgatgaaagaggagctggtgatttaatagtaattgctggaggagtaatgccagatgaagatgcagctgcaataagaaaacttggagtaagagaagttttacttcaagatacaccaccacaggcaataatagattcaataagaagtttagtagcagcaagaggagcaagataaccatggagatctcgaggcctgcagacatgcaagcttggcactggccgtcgttttacaacgtcgtgactgggaaaaccctggcgttacccaacttaatcgccttgcagcacatccccctttcgccagctggcgtaatagcgaagaggcccgcaccgatcgcccttcccaacagttgcgcagcctgaatggcgaatggcgctagcataaaaataagaagcctgcatttgcaggcttcttatttttatggcgcgccgccattatttttttgaacaattgacaattcatttcttattttttattaagtgatagtcaaaaggcataacagtgctgaatagaaagaaatttacagaaaagaaaattatagaatttagtatgattaattatactcatttatgaatgtttaattgaatacaaaaaaaaatacttgttatgtattcaattacgggttaaaatatagacaagttgaaaaatttaataaaaaaataagtcctcagctcttatatattaagctaccaacttagtatataagccaaaacttaaatgtgctaccaacacatcaagccgttagagaactctatctatagcaatatttcaaatgtaccgacatacaagagaaacattaactatatatattcaatttatgagattatcttaacagatataaatgtaaattgcaataagtaagatttagaagtttatagcctttgtgtattggaagcagtacgcaaaggcttttttatttgataaaaattagaagtatatttattttttcataattaatttatgaaaatgaaagggggtgagcaaagtgacagaggaaagcagtatcttatcaaataacaaggtattagcaatatcattattgactttagcagtaaacattatgacttttatagtgcttgtagctaagtagtacgaaagggggagctttaaaaagctccttggaatacatagaattcataaattaatttatgaaaagaagggcgtatatgaaaacttgtaaaaattgcaaagagtttattaaagatactgaaatatgcaaaatacattcgttgatgattcatgataaaacagtagcaacctattgcagtaaatacaatgagtcaagatgtttacataaagggaaagtccaatgtattaattgttcaaagatgaaccgatatggatggtgtgccataaaaatgagatgttttacagaggaagaacagaaaaaagaacgtacatgcattaaatattatgcaaggagctttaaaaaagctcatgtaaagaagagtaaaaagaaaaaataatttatttattaatttaatattgagagtgccgacacagtatgcactaaaaaatatatctgtggtgtagtgagccgatacaaaaggatagtcactcgcattttcataatacatcttatgttatgattatgtgtcggtgggacttcacgacgaaaacccacaataaaaaaagagttcggggtagggttaagcatagttgaggcaactaaacaatcaagctaggatatgcagtagcagaccgtaaggtcgttgtttaggtgtgttgtaatacatacgctattaagatgtaaaaatacggataccaatgaagggaaaagtataatttttggatgtagtttgtttgttcatctatgggcaaactacgtccaaagccgtttccaaatctgctaaaaagtatatcctttctaaaatcaaagtcaagtatgaaatcataaataaagtttaattttgaagttattatgatattatgtttttctattaaaataaattaagtatatagaatagtttaataatagtatatacttaatgtgataagtgtctgacagtgtcacagaaaggatgattgttatggattataagcggccggccagtgggcaagttgaaaaattcacaaaaatgtggtataatatctttgttcattagagcgataaacttgaatttgagagggaacttagatggtatttgaaaaaattgataaaaatagttggaacagaaaagagtattttgaccactactttgcaagtgtaccttgtacctacagcatgaccgttaaagtggatatcacacaaataaaggaaaagggaatgaaactatatcctgcaatgctttattatattgcaatgattgtaaaccgccattcagagtttaggacggcaatcaatcaagatggtgaattggggatatatgatgagatgataccaagctatacaatatttcacaatgatactgaaacattttccagcctttggactgagtgtaagtctgactttaaatcatttttagcagattatgaaagtgatacgcaacggtatggaaacaatcatagaatggaaggaaagccaaatgctccggaaaacatttttaatgtatctatgataccgtggtcaaccttcgatggctttaatctgaatttgcagaaaggatatgattatttgattcctatttttactatggggaaatattataaagaagataacaaaattatacttcctttggcaattcaagttcatcacgcagtatgtgacggatttcacatttgccgttttgtaaacgaattgcaggaattgataaatagttaacttcaggtttgtctgtaactaaaaacaagtatttaagcaaaaacatcgtagaaatacggtgttttttgttaccctaagtttaaactcctttttgataatctcatgaccaaaatcccttaacgtgagttttcgttccactgagcgtcagaccccgtagaaaagatcaaaggatcttcttgagatcctttttttctgcgcgtaatctgctgcttgcaaacaaaaaaaccaccgctaccagcggtggtttgtttgccggatcaagagctaccaactctttttccgaaggtaactggcttcagcagagcgcagataccaaatactgttcttctagtgtagccgtagttaggccaccacttcaagaactctgtagcaccgcctacatacctcgctctgctaatcctgttaccagtggctgctgccagtggcgataagtcgtgtcttaccgggttggactcaagacgatagttaccggataaggcgcagcggtcgggctgaacggggggttcgtgcacacagcccagcttggagcgaacgacctacaccgaactgagatacctacagcgtgagctatgagaaagcgccacgcttcccgaagggagaaaggcggacaggtatccggtaagcggcagggtcggaacaggagagcgcacgagggagcttccagggggaaacgcctggtatctttatagtcctgtcgggtttcgccacctctgacttgagcgtcgatttttgtgatgctcgtcaggggggcggagcctatggaaaaacgccagcaacgcggcctttttacggttcctggccttttgctggccttttgctcacatgttctttcctgcgttatcccctgattctgtggataaccgtattaccgcctttgagtgagctgataccgctcgccgcagccgaacgaccgagcgcagcgagtcagtgagcgaggaagcggaagagcgcccaatacgcagggccccctgcttcggggtcattatagcgattttttcggtatatccatcctttttcgcacgatatacaggattttgccaaagggttcgtgtagactttccttggtgtatccaacggcgtcagccgggcaggataggtgaagtaggcccacccgcgagcgggtgttccttcttcactgtcccttattcgcacctggcggtgctcaacgggaatcctgctctgcgaggctggccggctaccgccggcgtaacagatgagggcaagcggatggctgatgaaaccaagccaaccaggaagggcagcccacctatcaaggtgtactgccttccagacgaacgaagagcgattgaggaaaaggcggcggcggccggcatgagcctgtcggcctacctgctggccgtcggccagggctacaaaatcacgggcgtcgtggactatgagcacgtccgcgagctggcccgcatcaatggcgacctgggccgcctgggcggcctgctgaaactctggctcaccgacgacccgcgcacggcgcggttcggtgatgccacgatcctcgccctgctggcgaagatcgaagagaagcaggacgagcttggcaaggtcatgatgggcgtggtccgcccgagggcagagccatgacttttttagccgctaaaacggccggggggtgcgcgtgattgccaagcacgtccccatgcgctccatcaagaagagcgacttcgcggagctggtgaagtacatcaccgacgagcaaggcaagaccgatcgggccc

SEQ ID NO: 193 - DNA, 487 bp, Clostridium autoethanogenum
  misc_feature: promoter region of phosphate acetyltransferase
ggccgcaatatgatatttatgtccattgtgaaagggattatattcaactattattccagttacgttcatagaaattttcctttctaaaatattttattccatgtcaagaactctgtttatttcattaaagaactataagtacaaagtataaggcatttgaaaaaataggctagtatattgattgattatttattttaaaatgcctaagtgaaatatatacatattataacaataaaataagtattagtgtaggatttttaaatagagtatctattttcagattaaatttttgattatttgatttacattatataatattgagtaaagtattgactagcaaaattttttgatactttaatttgtgaaatttcttatcaaaagttatatttttgaataatttttattgaaaaatacaactaaaaaggattatagtataagtgtgtgtaattttgtgttaaatttaaagggaggaaatgaacatgaaaca

SEQ ID NO: 194 - DNA, 7884 bp, Artificial sequence; identical to SEQ ID NO: 153
  Synthetic polynucleotide
  misc_feature: pMTL82256-ptb-buk

SEQ ID NO: 195 - DNA, 6624 bp, Artificial sequence
  Synthetic polynucleotide
  misc_feature: pMTL82256-tesB
gagatctcgaggcctgcagacatgcaagcttggcactggccgtcgttttacaacgtcgtgactgggaaaaccctggcgttacccaacttaatcgccttgcagcacatccccctttcgccagctggcgtaatagcgaagaggcccgcaccgatcgcccttcccaacagttgcgcagcctgaatggcgaatggcgctagcataaaaataagaagcctgcatttgcaggcttcttatttttatggcgcgccgttctgaatccttagctaatggttcaacaggtaactatgacgaagatagcaccctggataagtctgtaatggattctaaggcatttaatgaagacgtgtatataaaatgtgctaatgaaaaagaaaatgcgttaaaagagcctaaaatgagttcaaatggttttgaaattgattggtagtttaatttaatatattttttctattggctatctcgatacctatagaatcttctgttcacttttgtttttgaaatataaaaaggggctttttagccccttttttttaaaactccggaggagtttcttcattcttgatactatacgtaactattttcgatttgacttcattgtcaattaagctagtaaaatcaatggttaaaaaacaaaaaacttgcatttttctacctagtaatttataattttaagtgtcgagtttaaaagtataatttaccaggaaaggagcaagttttttaataaggaaaaatttttccttttaaaattctatttcgttatatgactaattataatcaaaaaaatgaaaataaacaagaggtaaaaactgctttagagaaatgtactgataaaaaaagaaaaaatcctagatttacgtcatacatagcacctttaactactaagaaaaatattgaaaggacttccacttgtggagattatttgtttatgttgagtgatgcagacttagaacattttaaattacataaaggtaatttttgcggtaatagattttgtccaatgtgtagttggcgacttgcttgtaaggatagtttagaaatatctattcttatggagcatttaagaaaagaagaaaataaagagtttatatttttaactcttacaactccaaatgtaaaaagttatgatcttaattattctattaaacaatataataaatcttttaaaaaattaatggagcgtaaggaagttaaggatataactaaaggttatataagaaaattagaagtaacttaccaaaaggaaaaatacataacaaaggatttatggaaaataaaaaaagattattatcaaaaaaaaggacttgaaattggtgatttagaacctaattttgatacttataatcctcattttcatgtagttattgcagttaataaaagttattttacagataaaaattattatataaatcgagaaagatggttggaattatggaagtttgctactaaggatgattctataactcaagttgatgttagaaaagcaaaaattaatgattataaagaggtttacgaacttgcgaaatattcagctaaagacactgattatttaatatcgaggccagtatttgaaattttttataaagcattaaaaggcaagcaggtattagtttttagtggattttttaaagatgcacacaaattgtacaagcaaggaaaacttgatgtttataaaaagaaagatgaaattaaatatgtctatatagtttattataattggtgcaaaaaacaatatgaaaaaactagaataagggaacttacggaagatgaaaaagaagaattaaatcaagatttaatagatgaaatagaaatagattaaagtgtaactatactttatatatatatgattaaaaaaataaaaaacaacagcctattaggttgttgttttttattttctttattaatttttttaatttttagtttttagttcttttttaaaataagtttcagcctctttttcaatattttttaaagaaggagtatttgcatgaattgccttttttctaacagacttaggaaatattttaacagtatcttcttgcgccggtgattttggaacttcataacttactaatttataattattattttcttttttaattgtaacagttgcaaaagaagctgaacctgttccttcaactagtttatcatcttcaatataatattcttgacctatatagtataaatatatttttattatatttttacttttttctgaatctattattttataatcataaaaagttttaccaccaaaagaaggttgtactccttctggtccaacatatttttttactatattatctaaataatttttgggaactggtgttgtaatttgattaatcgaacaaccagttatacttaaaggaattataactataaaaatatataggattatctttttaaatttcattattggcctcctttttattaaatttatgttaccataaaaaggacataacgggaatatgtagaatatttttaatgtagacaaaattttacataaatataaagaaaggaagtgtttgtttaaattttatagcaaactatcaaaaattagggggataaaaatttatgaaaaaaaggttttcgatgttatttttatgtttaactttaatagtttgtggtttatttacaaattcggccggccgaagcaaacttaagagtgtgttgatagtgcagtatcttaaaattttgtataataggaattgaagttaaattagatgctaaaaatttgtaattaagaaggagtgattacatgaacaaaaatataaaatattctcaaaactttttaacgagtgaaaaagtactcaaccaaataataaaacaattgaatttaaaagaaaccgataccgtttacgaaattggaacaggtaaagggcatttaacgacgaaactggctaaaataagtaaacaggtaacgtctattgaattagacagtcatctattcaacttatcgtcagaaaaattaaaactgaatactcgtgtcactttaattcaccaagatattctacagtttcaattccctaacaaacagaggtataaaattgttgggagtattccttaccatttaagcacacaaattattaaaaaagtggtttttgaaagccatgcgtctgacatctatctgattgttgaagaaggattctacaagcgtaccttggatattcaccgaacactagggttgctcttgcacactcaagtctcgattcagcaattgcttaagctgccagcggaatgctttcatcctaaaccaaaagtaaacagtgtcttaataaaacttacccgccataccacagatgttccagataaatattggaagctatatacgtactttgtttcaaaatgggtcaatcgagaatatcgtcaactgtttactaaaaatcagtttcatcaagcaatgaaacacgccaaagtaaacaatttaagtaccgttacttatgagcaagtattgtctatttttaatagttatctattatttaacgggaggaaataattctatgagtcgcttttgtaaatttggaaagttacacgttactaaagggaatgtgtttaaactcctttttgataatctcatgaccaaaatcccttaacgtgagttttcgttccactgagcgtcagaccccgtagaaaagatcaaaggatcttcttgagatcctttttttctgcgcgtaatctgctgcttgcaaacaaaaaaaccaccgctaccagcggtggtttgtttgccggatcaagagctaccaactctttttccgaaggtaactggcttcagcagagcgcagataccaaatactgttcttctagtgtagccgtagttaggccaccacttcaagaactctgtagcaccgcctacatacctcgctctgctaatcctgttaccagtggctgctgccagtggcgataagtcgtgtcttaccgggttggactcaagacgatagttaccggataaggcgcagcggtcgggctgaacggggggttcgtgcacacagcccagcttggagcgaacgacctacaccgaactgagatacctacagcgtgagctatgagaaagcgccacgcttcccgaagggagaaaggcggacaggtatccggtaagcggcagggtcggaacaggagagcgcacgagggagcttccagggggaaacgcctggtatctttatagtcctgtcgggtttcgccacctctgacttgagcgtcgatttttgtgatgctcgtcaggggggcggagcctatggaaaaacgccagcaacgcggcctttttacggttcctggccttttgctggccttttgctcacatgttctttcctgcgttatcccctgattctgtggataaccgtattaccgcctttgagtgagctgataccgctcgccgcagccgaacgaccgagcgcagcgagtcagtgagcgaggaagcggaagagcgcccaatacgcagggccccctgcttcggggtcattatagcgattttttcggtatatccatcctttttcgcacgatatacaggattttgccaaagggttcgtgtagactttccttggtgtatccaacggcgtcagccgggcaggataggtgaagtaggcccacccgcgagcgggtgttccttcttcactgtcccttattcgcacctggcggtgctcaacgggaatcctgctctgcgaggctggccggctaccgccggcgtaacagatgagggcaagcggatggctgatgaaaccaagccaaccaggaagggcagcccacctatcaaggtgtactgccttccagacgaacgaagagcgattgaggaaaaggcggcggcggccggcatgagcctgtcggcctacctgctggccgtcggccagggctacaaaatcacgggcgtcgtggactatgagcacgtccgcgagctggcccgcatcaatggcgacctgggccgcctgggcggcctgctgaaactctggctcaccgacgacccgcgcacggcgcggttcggtgatgccacgatcctcgccctgctggcgaagatcgaagagaagcaggacgagcttggcaaggtcatgatgggcgtggtccgcccgagggcagagccatgacttttttagccgctaaaacggccggggggtgcgcgtgattgccaagcacgtccccatgcgctccatcaagaagagcgacttcgcggagctggtgaagtacatcaccgacgagcaaggcaagaccgatcgggccccctgcaggataaaaaaattgtagataaattttataaaatagttttatctacaatttttttatcaggaaacagctatgaccgcggccgcaaaatagttgataataatgcagagttataaacaaaggtgaaaagcattacttgtattcttttttatatattattataaattaaaatgaagctgtattagaaaaaatacacacctgtaatataaaattttaaattaatttttaattttttcaaaatgtattttacatgtttagaattttgatgtatattaaaatagtagaatacataagatacttaatttaattaaagatagttaagtacttttcaatgtgcttttttagatgtttaatacaaatctttaattgtaaaagaaatgctgtactatttactgtactagtgacgggattaaactgtattaattataaataaaaaataagtacagttgtttaaaattatattttgtattaaatctaatagtacgatgtaagttattttatactattgctagtttaataaaaagatttaattatatgcttgaaaaggagaggaatccaatgagtcaggcacttaaaaatttacttactttacttaatcttgaaaaaatagaagaaggtttatttagaggacagtcagaagatttaggattaagacaagtatttggaggtcaagtagttggtcaggcactttatgcagctaaagaaactgtacctgaagaaagacttgttcatagttttcattcttattttcttagacctggagattctaaaaaaccaattatatatgatgtagaaactcttagagatggaaattcatttagtgcaagaagagttgcagctattcaaaatggtaaacctatattttacatgacagcttcttttcaagcaccagaagctggatttgaacatcagaaaactatgccttcagcacctgctccagatggattaccatcagaaacacaaatagcacagagtttagctcatttacttcctccagtacttaaagataaatttatttgtgatagacctttagaagttagaccagttgaatttcataatcctcttaaaggacatgtagcagaaccacatagacaagtttggataagagctaatggaagtgtaccagatgatcttagagttcatcagtatcttcttggttatgcatctgatttaaattttcttcctgtagctttacaaccacatggaataggttttcttgaacctggaatacagatagcaactatagatcattcaatgtggtttcatagaccatttaatcttaatgaatggcttctttatagtgtagaatctacatcagcaagttctgctagaggatttgttaggggtgaattttatactcaagatggagtacttgttgctagtacagtacaggaaggtgttatgagaaatcataattaa